European Patent Application EP 4 623 992 A2, published October 1, 2025. Title: Antibodies specifically binding to human IL-1R7. Applicant: MAB Discovery GmbH. The sequence listing filed with the application follows.

SEQUENCE LISTING (1206 sequences)

SEQ ID NO: 1 - protein, 119 aa, Oryctolagus cuniculus
QSLEESGGRLVTPGTPLTLTCTISGIDLSAYAINWVRQAPGKGLEWIGGIANNGPTYYANWAKGRFTISKISTTVDLKITSPTTEDTATYFCARFPPGTNGGTDYFNIWGPGTLVTVSL

SEQ ID NO: 2 - protein, 114 aa, Oryctolagus cuniculus
QSVEESGGRLVTPGTPLTVTCTVSGFSLSGYDMNWVRQAPGKGLEWIGMIYPNSGTNYATWAKGRFTISKTPTTVALKITSPTTEDTATYFCARDSGWGAFDPWGPGTLVTISS

SEQ ID NO: 3 - protein, 119 aa, Oryctolagus cuniculus
QSLEESGGRLVTPGTPLTLTCTVSGFSLSTYAISWVRQAPGKGLEWIGGISNSGTTYYASWAKGRFTISKISTTVDLKITSPTTEDTATYFCARFPPGSNSGTDYFNIWGPGTLVTVSL

SEQ ID NO: 4 - protein, 113 aa, Oryctolagus cuniculus
QSLEESGGRLVTPGTPLTLTCTASGFSLSGLVVSWVRQAPGKGLEWIGVIGKSGNTYYASWAKGRFSISKTSSTTVDLKIASPTTEDTATYFCGRNISGSAVWGPGTLVTVSL

SEQ ID NO: 5 - protein, 126 aa, Oryctolagus cuniculus
QSLEESGGDLVKPGASLTLTCTASGFSFSSSYYMCWVRQAPGKWLEWIACIYAGSSGSTYYASWAKGRFTVSKTSSTTVTLEMTSLTAADTATYFCARDLGAGYAGYGYASDFNLWGPGTLVTVSS

SEQ ID NO: 6 - protein, 119 aa, Oryctolagus cuniculus
QSLEESGGRLVTPGTPLTLTCTVSGFSLSIYAISWVRQAPGKGLEWIGGIGNNGIIHYANWAKGRFTSSKISTTVDLKITSPTTEDTATYFCARFPPGSNSGTDYFNIWGPGTLVTVSL

SEQ ID NO: 7 - protein, 118 aa, Oryctolagus cuniculus
QSLEESGGDLVKPGASLTLTCTASGFSFSSSYYMCWVRQAPGKGLEWIGCIYGGSSGKTWYASWAKGRFTISKTSSTTVTLQMTSLTAADTATYFCARDNYDWYFNLWGPGTLVTVSS

SEQ ID NO: 8 - protein, 119 aa, Oryctolagus cuniculus
QSLEESGGRLVTPGTPLTLTCTVSGFSLSMYAINWVRQAPGKGLEWIGGIANNGPTYYASWAKGRFTISKISTTVDLRITSPTTEDTATYFCARFPPGSNSGTDYFNIWGPGTLVTVSL

SEQ ID NO: 9 - protein, 124 aa, Oryctolagus cuniculus
QSLEESGGDLVKPGASLTLTCKASGFDLSSYYYMCWFRQAPGKGPEWIACIYADDATTYYATWAKGRFTVSITSSTTVTLQMPSLTAADTATYFCARRDADYVGFIWAYYFNLWGPGTLVTVSS

SEQ ID NO: 10 - protein, 113 aa, Oryctolagus cuniculus
QSVEESGGRLVTPGTPLTLTCTVSGIDLSRNAMSWVRQAPGKGLEWIGIIRNTGTTWYASWAKGRFTISKTSTTVDLKITSPTTEDTATYFCARGNPGWASTWGPGTLVTVSS

SEQ ID NO: 11 - protein, 124 aa, Oryctolagus cuniculus
QEQLVESGGGLVQPGASLTLTCKTSGFSFSDNYAMCWVRQAPGKGLEWIACIYVGSGSTYYASWAQGRFTISKTSSTTVTLQMTSLTAADTATHFCARGVVIGNAYSMAHFSLWGSGTLVTVSS

SEQ ID NO: 12 - protein, 125 aa, Oryctolagus cuniculus
QSLEESGGGLVKPGASLTLTCTASGFSFSSGYYMCWVRQAPGKGLEWIGCIYTSSGSTYYASWAKGRFTISKTSSTTVTLQMTSLTAADTATYFCARRLNYVTYPAYGYGYFNLWGPGTLVTVSS

SEQ ID NO: 13 - protein, 121 aa, Oryctolagus cuniculus
QEQLEESGGDLVKPGASLTLTCTASGFSFNGNYYICWVRQAPGKGLEWIACIYAGSSGSTYYASWAKGRFTISKTSSTTVTLQMTSLTAADTATYFCVRDKPAGGSSYTLWGPGTLVTVSS

SEQ ID NO: 14 - protein, 120 aa, Oryctolagus cuniculus
QEQLEESGGDLVKPGASLTLTCTASGFSFSRSYYMCWVRQAPGKGLEWIACIYAGSSDSTYYASWAKGRFTISKTSSTTVTLQMTSLTAADTATYFCARGGGIIYTQNLWGPGTLVTVSS

SEQ ID NO: 15 - protein, 124 aa, Oryctolagus cuniculus
QSLEESGGDLVKPGASLTLTCTASGFSFVSMYWMCWVRQAPGKGLEWIACIYTGSSGKTHYASWAKGRSTISKTSSTTVTLQMTSLTAADTALYSCARAGSVGYGYDTAYFNLWGPGTLVTVSS

SEQ ID NO: 16 - protein, 114 aa, Oryctolagus cuniculus
QSVEESGGRLVTPGTPLTLTCTVSGFSLNSYDMSWVRQAPGKGLEYIGIIYDSGSTYYANWAKGRFTIAKTSTTVDLKITSPTTEDTATYFCARTLNTLPFNIWGPGTLVTVSL

SEQ ID NO: 17 - protein, 120 aa, Oryctolagus cuniculus
QEQLEESGGGLVQPEGSLTLTCTASGFSFSSSYWICWVRQAPGKGLEWIACIAAGSGSTYYASWAKGRFTISKTSSTTVTLQMTSLTAADTATYFCARDLGDDGYAYGLWGPGTLVTVSS

SEQ ID NO: 18 - protein, 120 aa, Oryctolagus cuniculus
QSLEESGGVLVKPGASLTLTCTASGIDFSSSYYICWVRQAPGKGLEWIACIYAGSSGSTYYASWAKGRFTISKTSSTTVTLQMTSLTAADTATYFCARGTGSSHYTSNLWGPGTLVTVSS

SEQ ID NO: 19 - protein, 120 aa, Oryctolagus cuniculus
QEQLVESGGGLVQPEGSLTLTCTASGFSFSDGYWMCWVRQAPGKGLEWIGCIYTGPGGTFYASWAKGRFTISKTSSTTVTLQLNSLTAADTATYFCARDLNGADSGSALWGPGTLVTVSS

SEQ ID NO: 20 - protein, 116 aa, Oryctolagus cuniculus
QSVEESGGRLVTPGTPLTLTCTASGFSLSSYAMSWVRQAPGKGLEWIGIIHYSGYTAYASWAKGRFTISKTSTTVDLKITSPTTEDTATYFCARGGDADNFYYNIWGPGTLVTVSL

SEQ ID NO: 21 - protein, 120 aa, Oryctolagus cuniculus
QEQLKESGGGLVTPGGTLTLTCTASGFTISNYQMTWVRQAPGKGLEYIGFIKADGSAYYANWAKGRFTISRTSTAVTLSLTTPTTGDTATYFCARDFYAGSSGNVNGDIWGPGTLVTVSL

SEQ ID NO: 22 - protein, 119 aa, Oryctolagus cuniculus
QSLEESGGRLVTPGTPLTLTCTVSGFSLNMYAINWVRQAPGKGLEWIGGIATNGIIHYASWVKGQFTISKISTTVDLKITSPTTEDTATYFCTRFPPGSNGGTAYFNIWGPGTLVTVSL

SEQ ID NO: 23 - protein, 114 aa, Oryctolagus cuniculus
QSVEESGGRLVTPGTPLTLTCTVSGFSLSNYDMNWVRQAPGKGLEWIGMIYPNSGTNYASWAKGRFTISKTPTTVALKITSPTTEDTATYFCARDSGWGAFDPWGPGTLVTVSS

SEQ ID NO: 24 - protein, 114 aa, Oryctolagus cuniculus
QSVEESGGRLVTPGTPLTLTCTVSGFSLSNYDMNWVRQAPGKGLEWIGMIYPNGGTNYATWAKGRFTISKTPTTVALKITSPTTEDTATYFCARDSGWGAFDPWGPGTLVTVSS

SEQ ID NO: 25 - protein, 112 aa, Oryctolagus cuniculus
QSVEESGGRLVTPGTPLTLTCTVSGIDLSSNAMIWVRQAPGKGLEWIGIIYASDSTYYATWAKGRFTISKTSTTVDLRMTSLTTEDTATYFCARGYSDIDIWGPGTLVTVSL

SEQ ID NO: 26 - protein, 119 aa, Oryctolagus cuniculus
QSLEESGGRLVTPGTPLTLTCTVSGFSLSMYTINWVRQAPGKGLEWIGGIATHGIIHYASWVKGRFTISKISTTVDLKITSPTTEDTATYFCARFPPGSNGGTAYFNIWGPGTLVTVSL

SEQ ID NO: 27 - protein, 121 aa, Oryctolagus cuniculus
QSVEESGGRLVTPGTPLTLTCTASGFSLSSNSISWVRQAPGKGLEWLGIISSSGSTYYASWAKGRFTISKASSTTVDLKITSPTTEDTATYFCAKGLGRGEYTSNDAFDPWGPGTLVTVSS

SEQ ID NO: 28 - protein, 118 aa, Oryctolagus cuniculus
QSLEESGGDLVKPGASLTLTCTASGFSFTSTYWMSWVRQAPGKGPEWIGCIVTGRGNTYYANWAKGRFTISKTSSTTVTLQMTSLTAADTATYFCARGSSDEIALDLWGQGTLVTVSS

SEQ ID NO: 29 - protein, 118 aa, Oryctolagus cuniculus
QSVEESGGRLVAPGTPLTLTCTVSGFSLNNYALSWVRQAPGKGLEYIGFINIIHGAYYASWAKGRFTISKTSTTVDLKITSPTTEDTATYFCARGPYYVGSEYVFDPWGPGTLVTVSS

SEQ ID NO: 30 - protein, 118 aa, Oryctolagus cuniculus
QSLEESGGRLVTPGGSLTLTCTVSGIDLSSHATSWVRQAPGKGLEWIGFIKTGGSAYYASWAKGRFTISKTSATVDLKITSPTTEDTATYFCASMFYAGDSGHYLHLWGPGTLVTVSS

SEQ ID NO: 31 - protein, 108 aa, Oryctolagus cuniculus
QSVEESGGGLVTPGGPLTLTCTVSGFSLSTYGVSWVRQAPGKGLEWIGYINTGGSASYATWAKGRFTISKTSTTVDLKITSPTTEDTATYFCAANNLWGPGTLVTVSS

SEQ ID NO: 32 - protein, 120 aa, Oryctolagus cuniculus
QSLEESGGDLVKPGASLTLTCTASGFSFSSNYYICWVRQAPGKGLEWIACIYTGSTGSTYYASWAKGRFTISKTSSTTVTLQMTSLTAADRATYFCARGGYSYGGAVSLWGPGTLVTVSS

SEQ ID NO: 33 - protein, 116 aa, Oryctolagus cuniculus
QSVEESGGRLVTPGTPLTLTCTVSGFSLTTYAMTWVRQAPGKGLEWIGIISNSGATAYASWAKGRFTISKTSTTVDLKITTPTTEDTATYFCARGRSGGWDALDPWGPGTLVTVSS

SEQ ID NO: 34 - protein, 122 aa, Oryctolagus cuniculus
QEQLEESGGDLVKPEGSLTLTCTASGFSFSSSYWICWVRQAPGKGLEWIACIGTSSTISYYASWAKGRFTISKTSSTTVTLRMTSLTAADTATYFCAREDYAGGTDYYFRLWGPGTLVTVSS

SEQ ID NO: 35 - protein, 116 aa, Oryctolagus cuniculus
QSVEESGGRLVTPGTPLTLTCTVSGFSLNNYAMSWVRQAPGKGLEWIGIIHYSGYIAYANWAKGRFTISKTSTTVDLKITSPTTEDTATYFCARGGDADNFYYNIWGPGTLVTVSL

SEQ ID NO: 36 - protein, 120 aa, Oryctolagus cuniculus
QEQLKESGGGLVTPGGTLTLTCTASGFTISNYQMTWVRQAPGKGLEYIGFIKPGGSAYYASWAKGRFTISRTSTTVTLKLTSPTTGDTATYFCARDFYAGSSGNVNGDIWGPGTLVTVSL

SEQ ID NO: 37 - protein, 116 aa, Oryctolagus cuniculus
QSLEESGGDLVKPGASLTLTCTASGFSFSSTYWACWVRQAPGKGLEWIACIDGGSSGITGYANWAKGRFTLSRTSSTAVTLQMTSLTAADTATYFCARELDYFNLWGPGTLVTVSS

SEQ ID NO: 38 - protein, 120 aa, Oryctolagus cuniculus
QEQLKESGGGLVTPGGTLTLTCTASGFTISSYQMTWVRQAPGKGLEYIGFINTGGSAYYASWAKGRFTISRTSTTVDLIITSPTTGDTATYFCARDFYAGSSGNVNGDIWGPGTLVTVSL

SEQ ID NO: 39 - protein, 119 aa, Oryctolagus cuniculus
QSLEESGGDLVKPGASLTLTCTASGFSFSSSYYMCWVRQAPGKGLEWIACIYAGSSGSTYYASWAKGRFTISKTSSTTVTLQMTSLTAADTATYFCARGAGSNGDFNLWGPGTLVTVSS

SEQ ID NO: 40 - protein, 120 aa, Oryctolagus cuniculus
QSLEESGGDLVKPGASLTLTCKASGFDFSSNYYMCWVRQAPGKGLEWIACIYTGSSGSTYYASWAKGRFTISKTSSTTVTLQMTSLTAADRATYFCARGAGSYGGAVRLWGPGTLVTVSS

SEQ ID NO: 41 - protein, 121 aa, Oryctolagus cuniculus
QSLEESGGDLVKPEGSLTLTCTASGFSFSSSYYMCWVRQAPGKGLEWIACIHAGSSGAAYYATWAKGRFTISKASSTTVTLHMTSLTAADTATYFCVRDGYDDYGDPFNLWGPGTLVTVSS

SEQ ID NO: 42 - protein, 118 aa, Oryctolagus cuniculus
QSVEESGGHLVTPGTPLTLTCTVSGFSLSNWIMSWVRQAPGEGLEWIGIITTSGNTYYASWAKGRFTISKTSTTVDLKITSPTTEDTATYFCARISAGSDSYIIDNIWGPGTLVTVSL

SEQ ID NO: 43 - protein, 120 aa, Oryctolagus cuniculus
QSLEESGGDLVKPGASLTLTCTASGFSLSSTYSMCWVRQAPGKGLEWVACIYTGSSGGTYYASWAKGRFTISKTSSTTVGLKMTSLTAADTATYFCARDAGNSGYYINLWGPGTLVTVSS

SEQ ID NO: 44 - protein, 112 aa, Oryctolagus cuniculus
QSLEESGGDLVKPGASLTLTCTASGFDFSSGYDMCWVRQAPGKGLELIACIYTVNDNTWYASWAKGRFTISKTSSTTVTLQMTSLTAADTATYFCARLYKLWGPGTLVTVSS

SEQ ID NO: 45 - protein, 120 aa, Oryctolagus cuniculus
QSLEESGGDLVKPGASLTLTCTASGIYFSSTYYTCWVRQAPGKGLEWIACIVDGSSGNTYYASWAKGRFTISKSSSTTVTLQMTSLTVADTATYFCGRPYVGYGYATDLWGPGTLVTVSS

SEQ ID NO: 46 - protein, 116 aa, Oryctolagus cuniculus
QSVEESGGRLVTPGTPLTLTCTVSGFSLSSAAMGWVRQAPGKGLEYIGYISTSGTPYYASWVNGRFTISKTSTTVDLKITSPTTEDTATYFCARDSYAGDYAFNLWGPGTLVTVSS

SEQ ID NO: 47 - protein, 114 aa, Oryctolagus cuniculus
QSVEESGGRLVTPGTPLTLTCTVSGFSLNSYDMSWVRQAPGKGLEYIGIIYNSGTTYYANWAKGRFTIAKTSTTVNLKITSPTTEDTATYFCARTHNTLPFYIWGPGTLVTVSL

SEQ ID NO: 48 - protein, 119 aa, Oryctolagus cuniculus
QSLEESGGDLVKPEGSLTLTCTASGFSFSSTYWICWVRQAPGKGLEWIACIYTDSSTSTYYASWAKGRFTISKTSSTTVTLQMTSLTAADTATYFCARGSGGSDYFNLWGPGTLVTVSS

SEQ ID NO: 49 - protein, 121 aa, Oryctolagus cuniculus
QEELVESGGGLVQPEGSLTLTCTASGFSFSSSYWICWVRQAPGKGLEWIACIVGGGGVNTYYANWAKGRFTISKTSSTTVTLEMTSLTVADTATYFCARDLGADGYAYHLWGPGTLVTVSS

SEQ ID NO: 50 - protein, 121 aa, Oryctolagus cuniculus
QELVESGGGLVQAGESLKLSCKASGIDFSSDGISWVRQAPGKGLKWIAFIYPGVGITHYAHSVKGRLTISSDNAQNTVFLQMTSLTASDTATYFCVRDPIYDDYGGRLDLWGQGTLVTVSS

SEQ ID NO: 51 - protein, 119 aa, Oryctolagus cuniculus
QSLEESGGRLVTPGTPLTLTCTVSGFSLSSYAISWVRQAPGKGLEWIGGVANNGITNYASWARGRFTISKISTTVDLKIISPTTEDTATYFCARFPPGSNGGTDYFNIWGPGTLVTVSL

SEQ ID NO: 52 - protein, 116 aa, Oryctolagus cuniculus
QSVEESGGRLVTPGTPLTLTCTVSGIDLSSNALGWVRQAPGKGLEYIGYISTGGSAYYATWVNGRFTISKTSTTVDLKMTSLTAADTATYFCARDSYAGDYAFNLWGPGTLVTVSS

SEQ ID NO: 53 - protein, 114 aa, Oryctolagus cuniculus
QSLEESGGRLVTPGTPLTLTCTVSGFSLNSYDMSWVRQAPGKGLEYIGIIYDSGSTYYASWAKGRFTIAKTSTTVDLKITSPTTEDTATYFCARARNTLPFNIWGPGTLVTVSL

SEQ ID NO: 54 - protein, 119 aa, Oryctolagus cuniculus
QSVEESGGRLVTPGTPLTLTCTVSGIDLSNYAMGWVRQAPGKGLEWIGVISSNGGTVYANWAKGRFTISKVSTSVPLKITSPTTEDTATYFCARGLYSASGWSYCFDIWGPGTLVTVSL

SEQ ID NO: 55 - protein, 118 aa, Oryctolagus cuniculus
QSVEESGGRLVTPGGSLTLTCTVSGIDLSVYAMSWVRQAPGKGLEWIGIITFSGNTYYASWAKGRFTISKTSTTVDLKITSPATGDTATYFCARFDFLVGLTYAGVLWGPGTLVTVSS

SEQ ID NO: 56 - protein, 118 aa, Oryctolagus cuniculus
QSVEESGGRLVTPGTPLTLTCAVSGFSLSTYGVSWVRQAPGKGLEWIGYINIYGRTYYANWAKSRFTISKTSTTVDLKMTSPTTEDTATYFCARNGASGTYYSSLYIWGPGTLVTVSL

SEQ ID NO: 57 - protein, 119 aa, Oryctolagus cuniculus
QSLEESGGRLVTPGTPLTLTCTVSGFSLSMYAINWVRQAPGKGLEWIGGIANNGPTYYASWAKGRFTISKISTTVDLKITSPTTEDTATYFCARFPPGSNSGTDYFNIWGPGTLVTVSL

SEQ ID NO: 58 - protein, 111 aa, Oryctolagus cuniculus
QSVEESGGRLVTPGTPLTLTCTVSGIDLSRYAMSWVRQAPGKGLEYIGIISSSGNSYYASWAKGRFTISKASTTVDLKITVPTTEDTATYFCVGGSGWDLWGQGTLVTVSS

SEQ ID NO: 59 - protein, 115 aa, Oryctolagus cuniculus
QSLEESGGRLVTPGGSLTLTCTVSGIDLSSYAMGWVRQAPGKGLEYIGIISSGLTYYASWAKGRFTISKTSTTVDLKMTSLTTEDTATYFCARGLGAASATWDIWGPGTLVTVSL

SEQ ID NO: 60 - protein, 120 aa, Oryctolagus cuniculus
QSLEESGGDLVKPGASLALTCTASGFSFSSSYWICWVRQAPGKGLEWIACINFGRSGNIYYARWAKGRFTISKTSSTTVTLQMTSLTAADTATYFCARDKAGDSYYFNLWGPGTLVTVSS

SEQ ID NO: 61 - protein, 112 aa, Oryctolagus cuniculus
QSLEESGGRLVTPGTPLTLTCTASGFSLNNYYMTWVRQAPGEGLEYIGFIDPYSSPYYASWAKGRFTISRTSTTVDLKISSPTAEDTATYFCARGVAVGDIWGPGTLVTVSL

SEQ ID NO: 62 - protein, 112 aa, Oryctolagus cuniculus
QSLEESGGRLVTPGTPLTLTCTVSGIDLSSYHMSWVRQAPGKGLEWIGVIYGSGSAWYASWAKGRFTISKTSTTVDLKITSPTTEDTATYFCVRGILVSDLWGPGTLVTVSS

SEQ ID NO: 63 - protein, 121 aa, Oryctolagus cuniculus
QQQLEESGGGLVKPEGSLTLTCKASGFDFSTIPMCWVRQAPGKGLEWIACIYPDYGDTFYATWAKGRFTISKTSSTTVTLQMTSLTVADTATYFCARGPIMVVSPSYFNFWGPGTLVTVSS

SEQ ID NO: 64 - protein, 123 aa, Oryctolagus cuniculus
QSLEESGGDLVQPGASLTLTCTASGFIFSDNYAMCWVRQAPGKGLEWIACIFGSSGSIAYATWAKGRFTISKTSSTTVTLQMTSLAAADTATYFCARSYYSGGYKYVYVFDLWGPGTLVTVSS

SEQ ID NO: 65 - protein, 113 aa, Oryctolagus cuniculus
QEQLVESGGGLFQPGGSLTLTCTASGFTISSYHMGWVRQAPGEGLEYIGFITTTGGSYYASWARGRFTISKTSTTVDLKMTSLTAADTATYFCAKGIAVASLWGPGTLVTVSS

SEQ ID NO: 66 - protein, 118 aa, Oryctolagus cuniculus
QSLEESGGDLVKPGASLRLTCTASGLSFSSRYWIYWVRQAPGKGLEWIACIDTGSRGFTYYPSWAKGRFTISKTSSTTVTLQMTSLTAADTATYFCARLDTYDDYDLWGPGTLVTVSS

SEQ ID NO: 67 - protein, 118 aa, Oryctolagus cuniculus
QSVEESGGRLVTPGTPLTLTCTASGFSLYSYFLTWVRQSPGKGLEWIGFMNSGGSTYYASWVNGRFTISKTSATVDLKITGATTEDTATYFCARMFYAGDSGHYFDLWGPGTLVTVSS

SEQ ID NO: 68 - protein, 121 aa, Oryctolagus cuniculus
QSVEESGGRLVTPGTPLTLTCTVSGIDLSSYAMSWVRQAPGKGLEWIGMIRSSGITWYASWAKGRFTISKTSTTVDLKITSPTTEDTATYFCARDSDYDDYGNSYYGMDPWGPGTLVTVSS

SEQ ID NO: 69 - protein, 120 aa, Oryctolagus cuniculus
QEQLEESGGDLVKPEGSLTLTCTASGFDFSSNAMCWVRQAPGKGLEWIACIYAGSRGSAYYASWVNGRFSISKTSSTTVTLQMTSLTAADTATYFCAREYVGSQGYFNLWGPGTLVTVSS

SEQ ID NO: 70 - protein, 118 aa, Oryctolagus cuniculus
QSVEESGGRLVTPGTPLTLTCTVSGFSLSVYAMSWVRQAPGKGLEWIGIITWSADTYYTSWAKGRFSISKTSTTVDLKVASPTTEDTATYFCARFDYLVGGTWAGVLWGPGTLVTVSS

SEQ ID NO: 71 - protein, 117 aa, Oryctolagus cuniculus
QSVEESGGRLVTPGTPLTLTCTASGFSLNSYAMGWVRQAPGKGLEWIGINGVSGTTYYATWANGRFTISKTSTTVDLKIIRPTTEDTATYFCARGVGDTTDTQLDLWGQGTLVTVSS

SEQ ID NO: 72 - protein, 120 aa, Oryctolagus cuniculus
QEQLVESGGGLVQPEGSLTLTCTASGFDFSGSYWNCWVRQAPGKGLEWIACIDGEGSGNTYYASWVNGRFTISKTSSTTVTLQMTRLTAADTATYFCARDPSAWGGLDLWGPGTLVTVSS

SEQ ID NO: 73 - protein, 118 aa, Oryctolagus cuniculus
QSLEESGGDLVKPGASLTLTCKASGFSFSSGYDMCWVRQAPGKGLEWIACIDTGDGSTYYASWVNGRFTISKTSSTTVTLQMTSLTAADTATYFCARYNNGWDYFNLWGPGTLVTVSS

SEQ ID NO: 74 - protein, 108 aa, Oryctolagus cuniculus
QSVEESGGRLVTPGTPLTLTCTVSGFSLIAYGVNWVRQAPGKGLQWIGSISNSGGTYYASWAKGRFTVSKTSTTVDLRITSPTTEDTATYFCGRGSLWGPGTLVTVSS

SEQ ID NO: 75 - protein, 124 aa, Oryctolagus cuniculus
QEQLVESGGGLVQPEGSLTLTCTASGFTISNSYYMCWVRQAPGKGLEWIGCIDAGSVGDTSYATWAKGRFTISKTSSTTVTLQMTSLTAADTATYFCARRYGAGSGYFISPNLWGPGTLVTVSS

SEQ ID NO: 76 - protein, 120 aa, Oryctolagus cuniculus
QEQLVESGGGLVQPEGSLTLTCKASGFDFSSNAMCWVRQAPGKGPEWIACIYNGDGSTYYASWVNGRFTISRSTSLNTVTLQMTSLTAADTATYFCAREYVDSQGYFNLWGPGTLVTVSS

SEQ ID NO: 77 - protein, 117 aa, Oryctolagus cuniculus
QSLEESGGRLVTPGTPLTLTCTVSGFSLSSYAMGWVRQAPGKGLEWIGIISNSGATAYASWAKGRFTISKTSSTTVDLKMTTPTTEDTATYFCARGRSGGWDAFDPWGPGTLVTVSS

SEQ ID NO: 78 - protein, 108 aa, Oryctolagus cuniculus
QSLEESGGRLVTPGTPLTLTCTVSGIDLNTNGVSWVRQAPGKGLEWIGYIFTGGNTYYASWAKGRFTISKTSTTVDLKMTSLTTADTATYFCARFDIWGPGTLVTVSL

SEQ ID NO: 79 - protein, 121 aa, Oryctolagus cuniculus
QEQLEESGGGLVKPGASLTFTCRASGFSFSSGYYMCWVRQAPGKGLEWIACIYVGITGSTYYASWAKGRFTISKTSSTSVTLQMTSLTAADTATYFCARDTGNSNYQFNLWGPGTLVTVSS

SEQ ID NO: 80 - protein, 126 aa, Oryctolagus cuniculus
QSLEESGGDLVKPGASLTLTCTASGFSFSSGYCLCWVRQAPGKGLEWIACKHGGASGTTYYATWAKGRFTISKTSSTTVTLQVTSLTVADTATYFCARDDVSVGDANYPYTAFDLWGPGTLVTVSS

SEQ ID NO: 81 - protein, 120 aa, Oryctolagus cuniculus
QSLEESGGDLVKPGASLTLTCTASGSDISSYWMCWVRQAPGKGLEWIACSYAGGSGGTYYASWAKGRFTISKTSSTTVTLQMTSLTAADTATYFCAREAYSSANSYYDLWGPGTLVTVSS

SEQ ID NO: 82 - protein, 120 aa, Oryctolagus cuniculus
QSLEESGGDLVKPGASLTLTCTASGFSFSSYYYMSWVRQAPGKGLEWIACTDGTGGITYYASWAKGRFTTSKTSPTTVTLQMTSLTAADTATYFCARDPTAAGGVYFDLWGPGTLVTVSS

SEQ ID NO: 83 - protein, 118 aa, Oryctolagus cuniculus
QEQLEESGGDLVKPEGSLTLTCTASGFDFSYNTICWVRQAPGKGLEWIAYINTGSSGTTYYASWAKGRFTISKTSSTTVTLQLNSLTAADTATYFCAGGSGYSKFRLWGPGTLVTVSS

SEQ ID NO: 84 - protein, 118 aa, Oryctolagus cuniculus
QSLEESGGDLVKPGASLTLTCTASGFSFSSSYYMCWVRQAPGKGLEWIACIYAGSSGSTYYASWAKGRFTISKTSSTTVALQMTSLTAADTATYFCARDRGDTDISLWGPGTLVTVSS

SEQ ID NO: 85 - protein, 118 aa, Oryctolagus cuniculus
QSVEESGGRLVAPGTPLTLTCTVSGFSLSNYAMSWVRQAPGKGLEYIGFINIIDSTYYTNWAKGRFTISKTSTTVDLKMTSPTTEDTATYFCARGPYYVNNENVFDPWGPGTLVTVSS

SEQ ID NO: 86 - protein, 116 aa, Oryctolagus cuniculus
QSLEESGGRLVTPGGSLTLTCTVSGIDLSNYAVGWVRQAPGKGLEYIGVINAGGSAYYATWAKGRFTISRTSTTVDLKITSPTTEDTATYFCARSYAGNRYDFAIWGPGTLVTVSL

SEQ ID NO: 87 - protein, 116 aa, Oryctolagus cuniculus
QSLEESGGDLVKPGASLTLTCTASGFSVSSSYYMCWVRQAPGKGLEWIACIYADSSGSTYYASWAKGRFTISSTSSTTVTLQMTSLTAADTATYFCARGPYSFDFWGPGTLVTVSS

SEQ ID NO: 88 - protein, 120 aa, Oryctolagus cuniculus
QSLEESGGDLVKPGASLTLTCTASGFSFSSRYYVCWVRQAPGKGLEWIACIDAGDGSTDYARWAKGRFTISKTSSTTVTLQMTGLTAADTATYFCARGDAYRDDYASDLWGPGTLVTVSS

SEQ ID NO: 89 - protein, 117 aa, Oryctolagus cuniculus
QSLEESGGRLVTPGESLTLTCTVSGIDLSANAMSWVRQAPGKGLEWIGTIFDTYLTYNANWAKGRFTISRTSTTVELKMTSPTIEDTATYFCARYIGSVGYRRMDIWGPGTLVTVAL

SEQ ID NO: 90 - protein, 118 aa, Oryctolagus cuniculus
QSVEESGGRLVTPGGSLTLTCTASGFSLNNYHMSWVRQAPGKGLEWIGFIRTDGSAFYATWAKGRFTISKTSATVDLKVTSATTEDTATYFCARMFYAGDSGHYFDLWGPGTLVTVSS

SEQ ID NO: 91 - protein, 118 aa, Oryctolagus cuniculus
QSVEESGGRLVTPGTPLTLTCTVSGFSLSNYGLTWVRQAPGKGLEWIGYINNNGRTYYASRAKGRFTISKTSTTVDLQMTSPTTEDTATYFCARNGAGGYYYSSLYIWGPGTLVTVSL

SEQ ID NO: 92 - protein, 118 aa, Oryctolagus cuniculus
QSLEESGGDLVKPGASLTLTCTASGFSFSSSYYMCWVRQAPGKGLEWIACVYAGSSGSTYYASWAKGRFTISKTSSTTVTLQMTSLTAADTATYFCARDRGGTDISLWGPGTLVTVSS

SEQ ID NO: 93 - protein, 116 aa, Oryctolagus cuniculus
QSVEESGGRLVTPGTPLTLTCKASGFSLSTYAMSWVRQAPGKGLEYIGIIDASVTTYYASWAKGRFTISKTSTTVDLTITSPTTEDTATYFCARSSSTYAYGFDPWGPGTLVTVSS

SEQ ID NO: 94 - protein, 118 aa, Oryctolagus cuniculus
QEQLKESGGGLVQPGGSLKLSCKASGFDFSNYGVSWVRQAPGKGLEWVGYIDPVFRSAYYASWVNGRFTISSHNAQNTLYLQLNSLTAADTATYFCARKGYFHYFNLWGPGTLVTVSS

SEQ ID NO: 95 - protein, 119 aa, Oryctolagus cuniculus
QSLEESGGDLVKPGASLTLTCTASGFSFSVSYWICWVRQAPGKGLEWIACIGGNSGNIYYARWAKGRFTISKTSSTTVTLQMTSLTAADTATYFCARDRAGNSYYFNLWGPGTLVTVSS

SEQ ID NO: 96 - protein, 112 aa, Oryctolagus cuniculus
QSLEESGGDLVKPGASLTLTCTASGFSFSSGYDMCWVRQAPGKGLEWIGCIYSSNGLTWYATWAKGRFTVSKTSSTTVTLQMTSLTAADTASYFCWRVWSLWGPGTLVTVSS

SEQ ID NO: 97 - protein, 119 aa, Oryctolagus cuniculus
QEQLVEYGGDLVQPEGSLTLTCKASGFDFSSNAMCWVRQAPGKGLEWIGCIVTGSGSTYYASWAKGRITISETSSTTVTLQMTSLTAADTATYFCARGYDGYGYVLVLWGPGTLVTVSS

SEQ ID NO: 98 - protein, 120 aa, Oryctolagus cuniculus
QSLEESGGDLVKPGASLTLTCTASGFSFSSSYYMCWVRQAPGKGLEWVAGVDGSGGIKWYANWAKGRFTISKTSPTTVTLQMTSLTAADTATYFCARDPTAAGGVYFDLWGPGTLVTVSS

SEQ ID NO: 99 - protein, 122 aa, Oryctolagus cuniculus
QSLEESGGDLVKPGASLTLTCTASGFSFSSSYWIYWVRQAPGKGLEWIACFHAGSGSTYYASWVNGRFTISKTSSTTVTLQMTSLTAADTATYFCARGSGSIYYTPSYFDLWGPGTLVTVSS

SEQ ID NO: 100 - protein, 108 aa, Oryctolagus cuniculus
QSVEESGGRLVTPGTPLTLTCTVSGFSLSRYGVSWVRQAPGKGLEWIAWISSSGSAYYATWAKGRFTISKTSTTVDLKITSPTTEDTATYFCGESDIWGPGTLVTVSL

SEQ ID NO: 101 - protein, 119 aa, Oryctolagus cuniculus
QSLEESGGGLVQPEGSLTLACTASGFSFNNNYYMCWVRQAPGKGLEWVACIYTGSTGSTYYANWAKGRFTISKLSSTTVTLQMTSLTAADTATYFCARDDKVEHGYGLWGPGTLVTVSS

SEQ ID NO: 102 - protein, 128 aa, Oryctolagus cuniculus
QSLEESGGDLVKPGASLTLTCTASGFSFSSNYYMCWVRQAPGKGLEWIACIYAGSSGSSYYASWAKGRFTISKTSSTTVTLQMTSLTAADTATYFCARSMEAYGYAGYAMPGYYFNLWGPGTLVTVSS

SEQ ID NO: 103 - protein, 121 aa, Oryctolagus cuniculus
QSVEESGGRLVTPGTPLTLTCTVSGFSLSSYAMSWVRQAPGKGLEWIGIIRRSGATWYANWARGRFTISKTSTTVDLKITSPTTEDTATYFCARDSDYDDYGDSYYGMDPWGPGTLVTVSS

SEQ ID NO: 104 - protein, 127 aa, Oryctolagus cuniculus
QSLEESGGDLVKPGASLTLTCTASGFSFSSSYCMCWVRQAPGKGLEWIGCIYDGSSDSAYYATWAKGRFTISKTSSTTVTLQMTSLTAADTATYFCARDYDTYDYDGYTYAAGFDLWGPGTLVTVST

SEQ ID NO: 105 - protein, 116 aa, Oryctolagus cuniculus
QSLEESGGRLVTPGTPLTLTCTVSGIDLSSYAMGWVRQAPGKGLQYIGIITYGGSTYYASWAKGRFTISKTSTTVNLKMTSLTTEDTATYFCARGLGGASTTWDIWGPGTLVTVSL

SEQ ID NO: 106 - protein, 123 aa, Oryctolagus cuniculus
QSLEESGGDLVKPGASLTLTCTASGFSFSSGYDMCWVRQAPGKGLEWIACIAVYSSGSTYYASWAKGRFTISKTSSTTVTLQMPSLTAADTATYFCARDIITDSVWITRLDLWGQGTLVTVSS

SEQ ID NO: 107 - protein, 118 aa, Oryctolagus cuniculus
QSVEESGGRLVTPGTPLTLTCTASGFSFSDYYMSWVRQAPGKGLEWIGVVSWNGNTYYASWAKGRFTVSKTSTTVDLKIISPTTEDTATYFCARFDYLVGDTYAGVLWGPGTLVTVSS

SEQ ID NO: 108 - protein, 119 aa, Oryctolagus cuniculus
QSLEESGGRLVTPGTPLTLTCTVSGIDLSSHATSWVRQAPGKGLEWIGFIKSGGSTYYASWAKGRFTISETSATVDLKITSPTTEDTATYFCASMFYAGDSSGNYLHLWGPGTLVTVSS

SEQ ID NO: 109 - protein, 121 aa, Oryctolagus cuniculus
QSLEESGGDLVKPGASLTLTCTASGFSFSSGYWICWVRQAPGKGLEWIACIDAGSNGSTYYASWARGRFTISKTSSTTVTLQMTSLTAADTATYFCAREGSSAYPSYFNFWGPGTLVTVSS

SEQ ID NO: 110 - protein, 116 aa, Oryctolagus cuniculus
QSLEESGGRLVTPGGSLTLTCTVSGIDLSSYTMAWVRQAPGKGLEYIGVINTGGSAYYASWAKGRFTISKTSTTVDLKITSPTTEDTATYFCARSYGGNRYDFNIWGPGTLVTVSL

SEQ ID NO: 111 - protein, 119 aa, Oryctolagus cuniculus
QSVEESGGRLVTPGTPLTLTCTASGFSLSSYHMCWVRQAPGKGLEWIGFIKADGNTYYATWAKGRFTISRSSATVDLKITSATAEDTATYFCARMFYAGHTSGHYFDLWGPGTLVTVSS

SEQ ID NO: 112 - protein, 130 aa, Oryctolagus cuniculus
QSLEESGGDLVKPEASLTLTCTASGFSFSGDYDMCWVRQAPGKGLEWIACIGAGSSNDTYYASWAKGRFTISKTSSTTVTLQMTSLTAADTATYFCARGFDYTYGDAGYTYSTSHYFNLWGPGTLVTVSS

SEQ ID NO: 113 - protein, 120 aa, Oryctolagus cuniculus
QSLEESGGGLVQPEGSLTLTCTASGFSFSSSYYMCWVRQAPGKGLEWIACISVGSSGSTYYANWAKGRFTISKTSSTTVTLQMTSLTAADTATYFCAREGADYQGHFNLWGPGTLVTVSS

SEQ ID NO: 114 - protein, 121 aa, Oryctolagus cuniculus
QSVEESGGRLVTPGTPLTLTCTVSGFSLSSYAMSWVRQAPGKGLEWIGIIRRSGFTYYASWARGRFTISKTSTTVDLKITSPTTEDTATYFCARDSDYDDYGNSYYGMDPWGPGTLVTVSS

SEQ ID NO: 115 - protein, 119 aa, Oryctolagus cuniculus
QSVEESGGRLVTPGTPLTLTCTVSGFSLSSYTMTWVRQAPGKGLEWIGLISRSGRTYYATWAKGRLTISKTSTTVDLKITSPTTEDTATYFCAREIGSGYDAPYYFNLWGPGTLVTVSS

SEQ ID NO: 116 - protein, 119 aa, Oryctolagus cuniculus
QSLEESGGGLVQPEGSLTLTCTASGFSFNSKYYMCWVRQAPGKGLEWIACIYTGTTGSTYYASWAKYRFTISKISSTTVTLQMTSLTAADTATYFCARDDRVEHGYGLWGPGTLVTVSS

SEQ ID NO: 117 - protein, 119 aa, Oryctolagus cuniculus
QEQLEESGGGLVKPEGSLTLTCKASGFTISSYYIYWVRQAPGKGLEWIGCIAIINSITYYANWAKGRFTISKTSSTTVTLQMTSLTAADTATYFCARDLSSSIYDMDLWGPGTLVTVSS

SEQ ID NO: 118 - protein, 121 aa, Oryctolagus cuniculus
QSLEESGGDLVKPGASLTLTCKASGLDFSSVYDMCWVRQAPGKGLEWIACIYSDGSGSTYYANWAKGRFTISETSSTTVTLQMTNLTAADTATYFCARVLNGWGEYYFNLWGPGTLVTVSS

SEQ ID NO: 119 - protein, 112 aa, Oryctolagus cuniculus
QSVEESGGRLVTPGTPLTLTCTASGFSLSSYHMSWVRQAPGKGLEYIGFIVGTGDTYYASWAKGRFTISKTSTTVDLKITSPTTEDTATYFCGRGVAAGDIWGPGTLVTVSL

SEQ ID NO: 120 - protein, 113 aa, Oryctolagus cuniculus
QSLEESGGRLVTPGTPLTLTCTASGFSLSGLVVSWVRQAPGKGLEWIGVIGKSGSTYYASWAKGRFSISKTSSTTVDLKIASPTTEDTATYFCGRNISGSAVWGPGTLVTVSL

SEQ ID NO: 121 - protein, 119 aa, Oryctolagus cuniculus
QEQLVESGGGLVQPEGSLTLTCKASGFDFNRDAMSWVRQAPGKGLEWIGSIVSGSGSTYYASWAKGRFTISETSSTTVTLQMTSLTAADTATYFCARGGDGYGYVLVLWGPGTLVTVSS

SEQ ID NO: 122 - protein, 115 aa, Oryctolagus cuniculus
QSLEESGGDLVKPGASLKLSCAASGFTLSSYWICWVRQAPGKGLEWIACIYAGSSGSTYYASWAKGRFTISKTSSTTVTLQMTSLTAADTATYFCARGISYALLWGPGTLVTVSS

SEQ ID NO: 123 - protein, 116 aa, Oryctolagus cuniculus
QSVEESGGRLVTPGTPLTLTCTVSGIDLSRYAMIWVRQAPGKGLESIGIIDIRGTTYYASWAKGRFTISKTSSTTVDLKMTSLTTEDTATYFCARGGVGHEVNNLWGPGTLVTVSS

SEQ ID NO: 124 - protein, 121 aa, Oryctolagus cuniculus
QSLEESGGDLVKPGASLTLTCTASGFSFSNNYWICWVRQAPGKGLEWIACIVAGSSGRTYYANWAKGRFTISKTSSTTVTLQMTSLTAADTATYFCARKLSDWDYGYFNLWGPGTLVTVSS

SEQ ID NO: 125 - protein, 127 aa, Oryctolagus cuniculus
QSLEESGGDLVKPGASLTLTCTASGIDFSTYYYMCCVRQAPGKGLEWIACIHAGSSGSTYYASWAKGRFTISKTSSTTVTLQMTSLTAADTATYFCARGYAGYYGYGYPTPSWLDLWGQGTLVTVSS

SEQ ID NO: 126 - protein, 119 aa, Oryctolagus cuniculus
QSVEESGGRLVTPGTPLTLTCKASGFSLSSYWMSWVRQAPGEGLEWIGTINAASGATWYASWAKGRFTISKTSTTVDLKMTSLTTEDTATYFCARGGTTGSNYYGMDPWGPGTLVTVSS

SEQ ID NO: 127 - protein, 109 aa, Oryctolagus cuniculus
QSVEESGGRLVTPGTPLTLTCTVSGIDLSRNAASWVRQAPGKGLEWIGIISTGGSTYYATWAKGPFTISKTSTTVDLKMTSLTTEDTATYFCVVGIRFWGPGTLVTVSS

SEQ ID NO: 128 - protein, 122 aa, Oryctolagus cuniculus
QSVEESGGRLVTPGTPLTLTCTVSGFSLSNYAMTWVRQAPGKGLEWIGIIINTGYTYYASWAKGRFTISKASTTVDLKITSPTTEDTATYFCARVLGAGSSYYTSYDRLDLWGQGTLVTVSS

SEQ ID NO: 129 - protein, 116 aa, Oryctolagus cuniculus
QSLEESGGRLVTPGTPLTLTCTVSGIDLISNAISWVRQAPGKGLEWIGHSDIRGSAYYASWAKGRFTISRTSSTTVDLKMTSLTTEDTATYFCARIADVNTQLDLWGQGTLVTVSS

SEQ ID NO: 130 - protein, 120 aa, Oryctolagus cuniculus
QSLEESGGDLVKPGASLTLTCAASGFSFSVGYYMCWVRQAPGKGLEWVACIYAGSNGSTYYASWAKGRFTFSKPSSTTVTLQMTSLTAADTATYFCARGAGYAGYGFNLWGPGTLVTVSS

SEQ ID NO: 131 - protein, 125 aa, Oryctolagus cuniculus
QEQLVESGGGLVKPEGSLTLTCTASGFSFSSSYWICWVRQAPGKGLEWIACIYADGSGSIYCATWAKGRFTISKTSSTTVTLQMTSLTAADTATYFCSRGNAGSYWDIYYGMDLWGPGTLVTVSS

SEQ ID NO: 132 - protein, 118 aa, Oryctolagus cuniculus
QSLEESGGDLVKPGASLTLTCTASGFSFSSSYYMCWVRQAPGKGLEWIACIYIGDGNTYYASWAKGRFTISKTSSTTVTLQMTSLTAADTATYFCARGSGGYFVDNLWGPGTLVTVSS

SEQ ID NO: 133 - protein, 118 aa, Oryctolagus cuniculus
QSVEESGGRLVTPGTPLTLTCTASGFDINNYHMTWVRQAPGKGLEWIGFIKAGGSAGYASWAKGRFTISKTSATVDLRITGATTEDTGTYFCVRMFYAGDSGHYFDLWGPGTLVTVSS

SEQ ID NO: 134 - protein, 118 aa, Oryctolagus cuniculus
QSVEESGGRLVTPGTPLTLTCTVSGFSLSSYDMTWVRQAPGKGLEWIGVISSSDSTYYASWAKGRFTISKPSSTTVDLKVTSPTTEDTATYFCARDHPAFSTVDLDIWGPGTLVTVSL

SEQ ID NO: 135 - protein, 121 aa, Oryctolagus cuniculus
QEQLVESGGGLVKSGASLTLTCTASGFSLSSSYCVCWVRQAPGKGLEWIACIYGGSSGGTYYASWAKGRITISKTSSTTVTLQMTSLTAADTATYFCARDAGSSGYYINLWGPGTLVTVSS

SEQ ID NO: 136 - protein, 118 aa, Oryctolagus cuniculus
QSLEESGGDLVKPGASLTLTCTASGFSFSSNAMCWVRQAPGKGPEWIGCIYTSSSGSTYYASWVNGRFTISKTSSTTVTLQMTSLTVADTATYFCARYNNGWDYFNLWGPGTLVTVSS

SEQ ID NO: 137 - protein, 121 aa, Oryctolagus cuniculus
QEQLVESGGGLVKPGASLTLTCTASGFSFNGNYYMCWVRQAPGKGLEWIACIYADNSGSTYYASWAKGRFTISKTSSTTVTLQMTSLTAADPATYFCVRHKPAGGSSYILWGPGTLVTVSS

SEQ ID NO: 138 - protein, 112 aa, Oryctolagus cuniculus
QSLEESGGRLVTPGTPLTLTCTVSGIDLSSYHMNWVRQAPGKGLEWIGVIYGSGSTDYASWAKGRFTISKTSTTVDLKITSPTTEDTATYFCARGILVSNLWGPGTLVTVSS

SEQ ID NO: 139 - protein, 116 aa, Oryctolagus cuniculus
QSLEESGGDLVKPGASLTLTCTASGFTISSSYYMCWVRQAPGKGLEWIACIYSDSSGSTYNANWVKGRFTISKTSSTTVTLRMTSLTAADTATYFCARGTYPFTLWGPGTLVTVSS

SEQ ID NO: 140 - protein, 118 aa, Oryctolagus cuniculus
QSVEESGGRLVTPGTPLTLTCTVSGFSLSSYPVNWVRQAPGKGLEWIGVIGNRGSTDYASWAKGRFTISKTSTTVDLKITSPTTEDTATYFCARGSGYGTGWDAFDPWGPGTLVTVSS

SEQ ID NO: 141 - protein, 114 aa, Oryctolagus cuniculus
QSLKESGGGLVTPGTPLTLTCKVSGFSLSSYDMSWVRQAPGKGLEWIGTIYDGGSTYYASWTKGRFTISKASTTVDLKITSPTTEDTATYFCARGSTNMEFWFWGPGTLVSVSS

SEQ ID NO: 142 - protein, 119 aa, Oryctolagus cuniculus
QSVEESGGRLVTPGTPLTLTCTVSGFSLNNYGMTWVRQAPGKGLEWIGIINIIDNTYYASWAKGRFTISKTSTTVDLKITSPTTEDTATYFCARADYYPDTTGWYLNIWGPGTLVTVSL

SEQ ID NO: 143 - protein, 113 aa, Oryctolagus cuniculus
QSVEESGGRLVTPGTPLTLTCTVSGFSLSTYWMSWVRQAPGKGLEWIGTISTGGSAYYASWAKSRFTISKTSTTVDLKITSPTTEDTATYFCARDGDSYFKLWGPGTLVTVSS

SEQ ID NO: 144 - protein, 115 aa, Oryctolagus cuniculus
QSLEESGGRLVTPGTPLTLTCTVSGIDLSSYAMGWVRQAPGKGLEYIGYINRGNTYYANWAKGRFTISKTSTTVDLKITSPTTEDTATYFCARDSYGGDYAFNLWGPGTLVTVSS

SEQ ID NO: 145 - protein, 121 aa, Oryctolagus cuniculus
QSLEESGGGLVKPGASLTLTCTASGFSFSSSYYMCWVRQAPGKGLEWIACIHAGSSGSAYYASWAKGRFTISKTSSTTVTLQMTSLTAADTATYFCARDGYDDYGDPFNLWGPGTLVTVSS

SEQ ID NO: 146 - protein, 126 aa, Oryctolagus cuniculus
QSLEESGGDLVKPGASLTLTCTASGFSFSSGQDMCWVRQAPGKGLEWIACIYGGDGNTYYASWAKGRFTIYKTSSTTVTLKMTSPTAADTATYLCARLHYSPYGDAGYPYVSFNLWGPGTLVTVSS

SEQ ID NO: 147 - protein, 114 aa, Oryctolagus cuniculus
QSVEESGGRLVTPGTPLTLTCTASGFSLSSYNMGWVRQAPGKGLEWIGYIWSGGSAYYASWAKGRFTISRTSTTVTLKMTSLTAADTATYFCARNGASGTFDIWGPGTLVTVSL

SEQ ID NO: 148 - protein, 121 aa, Oryctolagus cuniculus
QEQLVESGGGLVQPEGSLTLTCTASGFSFSSSYYMCWVRQAPGKGLEWIACIYAGSSGSTYYASWAKGRLTISKISSTTVTLQMTSLTAADTATYFCARGGGSGGVDNNLWGPGTLVTVSS

SEQ ID NO: 149 - protein, 113 aa, Oryctolagus cuniculus
AQVLTQTPSSVSAAVGGTVTINCQASQSLYNNKNLAWYQQKLGQPPKLLIYDVSTLASGVPSRFKGSGSGTQFTLTISGVQCDDAATYYCQGEFSCSSGDCYAFGGGTEVVVK

SEQ ID NO: 150 - protein, 110 aa, Oryctolagus cuniculus
AQVLTQTASSVSAVVGGTVTISCQSSQSVYDKKWLGWYQQKPGQPPKLLIYKASTLASGVPSRFKGSGSGTQFTLTISDLECDDAATYYCAGGYSGNIWSFGGGTEVVVK

SEQ ID NO: 151 - protein, 113 aa, Oryctolagus cuniculus
AQVLTQTPSSVSAAVGGTVTIICQASQSLYNNKNLAWYQQKLGQPPKLLIYDVSTLASGAPSRFKSSGSGKQFTLTISGVQCDDAATYYCQGEFSCSSGDCYAFGGGTEVVVK

SEQ ID NO: 152 - protein, 110 aa, Oryctolagus cuniculus
AQVLTQTASPVSAAVGDTVTISCQSSESVYNNNLLSWYQQKPGQPPKLLIYTTSSLASGVPSRFKGSGSGTQFTLTISGVQCDDAATVYCQGGYTDATYAFGGGTEVVVK

SEQ ID NO: 153 - protein, 104 aa, Oryctolagus cuniculus
DIVMTQTPSSVSAAVGGTVTINCQASQSVSNLLAWYQQKPGQPPKLLIYGASNLESGVPSRFRGSGSGTEFTLTISGMKAEDAATYYCQSGYYTFGAGTKVEIK

SEQ ID NO: 154 - protein, 113 aa, Oryctolagus cuniculus
AQVLTQTPSSVSAAVGGTVTINCQASQSLYNNKNLAWYQQKPGQPPKLLIYDASTLASGVPSRFKGSGSGTQFTLTISGVQCDDAATYYCQGEFSCGSGDCYAFGGGTEVVVK

SEQ ID NO: 155 - protein, 110 aa, Oryctolagus cuniculus
DPVLTQTPSSASEPVGGTVTIKCQASEDIESYLAWYQQKPGQPPKLLIYDASDLASGVPSRFKGSGSGTQFTLTISGVQCADAATYYCQSYYYGSSYVVAFGGGTEVVVK

SEQ ID NO: 156 - protein, 113 aa, Oryctolagus cuniculus
AQVLTQTPSSVSAAVGGTVTINCQASQSLYNNKNLGWYQQKLGQPPKLLIYDVSTLASGVPSRFKGSGSGTQFTLTISDLECDDAATYYCQGEFSCSSGDCYAFGGGTEVVVK

SEQ ID NO: 157 - protein, 111 aa, Oryctolagus cuniculus
DIVMTQTPASVEAAVGGSVTIKCQASQTISSYLAWYQQKPGQPPKLLIYGASTLASGVPSRFSGSGSGTEYTLTISGVQCDDAATYYCLYSYYTSNSADNTFGGGTEVVVK

SEQ ID NO: 158 - protein, 111 aa, Oryctolagus cuniculus
AAVLTQTPSPVSAAVGGTVSISCQSSQSVYDNNALAWYQQKPGQPPKLLIYETSTLASGVPSRFEGSGSGTQFTLTISDVQCDDAATYYCAGGYNSGSDAAFGGGTEVVVK

SEQ ID NO: 159 - protein, 110 aa, Oryctolagus cuniculus
AQVLTQTPSPVSAPVGGTVTISCQSSQNVDRNNRLAWYQQKLGQPPKLLIYYASILASGVPSRFKGSGSGTQFTLTINELQCDDAATYYCQGYYSGDINVFGVGTEVVVK

SEQ ID NO: 160 - protein, 111 aa, Oryctolagus cuniculus
DIVMTQTPASVEAAVGGTVTIKCQASQSIGSNLAWYQQKPGQPPKLLIYKASTLASGVPSRFKGSGSGTEFTLTISDLECADAATYYCQSYYGTSNSYGDAFGGGTEVVVK

SEQ ID NO: 161 - protein, 111 aa, Oryctolagus cuniculus
DVVMTQTPASVSEPVGGTVTIKCQASEDIESYLAWYQQKPGQPPKLLIYQASKLASGVSSRFSGSGYGTEFTLTLSDLECADAATYYCQCTLYGVNFVPNVFGGGTEVVVK

SEQ ID NO: 162 - protein, 111 aa, Oryctolagus cuniculus
DVVMTQTPASVSEPVGGTVTIKCQASEDIESYLAWYQQKPGQPPKLLIYSASTLASGVSSRFKGSGSGTEFTLTISDLECADAATYYCQCILYGVNFVPNTFGGGTEVVVK

SEQ ID NO: 163 - protein, 111 aa, Oryctolagus cuniculus
DVVMTQTPASVSAAVGGTVTIKCQASQNIYDNLAWYQQKPGQRPKLLIYGASNLESGVPSRFKGSGSGTEYTLTISDLECADAATYYCQCSYDGGSYVPNAFGGGTEVVVQ

SEQ ID NO: 164 - protein, 111 aa, Oryctolagus cuniculus
AAVLTQTPSPVSAAVGGTVSISCQSSPSVYNNNRLSWFQQKPGQPPKLLIYYASTLASGVPSRFKGSGSGTQFTLTISDVQCDDAATYYCAGGYSTISDNAFGGGTEVVVK

SEQ ID NO: 165 - protein, 110 aa, Oryctolagus cuniculus
DVVMTQTPASVSEPVGGTVTIKCQASQNIGNNLAWYQQKPGQPPKLLIDYASTLASGVPSRFKGSGSGTQFTLAISDLDCADAATYYCQCTFYGSGYVAAFGGGTEVVVK

SEQ ID NO: 166 - protein, 111 aa, Oryctolagus cuniculus
DVVMTQTPASVSEPVGGTVSINCQASEDIESYLAWYQQKPGQPPKLLIYGASNLASGVSSRFKGSGSGTEYTLTISDLECDDAATYYCQCGIYGVNFVPNVFGGGTEVVVK

SEQ ID NO: 167 - protein, 110 aa, Oryctolagus cuniculus
AYDMTQTPASVEVGVGGTVTIKCQASQNINSWLSWYQQKPGQPPKLLIYKASTLASGVSSRFKGSGSGTEFTLTISDLECADAATYYCQQGAGWNNLDNAFGGGTEVVVK

SEQ ID NO: 168 - protein, 111 aa, Oryctolagus cuniculus
AQVLTQTPSSVSAAVGGTVTINCQSSQSVYSNNHLAWYQQKPGQPPNLLIYRASKLASGVPSRFSGSRSGTQFTLTISGVQCDDAATYYCLGVYDDDADNAFGGGTEVVVK

SEQ ID NO: 169 - protein, 112 aa, Oryctolagus cuniculus
AVVMTQTASPVSAAVGGTVTINCQSSQIVHNNNNLAWYQLKPGQPPKLLIFQASTLASGVPSRFKGSGSGTQFTLTISDLECDDAAAYYCAGGYSTNTDTYIFGGGTEVVVR

SEQ ID NO: 170 - protein, 113 aa, Oryctolagus cuniculus
AQVLTQTPSSVSAAVGGTVTINCQASQSLYNKKNLAWYQQKLGQPPKLLIYDASTLTSGVSSRFKGSGSGTQFTLTISGVQCDDAATYYCQGEFSCSAGDCYAFGGGTELVVK

SEQ ID NO: 171 - protein, 110 aa, Oryctolagus cuniculus
AQVLTQTASSVSAVVGGTVTISCQSSQSVYDNKWLGWYQQKPGQPPKLLIYSASTLASGVPSRFKGSGSGTHFTLTISDLECDDATTYYCAGGYSGNIWSFGGGTEVVVK

SEQ ID NO: 172 - protein, 110 aa, Oryctolagus cuniculus
AQVLTQTPSPVSAAVGGTVTISCQSSQSVYDNKWLGWYQQKPGQPPKLLIYKASTLASGVPSRFKGSGSGTQFTLTISDLECDDATTYYCAGGYSGNIWSFGGGTEVVVK

SEQ ID NO: 173 - protein, 111 aa, Oryctolagus cuniculus
AAVLTQTPASVSAAVGGTVTISCQSSKSVFDNNWLSWFQQKPGQPPKLLIYKASTLASGVPSRFKGSGSGTQFTLTISDVQCDDAATYYCAGIYSSDSDNAFGGGTEVVVK

SEQ ID NO: 174 - protein, 113 aa, Oryctolagus cuniculus
AQVLTQTPSSVSAVVGGTVTINCQASQSLYNKKNLAWYQQKLGQPPKLLIYDASTLASGVPSRFKGSGSGTQFTLTISGVQCDDAASYYCQGEFSCSSGDCYAFGGGTELVVK

SEQ ID NO: 175 - protein, 110 aa, Oryctolagus cuniculus
AYDMTQTPFSVSAAVGGTVTINCQASETIYSYLNWYQQKPGQPPKLLIYSASTLASGVPSRFKGSGSGTQFTLTISGVECADAATYYCQQGYSGRNVENTFGGGTEVVVK

SEQ ID NO: 176 - protein, 111 aa, Oryctolagus cuniculus
AAVLTQTPSPVSAAVGGTVTISCQSSQNIYNKNQLSWFQQKPGQPPKLLIYEASKLASGVPSRFKGSGSGTQFTLTISDVQCDDAATYYCLGGYISSSDTTFGGGTEVVVK

SEQ ID NO: 177 - protein, 110 aa, Oryctolagus cuniculus
DVVMTQTPASVSTAVGGTVTIKCQASQSIGGSLAWYQQKPGQPPNLLIYSASNLASGVSSRFKGSRSGTEFTLTISDLECADAATYYCQCTYYDDSYDVPFGGGTEVVVK

SEQ ID NO: 178 - protein, 112 aa, Oryctolagus cuniculus
AAVLTQTPSPVSAAVGGTVTISCQSSQSVNNNKNLAWYQQKLGQPPKLLIYDTSTLASGVPSRFKGSGSGTQFTLTISDLECDDATTYYCAGGYSSSADTFAFGGGTEVVVR

SEQ ID NO: 179 - protein, 112 aa, Oryctolagus cuniculus
DIVMTQTPASVSAAVGGTVTIKCQASQNIGSTLAWYQQKPGQPPKRLIYGASTLSSGVPSRFKGSGSGTDFTLTISDLECADAATYYCQSNYGSNSGGYVFPFGGGTEVVVK

SEQ ID NO: 180 - protein, 111 aa, Oryctolagus cuniculus
DVVMTQTPASVSEPVGGTVTIKCQASEDIETYLAWYQQKPGQPPKLLIYRASTLASGVPSRFKGSGSGTQFTLTISDLECADAATYYCQCTLYGVNFVANAFGGGTEVVVK

SEQ ID NO: 181 - protein, 109 aa, Oryctolagus cuniculus
AFELTQTPSSVSAAVGGTVTINCQASEDIENYLAWYQQKPGQPPKLLIYSASTLASGVSSRFKGSGSGTEYTLTISDLGCADAATYYCQSYYDGAVTFTFGGGTEVVVK

SEQ ID NO: 182 - protein, 112 aa, Oryctolagus cuniculus
AQVLTQTASPVSAAVGGTVTIKCQSSQSVDNNWLSWYQQKPGQPPKLLIYTTSKLASGVPSRFKGSGSGTQFTLTISDVQCDDAATYYCLGGYDSMSADCFAFGGGTEVVVK

SEQ ID NO: 183 - protein, 111 aa, Oryctolagus cuniculus
AQVLTQTPSSVSAAVGGAVTINCQSSQSVYSNNHLAWYQQKPGQPPKLLIYRASKLASGVPSRFSGSGSGTQFTLTISGVQCDDAATYFCLGVYDDDADNAFGGGTAVVVK

SEQ ID NO: 184 - protein, 112 aa, Oryctolagus cuniculus
AVVMTQTASPVSAAVGGTVTINCQSSQSVHNNNNLAWYQQKPGQPPKLLIFQASTLASGVPSRFKGSGSGTQFTLTISDLECDDAAAYYCAGGYSTNTDTFTFGGGTEVVVR

SEQ ID NO: 185 - protein, 112 aa, Oryctolagus cuniculus
ALVMTQTPASVEAAVGGTVTISCQASEDISSSLAWYQQKPGQPPNLLIYRASNLASGVPSRFKGSGSGTQFTLTISGVQCADAATYYCQAYYYSISDDLYNAFGGGTEVVVK

SEQ ID NO: 186 - protein, 112 aa, Oryctolagus cuniculus
AVVMTQTASPVSAAVGGTVTISCQASQSVHNNNNLAWYQQKPGQPPKLLIFQASTLASGVPSRFKGSGSGTEFTLTISDLECDDAAAYYCAGGYSTNTDTFTFGGGTEVVVR

SEQ ID NO: 187 - protein, 111 aa, Oryctolagus cuniculus
DVVMTQTPASVSAAVGGTVTIKCQASEDIESYLAWYQQKPGQPPKLLIYRASTLASGVPSRFKGSGSGTQFTLTISDLECADAATYYCQCTIYGVNFVPNAFGGGTEVVVK

SEQ ID NO: 188 - protein, 111 aa, Oryctolagus cuniculus
DVVMTQTPASVSAAVGGTVTIKCQATEDIESFLAWYQQKPGQPPKLLIYRASTLESGVPSRFKGSGSGTEFTLTISDLECADAATYYCQCTVYGVNFVANAFGGGTEVVVR

SEQ ID NO: 189 - protein, 108 aa, Oryctolagus cuniculus
AIKMTQTPSSVSAAVGGTVTINCRASEDIKSYLAWYQQKPGQPPKLLIYDASDLASGVPSRFKGSGSGTEYTLTISGVQCDDAATYYCQSVWYAGGAAFGGGTEVVVQ

SEQ ID NO: 190 - protein, 113 aa, Oryctolagus cuniculus
AQVLTQTASPVSAAVGGTVTINCQASQSVYNHKNLAWYQQKPGQPPKLLIYDTSTLASGVSSRFKGSGSGTQFTLTISGVQCDDAATYYCAGEFSCASADCFAFGGGTEVVVK

SEQ ID NO: 191 - protein, 110 aa, Oryctolagus cuniculus
DVVMTQTPASVSEPVGGTVTIKCQASQSIGSSLAWYQQKAGQRPKLLIYYVSNLESGVSSRFSGSGSGTEFTLTISGVQCDDAATYYCQSYGYGSGYVFAFGGGTEVVVK

SEQ ID NO: 192 - protein, 113 aa, Oryctolagus cuniculus
AQVLTQTPSPVSAAVGGTVSISCQSSQSVYGVNELSWYQQKAGQPPKLLIYKAATLASGVPSRFKGSGSGTQFTLTISDVQCDDAATYYCLGNYDCESDDCYAFGGGTEVVVK

SEQ ID NO: 193 - protein, 113 aa, Oryctolagus cuniculus
DVVMTQTPASVEAPVGGTVTIKCQASQSISNLLAWYQQIPGQSPKLLIYDASDLASGVPSRFKGSGSGTEYTLTISDLECADAATYYCQCTYGSSSSSAYGWAFGGGTEVVVK

SEQ ID NO: 194 - protein, 111 aa, Oryctolagus cuniculus
AAVLTQTPSPVSAAVGGTVSISCQSSKSVYNNNWLSWFQQKPGQPPKLLIYGASTLASGVPSRFKGSGSGTQFTLTISDVQCDDAATYYCLGSYISSSDNAFGGGTEVVVK

SEQ ID NO: 195 - protein, 111 aa, Oryctolagus cuniculus
AAVLTQTPSPVSAAVGGTVSISCQSSPSVYNNNRLSWFQQKPGQPPKLLIYYASTLASGVPSRFKGSGSGTQFTLTISDVQCDDAATYYCAGGYSSISDNGFGRGTEVVVK

SEQ ID NO: 196 - protein, 112 aa, Oryctolagus cuniculus
DVVMTQTLPSVSEPVGGTVTIKCQASQSIGSYLSWYQQKPGQPPKLLIYDASTLASGVPSRFKGGGSGTQFTLTISDLECADAATYYCQGYYYYISNTYGYPFGGGTEVVVK

SEQ ID NO: 197 - protein, 110 aa, Oryctolagus cuniculus
DVVMTQTPASVSEPVGGTVTIKCQASQNIGNNLAWYQQKPGQPPKLLMYDASDLASRVPSRFSGSGSGTEFTLTISDLECADAATYYCQCTYGYSGYVSAFGGGTEVVVK

SEQ ID NO: 198 - protein, 110 aa, Oryctolagus cuniculus
ALVMTQTPSPVSAAVGGTVTINCQASEDIYSNLAWFQQKPGQPPKLLIYSASTLASGVSSRFKGSGSGTKFTLTISGLQCDDAATYYCLGVYTYISADNAFGGGTEVVVK

SEQ ID NO: 199 - protein, 113 aa, Oryctolagus cuniculus
AQVLTQTPSSVSAAVGGTVTINCQASQSLYNNKNLAWYQQKLGQPPKLLIYDVSTLASGVPSRFKGSGSGKQFTLTISGVQCDDAATYYCQGEFSCSSGDCYAFGGGTEVVVK

SEQ ID NO: 200 - protein, 111 aa, Oryctolagus cuniculus
AAVLTQTPSPVSAAVGGTVSISCQSSKTVYNNNWLAWFQQKPGQPPKLLIYGASTLASGVPSRFKGSGSGTQFTLTISDVQCDDAATYYCLGSYISSSDNGFGGGTEVVVK

SEQ ID NO: 201 - protein, 111 aa, Oryctolagus cuniculus
AAVLTQTPSPVSAAVGGTVTISCQSSPSVYNNVRLSWFQQKPGQPPKLLIYSASTLASGVPSRFKGSGSGTQFTLTISDVQCDDAATYYCAGGYSDISDNAFGGGTEVVVK

SEQ ID NO: 202 - protein, 112 aa, Oryctolagus cuniculus
AQVLTQTPSSVSAAVGGTVTISCQSSQSVYSTNLAWYQQKPGQPPKLLIDYASTLASGVPSRFKGSGSGTQFTLTISGVQCDDAAAYYCQGEFNCGSGDCSTFGGGTEVVVK

SEQ ID NO: 203 - protein, 110 aa, Oryctolagus cuniculus
DVVMTQTPASASAAVGGTVTINCQASENIANHLAWYQQKPGQPPKLLIYSASALASGVPSRFKGSGSGTEFALTISDLECDDAAIYYCQCTFWDINNFGGFGGGTEVVVK

SEQ ID NO: 204 - protein, 111 aa, Oryctolagus cuniculus
AAVLTQTPSPVSAAVGGTVTIKCQSSQSVYGNNELSWYQQKPGQPPKLLIYDASKLASGVPHRFSGSGSGTQFTLTISGVQCDDAATYYCLGGYDADADNAFGGGTEVVVK

SEQ ID NO: 205 - protein, 113 aa, Oryctolagus cuniculus
AQVLTQTPSSVSAAVGGTVTINCQASQSLYNKKNLAWYQQKLGQPPKLLIYDVSTLASGVPSRFKGSGSGTQFTLTISDLECGDAAAYFCQGEFSCSSGDCYAFGGGTEVVVK

SEQ ID NO: 206 - protein, 110 aa, Oryctolagus cuniculus
AQVLTQTASSVSAAVGGSVTISCQSSQSVYGSDALAWFQQRPGQSPKRLIYGASTLASGISSRFKGSGSGTQFTLTISDLECDDAATYFCAGAYSGNVGTFGGGTEVVVK

SEQ ID NO: 207 - protein, 110 aa, Oryctolagus cuniculus
AYDMTQTPASVEVAVGGTVTIKCQASQSISSNLAWYQQKSGQPPKLLIYLASTLASGVPSRFKGSGSGTEFTLTISDLECADAATYYCQQTYSGSNVENSFGGGTEVVVK

SEQ ID NO: 208 - protein, 111 aa, Oryctolagus cuniculus
AIDMTQTPSPVSAAVGDTVTINCQASENIYSFLAWYQQKPGHSPKLLIYSASTLESGVPSRFKGSGSGTQFTLTISDVQCDDAATYYCQQTYIYNNAEDNTFGGGTEVVVK

SEQ ID NO: 209 - protein, 112 aa, Oryctolagus cuniculus
DVVMTQTPASVEAAVGGTVTIKCQASQSISDYLSWYQQKPGQPPKLLIYRASNLASGVPSRFKASESGTEFTLTISDLECADAATYYCQCTFGATNDDYGNAFGGGTEVVVK

SEQ ID NO: 210 - protein, 113 aa, Oryctolagus cuniculus
DIVMTQTPASVEAAVGGTVTIKCQASQSISSYLSWYQQKPGQPPKLLIYDASDLASGVSSRFKGSGSGTEFTLTISDLECADAATYYCQCTVGSSGVTGYGNAFGGGTEVVVK

SEQ ID NO: 211 - protein, 112 aa, Oryctolagus cuniculus
DPVMTQTPASVSEPVGGTVTIKCQASQNINNLLAWYQQKPGQPPKLLIYKASTLASGVSSRFKGSGSGTEFTLTISDLECADAATYYCQNYYGYGLSTNYVVFGGGTEVVVK

SEQ ID NO: 212 - protein, 113 aa, Oryctolagus cuniculus
AQVLTQTPSSVSAAVGGTVTINCQASQSVYANNYLAWYQQKPGQPPKLLIYKASTLASGVPSRFSGSGSGTQFTLTINGVQCDDAATYYCQGEFSCSSGDCTAFGGGTEVVVK

SEQ ID NO: 213 - protein, 112 aa, Oryctolagus cuniculus
DVVMTQTPASVEAAVGGTVTIKCQASESISNYLSWYQQKPGQPPKLLICYDSTLESGVPSRFKGSGSGTDFTLTISDLECADAATYYCQCTAGSINVSYGNAFGGGTEVVVK

SEQ ID NO: 214 - protein, 113 aa, Oryctolagus cuniculus
AQVLTQTASPVSEPVGGTVTIKCQSSQSVYNNNWLSWFQQKPGQPPKRLIYGASTLASGVPSRFKGSGSGTHFTLTISDVQCDDAATYYCLGSYDCSSVDCNAFGGGTEVVVK

SEQ ID NO: 215 - protein, 112 aa, Oryctolagus cuniculus
AAVLTQTPSPVSAAVGGTVTISCQASQSVHKHKNLAWYQQKPGQPPKLLIYEASKLASGVPPRFSGSGSGTQFTLTMSDLECDDAATYYCAGGYDSTIDTFTFGGGTEVVVK

SEQ ID NO: 216 - protein, 113 aa, Oryctolagus cuniculus
DVVMTQTPASVEAAVGGTVTIKCQASQSISSYLSWYQQKPGQPPKLLIYRASSLKSGVPSRFKGTGSGTEFTLTISDLECADAATYYCQCTYGSSTSSRSGNAFGGGTEVVVT

SEQ ID NO: 217 - protein, 113 aa, Oryctolagus cuniculus
DIVMTQTPASVEAAVGGTVTIKCQASQNINNELSWYQQKPGQPPKLLIYKASTLASGVPSRFKGSGSGTQFTLTISDLECADAATYYCQSYYYGISSTYAFYTFGGGTEVVVK

SEQ ID NO: 218 - protein, 110 aa, Oryctolagus cuniculus
DVVMTQTPASASAAVGGAVTIKCRASEDIESYLAWYQQKPGQPPKLLIYSASSLASGVPSRFKGSGSGTEFTLTISDLECDDAATYYCQCTYWDSSTVGAFGGGTAVVVK

SEQ ID NO: 219 - protein, 111 aa, Oryctolagus cuniculus
AAVLTQTPSPVSAAVGGTVSISCQSSQSVYNDNDLAWFQQKPGQPPKLLIYGASTLASGVPSRFKGSGSGTQFTLTISGVQCDDAATYYCSGGYISSSDNAFGGGTEVVVK

SEQ ID NO: 220 - protein, 109 aa, Oryctolagus cuniculus
DVVMTQTPASVSAAVGGTVTIKCQASESIYSGLAWYQQKPGQPPKLLIYRASTLESGVSSRFKGSGSGTQFTLTISDLECADAATYYCQSTYYGSSGNAFGGGTEVVVK

SEQ ID NO: 221 - protein, 111 aa, Oryctolagus cuniculus
DIVMTQTPASVSAAVGGTVTINCQASQSISYYLNWYQQKPGQPPKLLIYRASTLASGVPSRFSGSGSGTQFTLTISGVQCDDAATYYCLYGYVTSSNADFAFGGGTEVVVE

SEQ ID NO: 222 - protein, 113 aa, Oryctolagus cuniculus
AQVLTQTPSSVSAAVGDTVTINCQASQSVYKNNYLAWFQQKPGQPPKRLIYSASTLDSGVSSRFKGSGSGTQFTLTISDVQCDDAATYYCLGTYDCVSADCGAFGGGTEVVVK

SEQ ID NO: 223 - protein, 112 aa, Oryctolagus cuniculus
AQVLTQTASSVSAAVGGTVTISCQSSQSVYNNNWLGWYQQKPGQPPKLLIYSASTLASGVPSRFKGSGSGTQFTLTISGVQCYDAATYYCQGTYSNNGWYFAFGGGTEVVVK

SEQ ID NO: 224 - protein, 113 aa, Oryctolagus cuniculus
DIVMTQTPASVSEPVGGTVTIKCQASEDIYNLLAWYHQKPGQPPKLLIYGASTLASGVPSRFKGSGSGTQFTLTISDLECADAATYYCQSYYYGISSTYAFYTFGGGTEVVVE

SEQ ID NO: 225 - protein, 109 aa, Oryctolagus cuniculus
AFELTQTPSSVSAAVGGTVTINCQASEDIESYLAWYQQKPGQPPKFLIYGASTLASGVPSRFKGSGSGTEYTLTISDLECADAATYYCQTYYGGINIFTFGGGTEVVVE

SEQ ID NO: 226 - protein, 113 aa, Oryctolagus cuniculus
AQVLTQTASPVSAAVGSTVTINCQASQSVYSNNYLSWFQQKPGQPPKLLIYDASDLASGVPSRFKGSGSGTQFTLTISDLECDDAATYYCLGTYDCSSTDCYAFGGGTEVVVK

SEQ ID NO: 227 - protein, 111 aa, Oryctolagus cuniculus
DVVMTQTPASVSEPVGGTVSLKCQASESIDSYLNWYQQKPGQPPKLLIYGASTLASGVSSRFKGSRSGTEYTLTISDLECADAATYYCQCTVYGVNFVPNAFGGGTEVVVK

SEQ ID NO: 228 - protein, 110 aa, Oryctolagus cuniculus
ALVMTQTPSSVSAAVGGTVTINCQASQNIYSSLAWYQQKPGQPPKLLIYGASNLESGVPSRFKGSGSGTEFTLTISALECDDAATYYCQGGYYISSTDNAFGGGTEVVVK

SEQ ID NO: 229 - protein, 110 aa, Oryctolagus cuniculus
AYDMTQTPASVEAVVGGSVTIKCQASQSISYYLAWYQQKPGQRPKLLIYRASTLASGVPSRFKGSGSGTEYTLTISDLECADAATYYCQQGYSSSNVDNAFGGGTEVVVK

SEQ ID NO: 230 - protein, 110 aa, Oryctolagus cuniculus
AFELTQTPSSVSAAVGGTVTIKCQASQNIYSRLAWYQQKPGQRPKLLIYAASTLASGVPSRFKGNGSGTEFTLTISDLECADAATYYCQGGYYGSSDTVTFGGGTEVVVK

SEQ ID NO: 231 - protein, 111 aa, Oryctolagus cuniculus
AAVLTQTPSPVSAAVGGTVTISCQSSQSVTDNFLSWFQQKPGQRPKLLIYGASTLASGVPSRFKGSGSGTQFTLTISDVQCDDAATYYCAGGYSGSSDVFAFGGGTEVVVK

SEQ ID NO: 232 - protein, 111 aa, Oryctolagus cuniculus
AYDMTQTPSSVSAAVGGTVTINCQASEDIESYLAWYQQKPGQPPKLLIYSASTLASGVPSRFKGSGSGTQFTLTISDLECADAATYYCQCTVYGVNYVPNAFGGGTEVVVK

SEQ ID NO: 233 - protein, 110 aa, Oryctolagus cuniculus
DVVMTQTPASVSAAVGGTVTIKCQASQSIGSSLAWYQQKPGQSPKLLIYSASNLASGVSSRFKGSGSGTEYTLTISDLECADAATYYCQCTYYGGSGDVPFGGGTEVVVK

SEQ ID NO: 234 - protein, 112 aa, Oryctolagus cuniculus
DIVMTQTPASVEAAVGGTVTIKCQASQSISSYLAWYQQKPGQPPKLLIYRTSILESGVPSRFKGSGSGTEFTLTISDLECADAATYYCQCTYGTTNTGHYVGFGGGTEVVVK

SEQ ID NO: 235 - protein, 109 aa, Oryctolagus cuniculus
DVVMTQTPASVSEPVGGTVTIKCQASQNIGSDLAWYQQKPGQRPKLLIYDASALASGVPSRFSGSGSGTEFTLTISGVQCDDSATYYCQCTYYSGSPHTFGGGTEVVVK

SEQ ID NO: 236 - protein, 114 aa, Oryctolagus cuniculus
DIVMTQTPASVEAAVGGTVTIKCQASQSISSYLAWYQQKPGQPPKLLIYRASTLASGVPSRFKGSGSGTEFTLTISDLECADAATYYCQSNYGSSSISNYGGGAFGGGTEVVVK

SEQ ID NO: 237 - protein, 110 aa, Oryctolagus cuniculus
AQVLTQTPASVSAAVRGTVTIKCQASESVVGKNELSWYHQKPGQPPKLLIFGTSTLASGVPSRFSGSGSETQFTLAISDLECGDAATYYCAGGYSGNMYVFGGGTEVVVK

SEQ ID NO: 238 - protein, 112 aa, Oryctolagus cuniculus
AAVLTQTPSPVSAAVGGTVTISCQASQSVHNNKNLAWYQQKPGQPPKLLIYDVSTVASGVPSRFKGSGSGTQFTLTISDLECDDAATYYCAGGYGSYTDTFAFGGGTEVVVK

SEQ ID NO: 239 - protein, 111 aa, Oryctolagus cuniculus
AAVLTQTPSPVSAAVGGTVTIKCQSSQSVYRNNELSWYQQKPGQPPKVLVYDASNLASGVPDRFSGSGSGTQFTLTISGVQCDDAATYYCLGGYDDDADNTFGGGTEVVVK

SEQ ID NO: 240 - protein, 111 aa, Oryctolagus cuniculus
DVVMTQTPASVSEPVGGTVTIKCQASEDIESFLAWYQQKPGQPPKLLIYSASTLASGVPSRFKGSGSGTQFTLTIGDLECADAATYFCQCTIYGVNFVPNAFGGGTEVVVK

SEQ ID NO: 241 - protein, 110 aa, Oryctolagus cuniculus
DVVMTQTPASVSEPVGGTVTIKCQASEDISSRLAWYQQKPGQPPKLLIYRASTLASGVPSRFKGSGSGPEYTLTISDLECADAATYYCQSNYAIISCGAAFGGGTEVVVK

SEQ ID NO: 242 - protein, 110 aa, Oryctolagus cuniculus
ALVMTQTPSSVSAAVGGTVTINCQASQNIYSNLAWYQQKPGQRPKLLIYGASNLESGVPSRFKGSGSGTEFTLTISDLECDDAATYYCQSAYYSSSAVYAFGGGTEVVVK

SEQ ID NO: 243 - protein, 111 aa, Oryctolagus cuniculus
AIDMTQTPSSVSAAVGDTVTINCQASENIYSFLAWYQQKPGQRPKLLIYDSSTLASGVPSRFSGSGSGTEFTLTISGIQCDDAATYYCQQTYIYNNAESNAFGGGTEVVVK

SEQ ID NO: 244 - protein, 110 aa, Oryctolagus cuniculus
AQVLTQTPSPVSAAVGGTVTINCQSSQSVADNNLLAWYQQKPGQPPKLLIYKASTLASGVPSRFKGSGYGTQFTLTISDLECDDAATYYCVGGYSTSGYAFGGGTEVVVK

SEQ ID NO: 245 - protein, 113 aa, Oryctolagus cuniculus
AQVLTQTPSPVSAAVGGTVTINCQASQSVYGTNRLAWYQQKPGQPPKLLIYDASTLASGVPSRFSGSGSGTQFTLTISGVQCDDAATYCCQGEFSCSNGDCIAFGGGTEVVVK

SEQ ID NO: 246 - protein, 110 aa, Oryctolagus cuniculus
AFELTQTPSSVSAAVGGTVTIKCQASQNIYSKFAWYQQKPGQRPKLLIYSASTLASGVPSRFKGNGSGTEFTLTISDLECADAATYYCQGGYYGSSDTVTFGGGTEVVVK

SEQ ID NO: 247 - protein, 110 aa, Oryctolagus cuniculus
AYDMTQTPASVEVALGGTVTIKCQASQSIGVSLAWYQQKPGQRPKLLIYSASTLASGVSSRFKGSGSGTEFTLTISGVECADAATYYCQQGYTSSNVDNVFGGGTEVVVK

SEQ ID NO: 248 - protein, 113 aa, Oryctolagus cuniculus
AQVLTQTASPVSAAVGSTVTINCQASQSVYNNNYLGWFQQKPGQPPKRLIYSASKLESGVPSRFSGSGSGTQFTLTISDVQCEDAATYYCLGSYDCSSADCNVFGGGTEVVVK

SEQ ID NO: 249 - protein, 111 aa, Oryctolagus cuniculus
DVVMTQTPASVSAAVGGTVTINCQASESIDNWLAWYQQKPGQPPKLLIYSASNLASGVSSRFEGSTSGTQFTLTISDLECADAATYYCQSTFYGVNPVPNAFGGGTEVVVK

SEQ ID NO: 250 - protein, 111 aa, Oryctolagus cuniculus
AAVLTQTPSPVSAAVGGTVTIKCQSSQSVYSNNNLAWYQQKPGQPPKLLIYDASNLASGVPDRFSGSGSGTQFTLTISGVQCDDAATYYCLGVYDDDADNAFGGGTEVVVK

SEQ ID NO: 251 - protein, 113 aa, Oryctolagus cuniculus
DVVMTQTPASVEAAVGGTVTIKCQASQSISSYLSWYQQKPGQPPKLLIYRASSLESGVPSRFKGTGSGTEFTLTISDLECADAATYYCQCTYGSSTSSRSGNAFGGGTEVVVK

SEQ ID NO: 252 - protein, 111 aa, Oryctolagus cuniculus
DVVMTQTPASVEADVGGTVTIKCQASQSIRSYLAWYQQKPGQPPKVLIYRASTLESGVPSRFKGSGSGTQFTLTISDLECADAATYYCQCTYGSSGSSFLAFGGGTEVVVK

SEQ ID NO: 253 - protein, 110 aa, Oryctolagus cuniculus
AYDMTQTPASVEVAVGGTVTIKCQASESISVNLAWYQQKSGQPPKLLIYLASTLASGVPSRFKGSGSGTEFTLTISDLECADAATYYCQQTYSGSNVENSFGGGTEVVLK

SEQ ID NO: 254 - protein, 111 aa, Oryctolagus cuniculus
AAVLTQTPSPVSAAVGGTVSISCQSSESIYKNNYLAWYQQKSGQPPKLLIYRASTLTSGVPSRFKGSGSGTQFTLTISDVQCDDAATYYCAGDYSSSSDNTFGGGTEVVVK

SEQ ID NO: 255 - protein, 110 aa, Oryctolagus cuniculus
DVVMTQTPASASEPVGGTVTIKCQASQNIYSDFAWYRQKPGQPPKLLIYSASALASGVPSRFKGSGSGTDFTLTISDLECDDAAIYYCQSTYWESNNIGTFGGGTEVVVK

SEQ ID NO: 256 - protein, 112 aa, Oryctolagus cuniculus
AAVLTQTPSPVSAAVGGTVTISCQASQSVYNHKNLAWYQQKPGQPPKLLIYSASSLASGVPSRFKGSGSGTQFTLTISDLDCDDAATYYCAGGYSGSADTFAFGGGTEVVVK

SEQ ID NO: 257 - protein, 109 aa, Oryctolagus cuniculus
AFELTQTPASVEAAVGGTVTIKCQASQSISAYLSWYQQKPGQPPKLLIYDASDLASGVSSRFKGSGSGTEYTLTISGVQCADAATYYCQSYAGISSGVAFGGGTEVVVK

SEQ ID NO: 258 - protein, 112 aa, Oryctolagus cuniculus
DIVMTQTPASVEAAVGGTVTIKCQASQTITSYLAWYQQKPGQPPKLLIYRASILESGVPSRFKGSGSGTEFTLTISDLECADAATYYCQCTYGTTNTGHYVGFGGGTEVVVK

SEQ ID NO: 259 - protein, 112 aa, Oryctolagus cuniculus
AQVLTQTPSPVSAAVGGTVTINCQASQSVYNNKNLAWYQQKPGQPPKLLIYDASKLASGVPLRFSGSGSGTQFTLTISGVQCDDAATYYCAGGYDSSVDTFAFGGGTEVVVK

SEQ ID NO: 260 - protein, 113 aa, Oryctolagus cuniculus
DTVMTQTPASVEAAVGGTVTIQCQASENIYSLLAWYQQKPGQPPKLLIYRASTLASGVPSRFKGSGSGTEFTLTISDLECADAATYYCQSHYCCSSNYDYIYAFGGGTEVVVK

SEQ ID NO: 261 - protein, 112 aa, Oryctolagus cuniculus
DPVLTQTPPSASEPAGGTVTIKCQASEDIYSLLAWYQQKPGQPPKLLIYAASTLASGVPSRFKGSGSGTQFTLTISDLECADAATYYCQSYYYSISDSVDYPFGGGTEVVVK

SEQ ID NO: 262 - protein, 113 aa, Oryctolagus cuniculus
DVVMTQTPASVEAAVGGTVTIKCQASQSISTYLSWYQQKPGQPPKLLIYRATTLESGVPSRFKGTGSGTEFTLTINDLECADAATYYCQCTYGSSASSSYGNAFGGGTEVVVK

SEQ ID NO: 263 - protein, 109 aa, Oryctolagus cuniculus
AQVLTQTPSSVSEPVGGTVTINCQASENIYSSLAWYQQKPGQPPKLLIYDASDLASGVPSRFSGSGLGTEFTLTISGVQCDDAATYYCQTYYPSSVTYAFGGGTEVVVK

SEQ ID NO: 264 - protein, 111 aa, Oryctolagus cuniculus
AYDMTQTPSSVSAAVGGTVTINCQASESIGSWLAWYQQKPGQPPKLLIYSASSLASGVSSRFGGSTSGTEYTLTISDLECADAATYYCQSTFYGVNPVPTAFGGGTEVVVK

SEQ ID NO: 265 - protein, 111 aa, Oryctolagus cuniculus
AQVLTQTASPVSAAVGGTVTINCQSSQSVYNNNRLSWFQQKPGQPPKQLIYRSSTLASGVPSRFSGSGSGTQFTLTISDVQCDDAATYYCAGGYSSSSDNAFGGGTEVVVK

SEQ ID NO: 266 - protein, 110 aa, Oryctolagus cuniculus
AAVLTQTPSPVSAAVGGTVTISCQASQSVYNNNNLAWYQQKPGQPPKLLIYTASSLASGVPSRFKGSGSGTQFTLTISEVQCEDAATYYCQGYYSGYINAFGGGTEVVVK

SEQ ID NO: 267 - protein, 112 aa, Oryctolagus cuniculus
DIVMTQTPASVEAAVGGTVTIKCQASQSIGSYLSWYQQKPGQPPKLLIYYASDLESGVPSRFKGSGSGTEFTLTISDLECADACTYYCQCTYGSISSSAGNAFGGGTEVVVK

SEQ ID NO: 268 - protein, 110 aa, Oryctolagus cuniculus
AQVLTQTASPVSAAVGGTVTISCQSSESVYNNNLLSWYKQKPGQPPKLLIYKASTLDSGVPSRFKGSGSGTQFTLTISGVQCDDAATYYCQGGYTDATYAFGGGTEVVVK

SEQ ID NO: 269 - protein, 112 aa, Oryctolagus cuniculus
AQVLTQTPSPVSATVGGTVTINCQASQSVYNNRLAWYQQKPGQPPKLLIYEASTLTSGVSSRFKGSGSGAQFTLTISGVQCADAATYYCQGEFSCSNGDCIAFGGGTEVVVK

SEQ ID NO: 270 - protein, 112 aa, Oryctolagus cuniculus
DVVMTQTPASVEAAVGGTVTIKCQASQSISTYSSWYEQKPGQPPKLLIYYASDLESGVPSRFKGSGSGTEFTLTISDLECADAATYYCQCTYGSISSSSGNAFGGGTEVVVK

SEQ ID NO: 271 - protein, 110 aa, Oryctolagus cuniculus
AQVLTQTPSSVSAAVGGTVTISCQSSQSVYASVWLGWYQQKPGQPPKQLIYAASTLASGVPSRFKGSGSGTQFTLTISDLECGDAATYYCAGGYIGDIYAFGGGTEVVVE

SEQ ID NO: 272 - protein, 113 aa, Oryctolagus cuniculus
DVVMTQTPASVEAAVGGTVTIKCQASQSIYNYLSWYQQKPGQPPKLLIYGASDLASGVPSRFSGSGSGTEFTLTISDLECADAATYYCQCTYGSSRVSSYGDAFGGGTEVVVK

SEQ ID NO: 273 - protein, 108 aa, Oryctolagus cuniculus
DVVMTQTPVSVSAAVGGTVTINCQASQNIYSYLAWYQQKSGQPPKLLIYDASDLESGVPSRFKGSGSGTEYTLTISDLECADAATYYCQSYYGISAYAFGGGTEVVVK

SEQ ID NO: 274 - protein, 111 aa, Oryctolagus cuniculus
DIVMTQTPASVSEPVGGTVTIKCQASQSIYSYLAWYQQKPGQRPKLLIYGASTLASGVPSRFKGSGSGTDFALTISDLECADAATYYCQDNYGSSTTYGNSFGGGTEVVVK

SEQ ID NO: 275 - protein, 113 aa, Oryctolagus cuniculus
DIVMTQTPASVEAAVGGTVTIKCQASESIGSVLAWYQQKPGQSPKLLIGSASTLASGVPSRFKGSGSGTQFTLTISDLECADAATYYCQSYYHSTSGSSYGNTFGGGTEVVVK

SEQ ID NO: 276 - protein, 111 aa, Oryctolagus cuniculus
ALVMTQTPSSVSAAVGGTVTINCQASQNIYSNLAWYQQKPGQPPKLLIYGASDLESGVPSRFKGSGSGTEYTLTISDLECDDAATYYCQSTYYNISADFYAFGGGTEVVVK

SEQ ID NO: 277 - protein, 111 aa, Oryctolagus cuniculus
AAVLTQTPSPVSAVVGGTVSISCQSNKNVYDNNALSWYQQKPGQPPKFLIYRASTLASGVPSRFKGSGSGTQFTLTISDVQCDDAATYYCAGDYISDSDNTFGGGTEVVVK

SEQ ID NO: 278 - protein, 113 aa, Oryctolagus cuniculus
DIVMTQTPASVSEPVGGTVTIKCQASQSIINYLSWYQQKPGQPPKLLIYRASTLESGVPSRFKGSGSGTEFTLTISDLECADAATYYCQCTYGSSSGSYGGWAFGGGTEVVVK

SEQ ID NO: 279 - protein, 110 aa, Oryctolagus cuniculus
DIVMTQTPASVSEPVGGTVTIKCQASQSIYSYLSWYQQKPGQPPKLLIYQASILASGVPSQFKGSGSGTDFTLTISDLECADAATYYCQSNYGFSSGSYAFGGGTEVVVK

SEQ ID NO: 280 - protein, 112 aa, Oryctolagus cuniculus
DVVMTQTPASVEAAVGGTVTIKCQASQSISSWLAWYQQKPGQPPKLLIYRASTLESGVPSRFKGSGSGTEFTLTISDLECADAATYYCQCTYGSLSSTYGWAFGGGTEVVVK

SEQ ID NO: 281 - protein, 112 aa, Oryctolagus cuniculus
AAVLTQTPSSVSAAVGGTVTINCQSSQSVNNAKNLAWYQQKPGQPPKLLIYDASTLASGVPSRFKGSGSGTQFTLIMSDLECGDAATYFCAGGYDRFIDTFAFGGGTEVVVK

SEQ ID NO: 282 - protein, 111 aa, Oryctolagus cuniculus
AAVLTQTPSPVSAAVGGTVSISCQSSKSVYDNNWLSWYQQKPGQPPKLLIYQASTLASGVPSRFKGSGSGTQFTLTISDVQCDDAATYYCAGGYITNSDNGFGGGTEVVVK

SEQ ID NO: 283 - protein, 110 aa, Oryctolagus cuniculus
DVVMTQTPASVSESVGGTVTIKCQASQSIGSSLAWYQQKPGQPPKLLIYYTSTLASGVPSRFSGSGSGTEFTLTTSGVQCDDAATYYCQSYGYGSGYVFAFGGGTEVVVK

SEQ ID NO: 284 - protein, 111 aa, Oryctolagus cuniculus
AIEMTQTPFSVSAAVGGTVTINCQASENIYRNLAWYQQKPGQPPKLLIYKASTLASGVSSRFKGSGSGTQFTLTIGGVQCDDAATYYCLYSYYIDSNVDFAFGGGTEVVVK

SEQ ID NO: 285 - protein, 111 aa, Oryctolagus cuniculus
DVVMTQTPASVSEPVGGTVTIKCQASEDIESYLAWYQQKPGQPPKLLIYSASTLASGVPSRFSGSGYGTEFTLTISDLECADAATYYCQCTLYGVNFVPNVFGGGTEVVVK

SEQ ID NO: 286 - protein, 113 aa, Oryctolagus cuniculus
DVVMTQTPASVSEPVGGTVTIKCQASQSISSWLSWYQQKPGQPPKVLIYDASDLASGVSSRFKGTGAGTEFTLTISDLECADAATYYCQCTVGSSGVTGYGNAFGGGTEVVVK

SEQ ID NO: 287 - protein, 109 aa, Oryctolagus cuniculus
DVVMTQTPASVSEPVGGTVTIKCQASQSIGSDLAWYQQKPGQPPKLLIYDASSLESGVPSRFKGSGSGTDFTLTISDLECADAATYYCQCTYYGGSPNVFGGGTEVVVK

SEQ ID NO: 288 - protein, 110 aa, Oryctolagus cuniculus
AIEMTQTPASVEAAVGGTVTIKCQGSQSISSYLSWYQQKPGQPPKLLIYGASTLASGVSSRFKGSGSGTEFTLTISGVECADAATYYCQQGYTTSNVDNTFGGGTEVVVK

SEQ ID NO: 289 - protein, 110 aa, Oryctolagus cuniculus
AAVLTQTPSPVSAPVGGTVSISCQSSPSVYSVYLSWYQQKPGQPPKLLIYRASTLASGVPSRFKGSGSGTQFTLTISDVQCDDAATYYCAGAYVGSSDNTFGGGTEMVVK

SEQ ID NO: 290 - protein, 111 aa, Oryctolagus cuniculus
AAVLTQTPSPVSAAVGGTVSISCQSSKSVYNNKWLSWFQQKPGQPPKLLIYGAFTLASGVPSRFRGSGSGTQFTLTISDVQCDDAATYYCAGDYSSNSDDAFGGGTEVVVK

SEQ ID NO: 291 - protein, 112 aa, Oryctolagus cuniculus
DIVMTQTPASVEAAVGGTVTIKCQASESVGDALAWYQQKPGQPPKLLIYRASTLESGVPSRFKGSGSGTEFTLTISDLECADVATYYCQSYWYTMGNSYGNTFGGGTEVVVK

SEQ ID NO: 292 - protein, 111 aa, Oryctolagus cuniculus
AAVLTQTPSPVSAAVGGTVSISCQSSKTIYNDNWLSWFQQKPGQPPKLLIYGASTLASGVPSRFKGSGSGTQFTLTISDVQCDDAATYYCLGSYINSSDNAFGGGTEVVVK

SEQ ID NO: 293 - protein, 111 aa, Oryctolagus cuniculus
AIKMTQTPSSVSAAVGGTVTINCRASEDIKSYLAWYQQKPGQPPKLLIYDASDLASGVPSRFKGSGSGTEYTLTISGVQCDDAATYYCQSAYYSSSTDGGAFGGGTEVVVK

SEQ ID NO: 294 - protein, 111 aa, Oryctolagus cuniculus
ALVMTQTPSSVSAPVGGTVTINCQASQSIYSNLAWYQQKPGQRPKLLIYGASNLESGVPSRFKGSGSGTQFTLTISDLECADAATYCCQGYYYADSDDNIAFGGGTEVVVE

SEQ ID NO: 295 - protein, 110 aa, Oryctolagus cuniculus
AQVLTQTASPVSAAVGSTVTISCQASQSVYNNNYLAWFQQKPGQPPKLLIYLASTLASGVPSRFKGSGSGTQFTLTISGVQCGDAATYYCQGYYSTGMFAFGGGTEVVVK

SEQ ID NO: 296 - protein, 111 aa, Oryctolagus cuniculus
DVVMTQTPSSVSAAVGGTVTINCRASEDIERFLAWYQQKPGQPPKLLIYKASTLASGVPSRFKGSGSGTDFTLTISDLECADAATYYCQCTLYGVNFVPNAFGGGTEVVVK

SEQ ID NO: 297 - protein, 5 aa, Oryctolagus cuniculus
AYAIN

SEQ ID NO: 298 - protein, 5 aa, Oryctolagus cuniculus
GYDMN

SEQ ID NO: 299 - protein, 5 aa, Oryctolagus cuniculus
TYAIS

SEQ ID NO: 300 - protein, 5 aa, Oryctolagus cuniculus
GLVVS

SEQ ID NO: 301 - protein, 6 aa, Oryctolagus cuniculus
SSYYMC

SEQ ID NO: 302 - protein, 5 aa, Oryctolagus cuniculus
IYAIS

SEQ ID NO: 303 - protein, 6 aa, Oryctolagus cuniculus
SSYYMC

SEQ ID NO: 304 - protein, 5 aa, Oryctolagus cuniculus
MYAIN

SEQ ID NO: 305 - protein, 6 aa, Oryctolagus cuniculus
SYYYMC

SEQ ID NO: 306 - protein, 5 aa, Oryctolagus cuniculus
RNAMS

SEQ ID NO: 307 - protein, 6 aa, Oryctolagus cuniculus
DNYAMC

SEQ ID NO: 308 - protein, 6 aa, Oryctolagus cuniculus
SGYYMC

SEQ ID NO: 309 - protein, 6 aa, Oryctolagus cuniculus
GNYYIC

SEQ ID NO: 310 - protein, 6 aa, Oryctolagus cuniculus
RSYYMC

SEQ ID NO: 311 - protein, 6 aa, Oryctolagus cuniculus
SMYWMC

SEQ ID NO: 312 - protein, 5 aa, Oryctolagus cuniculus
SYDMS

SEQ ID NO: 313 - protein, 6 aa, Oryctolagus cuniculus
SSYWIC

SEQ ID NO: 314 - protein, 6 aa, Oryctolagus cuniculus
SSYYIC

SEQ ID NO: 315 - protein, 6 aa, Oryctolagus cuniculus
DGYWMC

SEQ ID NO: 316 - protein, 5 aa, Oryctolagus cuniculus
SYAMS

SEQ ID NO: 317 - protein, 5 aa, Oryctolagus cuniculus
NYQMT

SEQ ID NO: 318 - protein, 5 aa, Oryctolagus cuniculus
MYAIN

SEQ ID NO: 319 - protein, 5 aa, Oryctolagus cuniculus
NYDMN

SEQ ID NO: 320 - protein, 5 aa, Oryctolagus cuniculus
NYDMN

SEQ ID NO: 321 - protein, 5 aa, Oryctolagus cuniculus
SNAMI

SEQ ID NO: 322 - protein, 5 aa, Oryctolagus cuniculus
MYTIN

SEQ ID NO: 323 - protein, 5 aa, Oryctolagus cuniculus
SNSIS

SEQ ID NO: 324 - protein, 6 aa, Oryctolagus cuniculus
STYWMS

SEQ ID NO: 325 - protein, 5 aa, Oryctolagus cuniculus
NYALS

SEQ ID NO: 326 - protein, 5 aa, Oryctolagus cuniculus
SHATS

SEQ ID NO: 327 - protein, 5 aa, Oryctolagus cuniculus
TYGVS

SEQ ID NO: 328 - protein, 6 aa, Oryctolagus cuniculus
SNYYIC

SEQ ID NO: 329 - protein, 5 aa, Oryctolagus cuniculus
TYAMT

SEQ ID NO: 330 - protein, 6 aa, Oryctolagus cuniculus
SSYWIC

SEQ ID NO: 331 - protein, 5 aa, Oryctolagus cuniculus
NYAMS

SEQ ID NO: 332 - protein, 5 aa, Oryctolagus cuniculus
NYQMT

SEQ ID NO: 333 - protein, 6 aa, Oryctolagus cuniculus
STYWAC

SEQ ID NO: 334 - protein, 5 aa, Oryctolagus cuniculus
SYQMT

SEQ ID NO: 335 - protein, 6 aa, Oryctolagus cuniculus
SSYYMC

SEQ ID NO: 336 - protein, 6 aa, Oryctolagus cuniculus
SNYYMC

SEQ ID NO: 337 - protein, 6 aa, Oryctolagus cuniculus
SSYYMC

SEQ ID NO: 338 - protein, 5 aa, Oryctolagus cuniculus
NWIMS

SEQ ID NO: 339 - protein, 6 aa, Oryctolagus cuniculus
STYSMC

SEQ ID NO: 340 - protein, 6 aa, Oryctolagus cuniculus
SGYDMC

SEQ ID NO: 341 - protein, 6 aa, Oryctolagus cuniculus
STYYTC

SEQ ID NO: 342 - protein, 5 aa, Oryctolagus cuniculus
SAAMG

SEQ ID NO: 343 - protein, 5 aa, Oryctolagus cuniculus
SYDMS

SEQ ID NO: 344 - protein, 6 aa, Oryctolagus cuniculus
STYWIC

SEQ ID NO: 345 - protein, 6 aa, Oryctolagus cuniculus
SSYWIC

SEQ ID NO: 346 - protein, 5 aa, Oryctolagus cuniculus
SDGIS

SEQ ID NO: 347 - protein, 5 aa, Oryctolagus cuniculus
SYAIS

SEQ ID NO: 348 - protein, 5 aa, Oryctolagus cuniculus
SNALG

SEQ ID NO: 349 - protein, 5 aa, Oryctolagus cuniculus
SYDMS

SEQ ID NO: 350 - protein, 5 aa, Oryctolagus cuniculus
NYAMG

SEQ ID NO: 351 - protein, 5 aa, Oryctolagus cuniculus
VYAMS

SEQ ID NO: 352 - protein, 5 aa, Oryctolagus cuniculus
TYGVS

SEQ ID NO: 353 - protein, 5 aa, Oryctolagus cuniculus
MYAIN

SEQ ID NO: 354 - protein, 5 aa, Oryctolagus cuniculus
RYAMS

SEQ ID NO: 355 - protein, 5 aa, Oryctolagus cuniculus
SYAMG

SEQ ID NO: 356 - protein, 6 aa, Oryctolagus cuniculus
SSYWIC

SEQ ID NO: 357 - protein, 5 aa, Oryctolagus cuniculus
NYYMT

SEQ ID NO: 358 - protein, 5 aa, Oryctolagus cuniculus
SYHMS

SEQ ID NO: 359 - protein, 5 aa, Oryctolagus cuniculus
TIPMC

SEQ ID NO: 360 - protein, 6 aa, Oryctolagus cuniculus
DNYAMC

SEQ ID NO: 361 - protein, 5 aa, Oryctolagus cuniculus
SYHMG

SEQ ID NO: 362 - protein, 6 aa, Oryctolagus cuniculus
SRYWIY

SEQ ID NO: 363 - protein, 5 aa, Oryctolagus cuniculus
SYFLT

SEQ ID NO: 364 - protein, 5 aa, Oryctolagus cuniculus
SYAMS

SEQ ID NO: 365 - protein, 5 aa, Oryctolagus cuniculus
SNAMC

SEQ ID NO: 366 - protein, 5 aa, Oryctolagus cuniculus
VYAMS

SEQ ID NO: 367 - protein, 5 aa, Oryctolagus cuniculus
SYAMG

SEQ ID NO: 368 - protein, 6 aa, Oryctolagus cuniculus
GSYWNC

SEQ ID NO: 369 - protein, 6 aa, Oryctolagus cuniculus
SGYDMC

SEQ ID NO: 370 - protein, 5 aa, Oryctolagus cuniculus
AYGVN

SEQ ID NO: 371 - protein, 6 aa, Oryctolagus cuniculus
NSYYMC

SEQ ID NO: 372 - protein, 5 aa, Oryctolagus cuniculus
SNAMC

SEQ ID NO: 373 - protein, 5 aa, Oryctolagus cuniculus
SYAMG

SEQ ID NO: 374 - protein, 5 aa, Oryctolagus cuniculus
TNGVS

SEQ ID NO: 375 - protein, 6 aa, Oryctolagus cuniculus
SGYYMC

SEQ ID NO: 376 - protein, 6 aa, Oryctolagus cuniculus
SGYCLC

SEQ ID NO: 377 - protein, 5 aa, Oryctolagus cuniculus
SYWMC

SEQ ID NO: 378 - protein, 6 aa, Oryctolagus cuniculus
SYYYMS

SEQ ID NO: 379 - protein, 5 aa, Oryctolagus cuniculus
YNTIC

SEQ ID NO: 380 - protein, 6 aa, Oryctolagus cuniculus
SSYYMC

SEQ ID NO: 381 - protein, 5 aa, Oryctolagus cuniculus
NYAMS

SEQ ID NO: 382 - protein, 5 aa, Oryctolagus cuniculus
NYAVG

SEQ ID NO: 383 - protein, 6 aa, Oryctolagus cuniculus
SSYYMC

SEQ ID NO: 384 - protein, 6 aa, Oryctolagus cuniculus
SRYYVC

SEQ ID NO: 385 - protein, 5 aa, Oryctolagus cuniculus
ANAMS

SEQ ID NO: 386 - protein, 5 aa, Oryctolagus cuniculus
NYHMS

SEQ ID NO: 387 - protein, 5 aa, Oryctolagus cuniculus
NYGLT

SEQ ID NO: 388 - protein, 6 aa, Oryctolagus cuniculus
SSYYMC

SEQ ID NO: 389 - protein, 5 aa, Oryctolagus cuniculus
TYAMS

SEQ ID NO: 390 - protein, 5 aa, Oryctolagus cuniculus
NYGVS

SEQ ID NO: 391 - protein, 6 aa, Oryctolagus cuniculus
VSYWIC

SEQ ID NO: 392 - protein, 6 aa, Oryctolagus cuniculus
SGYDMC

SEQ ID NO: 393 - protein, 5 aa, Oryctolagus cuniculus
SNAMC

SEQ ID NO: 394 - protein, 6 aa, Oryctolagus cuniculus
SSYYMC

SEQ ID NO: 395 - protein, 6 aa, Oryctolagus cuniculus
SSYWIY

SEQ ID NO: 396 - protein, 5 aa, Oryctolagus cuniculus
RYGVS

SEQ ID NO: 397 - protein, 6 aa, Oryctolagus cuniculus
NNYYMC

SEQ ID NO: 398 - protein, 6 aa, Oryctolagus cuniculus
SNYYMC

SEQ ID NO: 399 - protein, 5 aa, Oryctolagus cuniculus
SYAMS

SEQ ID NO: 400 - protein, 6 aa, Oryctolagus cuniculus
SSYCMC

SEQ ID NO: 401 - protein, 5 aa, Oryctolagus cuniculus
SYAMG

SEQ ID NO: 402 - protein, 6 aa, Oryctolagus cuniculus
SGYDMC

SEQ ID NO: 403 - protein, 5 aa, Oryctolagus cuniculus
DYYMS

SEQ ID NO: 404 - protein, 5 aa, Oryctolagus cuniculus
SHATS

SEQ ID NO: 405 - protein, 6 aa, Oryctolagus cuniculus
SGYWIC

SEQ ID NO: 406 - protein, 5 aa, Oryctolagus cuniculus
SYTMA

SEQ ID NO: 407 - protein, 5 aa, Oryctolagus cuniculus
SYHMC

SEQ ID NO: 408 - protein, 6 aa, Oryctolagus cuniculus
GDYDMC

SEQ ID NO: 409 - protein, 6 aa, Oryctolagus cuniculus
SSYYMC

SEQ ID NO: 410 - protein, 5 aa, Oryctolagus cuniculus
SYAMS

SEQ ID NO: 411 - protein, 5 aa, Oryctolagus cuniculus
SYTMT

SEQ ID NO: 412 - protein, 6 aa, Oryctolagus cuniculus
SKYYMC

SEQ ID NO: 413 - protein, 5 aa, Oryctolagus cuniculus
SYYIY

SEQ ID NO: 414 - protein, 6 aa, Oryctolagus cuniculus
SVYDMC

SEQ ID NO: 415 - protein, 5 aa, Oryctolagus cuniculus
SYHMS

SEQ ID NO: 416 - protein, 5 aa, Oryctolagus cuniculus
GLVVS

SEQ ID NO: 417 - protein, 5 aa, Oryctolagus cuniculus
RDAMS

SEQ ID NO: 418 - protein, 5 aa, Oryctolagus cuniculus
SYWIC

SEQ ID NO: 419 - protein, 5 aa, Oryctolagus cuniculus
RYAMI

SEQ ID NO: 420 - protein, 6 aa, Oryctolagus cuniculus
NNYWIC

SEQ ID NO: 421 - protein, 6 aa, Oryctolagus cuniculus
TYYYMC

SEQ ID NO: 422 - protein, 5 aa, Oryctolagus cuniculus
SYWMS

SEQ ID NO: 423 - protein, 5 aa, Oryctolagus cuniculus
RNAAS

SEQ ID NO: 424 - protein, 5 aa, Oryctolagus cuniculus
NYAMT

SEQ ID NO: 425 - protein, 5 aa, Oryctolagus cuniculus
SNAIS

SEQ ID NO: 426 - protein, 6 aa, Oryctolagus cuniculus
VGYYMC

SEQ ID NO: 427 - protein, 6 aa, Oryctolagus cuniculus
SSYWIC

SEQ ID NO: 428 - protein, 6 aa, Oryctolagus cuniculus
SSYYMC

SEQ ID NO: 429 - protein, 5 aa, Oryctolagus cuniculus
NYHMT

SEQ ID NO: 430 - protein, 5 aa, Oryctolagus cuniculus
SYDMT

SEQ ID NO: 431 - protein, 6 aa, Oryctolagus cuniculus
SSYCVC

SEQ ID NO: 432 - protein, 5 aa, Oryctolagus cuniculus
SNAMC

SEQ ID NO: 433 - protein, 6 aa, Oryctolagus cuniculus
GNYYMC

SEQ ID NO: 434 - protein, 5 aa, Oryctolagus cuniculus
SYHMN

SEQ ID NO: 435 - protein, 6 aa, Oryctolagus cuniculus
SSYYMC

SEQ ID NO: 436 - protein, 5 aa, Oryctolagus cuniculus
SYPVN

SEQ ID NO: 437 - protein, 5 aa, Oryctolagus cuniculus
SYDMS

SEQ ID NO: 438 - protein, 5 aa, Oryctolagus cuniculus
NYGMT

SEQ ID NO: 439 - protein, 5 aa, Oryctolagus cuniculus
TYWMS

SEQ ID NO: 440 - protein, 5 aa, Oryctolagus cuniculus
SYAMG

SEQ ID NO: 441 - protein, 6 aa, Oryctolagus cuniculus
SSYYMC

SEQ ID NO: 442 - protein, 6 aa, Oryctolagus cuniculus
SGQDMC

SEQ ID NO: 443 - protein, 5 aa, Oryctolagus cuniculus
SYNMG

SEQ ID NO: 444 - protein, 6 aa, Oryctolagus cuniculus
SSYYMC

SEQ ID NO: 445 - protein, 16 aa, Oryctolagus cuniculus
GIANNGPTYYANWAKG

SEQ ID NO: 446 - protein, 16 aa, Oryctolagus cuniculus
MIYPNSGTNYATWAKG

SEQ ID NO: 447 - protein, 16 aa, Oryctolagus cuniculus
GISNSGTTYYASWAKG

SEQ ID NO: 448 - protein, 16 aa, Oryctolagus cuniculus
VIGKSGNTYYASWAKG

SEQ ID NO: 449 - protein, 18 aa, Oryctolagus cuniculus
CIYAGSSGSTYYASWAKG

SEQ ID NO: 450 - protein, 16 aa, Oryctolagus cuniculus
GIGNNGIIHYANWAKG

SEQ ID NO: 451 - protein, 18 aa, Oryctolagus cuniculus
CIYGGSSGKTWYASWAKG

SEQ ID NO: 452 - protein, 16 aa, Oryctolagus cuniculus
GIANNGPTYYASWAKG

SEQ ID NO: 453 - protein, 17 aa, Oryctolagus cuniculus
CIYADDATTYYATWAKG

SEQ ID NO: 454 - protein, 16 aa, Oryctolagus cuniculus
IIRNTGTTWYASWAKG

SEQ ID NO: 455 - protein, 17 aa, Oryctolagus cuniculus
CIYVGSGSTYYASWAQG

SEQ ID NO: 456 - protein, 17 aa, Oryctolagus cuniculus
CIYTSSGSTYYASWAKG

SEQ ID NO: 457 - protein, 18 aa, Oryctolagus cuniculus
CIYAGSSGSTYYASWAKG

SEQ ID NO: 458 - protein, 18 aa, Oryctolagus cuniculus
CIYAGSSDSTYYASWAKG

SEQ ID NO: 459 - protein, 18 aa, Oryctolagus cuniculus
CIYTGSSGKTHYASWAKG

SEQ ID NO: 460 - protein, 16 aa, Oryctolagus cuniculus
IIYDSGSTYYANWAKG

SEQ ID NO: 461 - protein, 17 aa, Oryctolagus cuniculus
CIAAGSGSTYYASWAKG

SEQ ID NO: 462 - protein, 18 aa, Oryctolagus cuniculus
CIYAGSSGSTYYASWAKG

SEQ ID NO: 463 - protein, 17 aa, Oryctolagus cuniculus
CIYTGPGGTFYASWAKG

SEQ ID NO: 464 - protein, 16 aa, Oryctolagus cuniculus
IIHYSGYTAYASWAKG

SEQ ID NO: 465 - protein, 16 aa, Oryctolagus cuniculus
FIKADGSAYYANWAKG

SEQ ID NO: 466 - protein, 16 aa, Oryctolagus cuniculus
GIATNGIIHYASWVKG

SEQ ID NO: 467 - protein, 16 aa, Oryctolagus cuniculus
MIYPNSGTNYASWAKG

SEQ ID NO: 468 - protein, 16 aa, Oryctolagus cuniculus
MIYPNGGTNYATWAKG

SEQ ID NO: 469 - protein, 16 aa, Oryctolagus cuniculus
IIYASDSTYYATWAKG

SEQ ID NO: 470 - protein, 16 aa, Oryctolagus cuniculus
GIATHGIIHYASWVKG

SEQ ID NO: 471 - protein, 16 aa, Oryctolagus cuniculus
IISSSGSTYYASWAKG

SEQ ID NO: 472 - protein, 17 aa, Oryctolagus cuniculus
CIVTGRGNTYYANWAKG

SEQ ID NO: 473 - protein, 16 aa, Oryctolagus cuniculus
FINIIHGAYYASWAKG

SEQ ID NO: 474 - protein, 16 aa, Oryctolagus cuniculus
FIKTGGSAYYASWAKG

SEQ ID NO: 475 - protein, 16 aa, Oryctolagus cuniculus
YINTGGSASYATWAKG

SEQ ID NO: 476 - protein, 18 aa, Oryctolagus cuniculus
CIYTGSTGSTYYASWAKG

SEQ ID NO: 477 - protein, 16 aa, Oryctolagus cuniculus
IISNSGATAYASWAKG

SEQ ID NO: 478 - protein, 17 aa, Oryctolagus cuniculus
CIGTSSTISYYASWAKG

SEQ ID NO: 479 - protein, 16 aa, Oryctolagus cuniculus
IIHYSGYIAYANWAKG

SEQ ID NO: 480 - protein, 16 aa, Oryctolagus cuniculus
FIKPGGSAYYASWAKG

SEQ ID NO: 481 - protein, 18 aa, Oryctolagus cuniculus
CIDGGSSGITGYANWAKG

SEQ ID NO: 482 - protein, 16 aa, Oryctolagus cuniculus
FINTGGSAYYASWAKG

SEQ ID NO: 483 - protein, 18 aa, Oryctolagus cuniculus
CIYAGSSGSTYYASWAKG

SEQ ID NO: 484 - protein, 18 aa, Oryctolagus cuniculus
CIYTGSSGSTYYASWAKG

SEQ ID NO: 485 - protein, 18 aa, Oryctolagus cuniculus
CIHAGSSGAAYYATWAKG

SEQ ID NO: 486 - protein, 16 aa, Oryctolagus cuniculus
IITTSGNTYYASWAKG

SEQ ID NO: 487 - protein, 18 aa, Oryctolagus cuniculus
CIYTGSSGGTYYASWAKG

SEQ ID NO: 488 - protein, 17 aa, Oryctolagus cuniculus
CIYTVNDNTWYASWAKG

SEQ ID NO: 489 - protein, 18 aa, Oryctolagus cuniculus
CIVDGSSGNTYYASWAKG

SEQ ID NO: 490 - protein, 16 aa, Oryctolagus cuniculus
YISTSGTPYYASWVNG

SEQ ID NO: 491 - protein, 16 aa, Oryctolagus cuniculus
IIYNSGTTYYANWAKG

SEQ ID NO: 492 - protein, 18 aa, Oryctolagus cuniculus
CIYTDSSTSTYYASWAKG

SEQ ID NO: 493 - protein, 18 aa, Oryctolagus cuniculus
CIVGGGGVNTYYANWAKG

SEQ ID NO: 494 - protein, 17 aa, Oryctolagus cuniculus
FIYPGVGITHYAHSVKG

SEQ ID NO: 495 - protein, 16 aa, Oryctolagus cuniculus
GVANNGITNYASWARG

SEQ ID NO: 496 - protein, 16 aa, Oryctolagus cuniculus
YISTGGSAYYATWVNG

SEQ ID NO: 497 - protein, 16 aa, Oryctolagus cuniculus
IIYDSGSTYYASWAKG

SEQ ID NO: 498 - protein, 16 aa, Oryctolagus cuniculus
VISSNGGTVYANWAKG

SEQ ID NO: 499 - protein, 16 aa, Oryctolagus cuniculus
IITFSGNTYYASWAKG

SEQ ID NO: 500 - protein, 16 aa, Oryctolagus cuniculus
YINIYGRTYYANWAKS

SEQ ID NO: 501 - protein, 16 aa, Oryctolagus cuniculus
GIANNGPTYYASWAKG

SEQ ID NO: 502 - protein, 16 aa, Oryctolagus cuniculus
IISSSGNSYYASWAKG

SEQ ID NO: 503 - protein, 15 aa, Oryctolagus cuniculus
IISSGLTYYASWAKG

SEQ ID NO: 504 - protein, 18 aa, Oryctolagus cuniculus
CINFGRSGNIYYARWAKG

SEQ ID NO: 505 - protein, 16 aa, Oryctolagus cuniculus
FIDPYSSPYYASWAKG

SEQ ID NO: 506 - protein, 16 aa, Oryctolagus cuniculus
VIYGSGSAWYASWAKG

SEQ ID NO: 507 - protein, 17 aa, Oryctolagus cuniculus
CIYPDYGDTFYATWAKG

SEQ ID NO: 508 - protein, 17 aa, Oryctolagus cuniculus
CIFGSSGSIAYATWAKG

SEQ ID NO: 509 - protein, 16 aa, Oryctolagus cuniculus
FITTTGGSYYASWARG

SEQ ID NO: 510 - protein, 18 aa, Oryctolagus cuniculus
CIDTGSRGFTYYPSWAKG

SEQ ID NO: 511 - protein, 16 aa, Oryctolagus cuniculus
FMNSGGSTYYASWVNG

SEQ ID NO: 512 - protein, 16 aa, Oryctolagus cuniculus
MIRSSGITWYASWAKG

SEQ ID NO: 513 - protein, 18 aa, Oryctolagus cuniculus
CIYAGSRGSAYYASWVNG

SEQ ID NO: 514 - protein, 16 aa, Oryctolagus cuniculus
IITWSADTYYTSWAKG

SEQ ID NO: 515 - protein, 16 aa, Oryctolagus cuniculus
INGVSGTTYYATWANG

SEQ ID NO: 516 - protein, 18 aa, Oryctolagus cuniculus
CIDGEGSGNTYYASWVNG

SEQ ID NO: 517 - protein, 17 aa, Oryctolagus cuniculus
CIDTGDGSTYYASWVNG

SEQ ID NO: 518 - protein, 16 aa, Oryctolagus cuniculus
SISNSGGTYYASWAKG

SEQ ID NO: 519 - protein, 18 aa, Oryctolagus cuniculus
CIDAGSVGDTSYATWAKG

SEQ ID NO: 520 - protein, 17 aa, Oryctolagus cuniculus
CIYNGDGSTYYASWVNG

SEQ ID NO: 521 - protein, 16 aa, Oryctolagus cuniculus
IISNSGATAYASWAKG

SEQ ID NO: 522 - protein, 16 aa, Oryctolagus cuniculus
YIFTGGNTYYASWAKG

SEQ ID NO: 523 - protein, 18 aa, Oryctolagus cuniculus
CIYVGITGSTYYASWAKG

SEQ ID NO: 524 - protein, 18 aa, Oryctolagus cuniculus
CKHGGASGTTYYATWAKG

SEQ ID NO: 525 - protein, 18 aa, Oryctolagus cuniculus
CSYAGGSGGTYYASWAKG

SEQ ID NO: 526 - protein, 17 aa, Oryctolagus cuniculus
CTDGTGGITYYASWAKG

SEQ ID NO: 527 - protein, 18 aa, Oryctolagus cuniculus
YINTGSSGTTYYASWAKG

SEQ ID NO: 528 - protein, 18 aa, Oryctolagus cuniculus
CIYAGSSGSTYYASWAKG

SEQ ID NO: 529 - protein, 16 aa, Oryctolagus cuniculus
FINIIDSTYYTNWAKG

SEQ ID NO: 530 - protein, 16 aa, Oryctolagus cuniculus
VINAGGSAYYATWAKG

SEQ ID NO: 531 - protein, 18 aa, Oryctolagus cuniculus
CIYADSSGSTYYASWAKG

SEQ ID NO: 532 - protein, 17 aa, Oryctolagus cuniculus
CIDAGDGSTDYARWAKG

SEQ ID NO: 533 - protein, 16 aa, Oryctolagus cuniculus
TIFDTYLTYNANWAKG

SEQ ID NO: 534 - protein, 16 aa, Oryctolagus cuniculus
FIRTDGSAFYATWAKG

SEQ ID NO: 535 - protein, 16 aa, Oryctolagus cuniculus
YINNNGRTYYASRAKG

SEQ ID NO: 536 - protein, 18 aa, Oryctolagus cuniculus
CVYAGSSGSTYYASWAKG

SEQ ID NO: 537 - protein, 16 aa, Oryctolagus cuniculus
IIDASVTTYYASWAKG

SEQ ID NO: 538 - protein, 17 aa, Oryctolagus cuniculus
YIDPVFRSAYYASWVNG

SEQ ID NO: 539 - protein, 17 aa, Oryctolagus cuniculus
CIGGNSGNIYYARWAKG

SEQ ID NO: 540 - protein, 17 aa, Oryctolagus cuniculus
CIYSSNGLTWYATWAKG

SEQ ID NO: 541 - protein, 17 aa, Oryctolagus cuniculus
CIVTGSGSTYYASWAKG

SEQ ID NO: 542 - protein, 17 aa, Oryctolagus cuniculus
GVDGSGGIKWYANWAKG

SEQ ID NO: 543 - protein, 17 aa, Oryctolagus cuniculus
CFHAGSGSTYYASWVNG

SEQ ID NO: 544 - protein, 16 aa, Oryctolagus cuniculus
WISSSGSAYYATWAKG

SEQ ID NO: 545 - protein, 18 aa, Oryctolagus cuniculus
CIYTGSTGSTYYANWAKG

SEQ ID NO: 546 - protein, 18 aa, Oryctolagus cuniculus
CIYAGSSGSSYYASWAKG

SEQ ID NO: 547 - protein, 16 aa, Oryctolagus cuniculus
IIRRSGATWYANWARG

SEQ ID NO: 548 - protein, 18 aa, Oryctolagus cuniculus
CIYDGSSDSAYYATWAKG

SEQ ID NO: 549 - protein, 16 aa, Oryctolagus cuniculus
IITYGGSTYYASWAKG

SEQ ID NO: 550 - protein, 18 aa, Oryctolagus cuniculus
CIAVYSSGSTYYASWAKG

SEQ ID NO: 551 - protein, 16 aa, Oryctolagus cuniculus
VVSWNGNTYYASWAKG

SEQ ID NO: 552 - protein, 16 aa, Oryctolagus cuniculus
FIKSGGSTYYASWAKG

SEQ ID NO: 553 - protein, 18 aa, Oryctolagus cuniculus
CIDAGSNGSTYYASWARG

SEQ ID NO: 554 - protein, 16 aa, Oryctolagus cuniculus
VINTGGSAYYASWAKG

SEQ ID NO: 555 - protein, 16 aa, Oryctolagus cuniculus
FIKADGNTYYATWAKG

SEQ ID NO: 556 - protein, 18 aa, Oryctolagus cuniculus
CIGAGSSNDTYYASWAKG

SEQ ID NO: 557 - protein, 18 aa, Oryctolagus cuniculus
CISVGSSGSTYYANWAKG

SEQ ID NO: 558 - protein, 16 aa, Oryctolagus cuniculus
IIRRSGFTYYASWARG

SEQ ID NO: 559 - protein, 16 aa, Oryctolagus cuniculus
LISRSGRTYYATWAKG

SEQ ID NO: 560 - protein, 18 aa, Oryctolagus cuniculus
CIYTGTTGSTYYASWAKY

SEQ ID NO: 561 - protein, 17 aa, Oryctolagus cuniculus
CIAIINSITYYANWAKG

SEQ ID NO: 562 - protein, 18 aa, Oryctolagus cuniculus
CIYSDGSGSTYYANWAKG

SEQ ID NO: 563 - protein, 16 aa, Oryctolagus cuniculus
FIVGTGDTYYASWAKG

SEQ ID NO: 564 - protein, 16 aa, Oryctolagus cuniculus
VIGKSGSTYYASWAKG

SEQ ID NO: 565 - protein, 17 aa, Oryctolagus cuniculus
SIVSGSGSTYYASWAKG

SEQ ID NO: 566 - protein, 18 aa, Oryctolagus cuniculus
CIYAGSSGSTYYASWAKG

SEQ ID NO: 567 - protein, 16 aa, Oryctolagus cuniculus
IIDIRGTTYYASWAKG

SEQ ID NO: 568 - protein, 18 aa, Oryctolagus cuniculus
CIVAGSSGRTYYANWAKG

SEQ ID NO: 569 - protein, 18 aa, Oryctolagus cuniculus
CIHAGSSGSTYYASWAKG

SEQ ID NO: 570 - protein, 17 aa, Oryctolagus cuniculus
TINAASGATWYASWAKG

SEQ ID NO: 571 - protein, 16 aa, Oryctolagus cuniculus
IISTGGSTYYATWAKG

SEQ ID NO: 572 - protein, 16 aa, Oryctolagus cuniculus
IIINTGYTYYASWAKG

SEQ ID NO: 573 - protein, 16 aa, Oryctolagus cuniculus
HSDIRGSAYYASWAKG

SEQ ID NO: 574 - protein, 18 aa, Oryctolagus cuniculus
CIYAGSNGSTYYASWAKG

SEQ ID NO: 575 - protein, 18 aa, Oryctolagus cuniculus
CIYADGSGSIYCATWAKG

SEQ ID NO: 576 - protein, 17 aa, Oryctolagus cuniculus
CIYIGDGNTYYASWAKG

SEQ ID NO: 577 - protein, 16 aa, Oryctolagus cuniculus
FIKAGGSAGYASWAKG

SEQ ID NO: 578 - protein, 16 aa, Oryctolagus cuniculus
VISSSDSTYYASWAKG

SEQ ID NO: 579 - protein, 18 aa, Oryctolagus cuniculus
CIYGGSSGGTYYASWAKG

SEQ ID NO: 580 - protein, 18 aa, Oryctolagus cuniculus
CIYTSSSGSTYYASWVNG

SEQ ID NO: 581 - protein, 18 aa, Oryctolagus cuniculus
CIYADNSGSTYYASWAKG

SEQ ID NO: 582 - protein, 16 aa, Oryctolagus cuniculus
VIYGSGSTDYASWAKG

SEQ ID NO: 583 - protein, 18 aa, Oryctolagus cuniculus
CIYSDSSGSTYNANWVKG

SEQ ID NO: 584 - protein, 16 aa, Oryctolagus cuniculus
VIGNRGSTDYASWAKG

SEQ ID NO: 585 - protein, 16 aa, Oryctolagus cuniculus
TIYDGGSTYYASWTKG

SEQ ID NO: 586 - protein, 16 aa, Oryctolagus cuniculus
IINIIDNTYYASWAKG

SEQ ID NO: 587 - protein, 16 aa, Oryctolagus cuniculus
TISTGGSAYYASWAKS

SEQ ID NO: 588 - protein, 15 aa, Oryctolagus cuniculus
YINRGNTYYANWAKG

SEQ ID NO: 589 - protein, 18 aa, Oryctolagus cuniculus
CIHAGSSGSAYYASWAKG

SEQ ID NO: 590 - protein, 17 aa, Oryctolagus cuniculus
CIYGGDGNTYYASWAKG

SEQ ID NO: 591 - protein, 16 aa, Oryctolagus cuniculus
YIWSGGSAYYASWAKG

SEQ ID NO: 592 - protein, 18 aa, Oryctolagus cuniculus
CIYAGSSGSTYYASWAKG

SEQ ID NO: 593 - protein, 14 aa, Oryctolagus cuniculus
FPPGTNGGTDYFNI

SEQ ID NO: 594 - protein, 9 aa, Oryctolagus cuniculus
DSGWGAFDP

SEQ ID NO: 595 - protein, 14 aa, Oryctolagus cuniculus
FPPGSNSGTDYFNI

SEQ ID NO: 596 - protein, 7 aa, Oryctolagus cuniculus
NISGSAV

SEQ ID NO: 597 - protein, 17 aa, Oryctolagus cuniculus
DLGAGYAGYGYASDFNL

SEQ ID NO: 598 - protein, 14 aa, Oryctolagus cuniculus
FPPGSNSGTDYFNI

SEQ ID NO: 599 - protein, 9 aa, Oryctolagus cuniculus
DNYDWYFNL

SEQ ID NO: 600 - protein, 14 aa, Oryctolagus cuniculus
FPPGSNSGTDYFNI

SEQ ID NO: 601 - protein, 16 aa, Oryctolagus cuniculus
RDADYVGFIWAYYFNL

SEQ ID NO: 602 - protein, 8 aa, Oryctolagus cuniculus
GNPGWAST

SEQ ID NO: 603 - protein, 15 aa, Oryctolagus cuniculus
GVVIGNAYSMAHFSL

SEQ ID NO: 604 - protein, 17 aa, Oryctolagus cuniculus
RLNYVTYPAYGYGYFNL

SEQ ID NO: 605 - protein, 11 aa, Oryctolagus cuniculus
DKPAGGSSYTL

SEQ ID NO: 606 - protein, 10 aa, Oryctolagus cuniculus
GGGIIYTQNL

SEQ ID NO: 607 - protein, 15 aa, Oryctolagus cuniculus
AGSVGYGYDTAYFNL

SEQ ID NO: 608 - protein, 9 aa, Oryctolagus cuniculus
TLNTLPFNI

SEQ ID NO: 609 - protein, 11 aa, Oryctolagus cuniculus
DLGDDGYAYGL

SEQ ID NO: 610 - protein, 11 aa, Oryctolagus cuniculus
GTGSSHYTSNL

SEQ ID NO: 611 - protein, 11 aa, Oryctolagus cuniculus
DLNGADSGSAL

SEQ ID NO: 612 - protein, 11 aa, Oryctolagus cuniculus
GGDADNFYYNI

SEQ ID NO: 613 - protein, 14 aa, Oryctolagus cuniculus
DFYAGSSGNVNGDI

SEQ ID NO: 614 - protein, 14 aa, Oryctolagus cuniculus
FPPGSNGGTAYFNI

SEQ ID NO: 615 - protein, 9 aa, Oryctolagus cuniculus
DSGWGAFDP

SEQ ID NO: 616 - protein, 9 aa, Oryctolagus cuniculus
DSGWGAFDP

SEQ ID NO: 617 - protein, 7 aa, Oryctolagus cuniculus
GYSDIDI

SEQ ID NO: 618 - protein, 14 aa, Oryctolagus cuniculus
FPPGSNGGTAYFNI

SEQ ID NO: 619 - protein, 15 aa, Oryctolagus cuniculus
GLGRGEYTSNDAFDP

SEQ ID NO: 620 - protein, 10 aa, Oryctolagus cuniculus
GSSDEIALDL

SEQ ID NO: 621 - protein, 13 aa, Oryctolagus cuniculus
GPYYVGSEYVFDP

SEQ ID NO: 622 - protein, 13 aa, Oryctolagus cuniculus
MFYAGDSGHYLHL

SEQ ID NO: 623 - skipped

SEQ ID NO: 624 - protein, 11 aa, Oryctolagus cuniculus
GGYSYGGAVSL

SEQ ID NO: 625 - protein, 11 aa, Oryctolagus cuniculus
GRSGGWDALDP

SEQ ID NO: 626 - protein, 13 aa, Oryctolagus cuniculus
EDYAGGTDYYFRL

SEQ ID NO: 627 - protein, 11 aa, Oryctolagus cuniculus
GGDADNFYYNI

SEQ ID NO: 628 - protein, 14 aa, Oryctolagus cuniculus
DFYAGSSGNVNGDI

SEQ ID NO: 629 - protein, 7 aa, Oryctolagus cuniculus
ELDYFNL

SEQ ID NO: 630 - protein, 14 aa, Oryctolagus cuniculus
DFYAGSSGNVNGDI

SEQ ID NO: 631 - protein, 10 aa, Oryctolagus cuniculus
GAGSNGDFNL

SEQ ID NO: 632 - protein, 11 aa, Oryctolagus cuniculus
GAGSYGGAVRL

SEQ ID NO: 633 - protein, 12 aa, Oryctolagus cuniculus
DGYDDYGDPFNL

SEQ ID NO: 634 - protein, 13 aa, Oryctolagus cuniculus
ISAGSDSYIIDNI

SEQ ID NO: 635 - protein, 11 aa, Oryctolagus cuniculus
DAGNSGYYINL

SEQ ID NO: 636 - protein, 4 aa, Oryctolagus cuniculus
LYKL

SEQ ID NO: 637 - protein, 11 aa, Oryctolagus cuniculus
PYVGYGYATDL

SEQ ID NO: 638 - protein, 11 aa, Oryctolagus cuniculus
DSYAGDYAFNL

SEQ ID NO: 639 - protein, 9 aa, Oryctolagus cuniculus
THNTLPFYI

SEQ ID NO: 640 - protein, 10 aa, Oryctolagus cuniculus
GSGGSDYFNL

SEQ ID NO: 641 - protein, 11 aa, Oryctolagus cuniculus
DLGADGYAYHL

SEQ ID NO: 642 - protein, 13 aa, Oryctolagus cuniculus
DPIYDDYGGRLDL

SEQ ID NO: 643 - protein, 14 aa, Oryctolagus cuniculus
FPPGSNGGTDYFNI

SEQ ID NO: 644 - protein, 11 aa, Oryctolagus cuniculus
DSYAGDYAFNL

SEQ ID NO: 645 - protein, 9 aa, Oryctolagus cuniculus
ARNTLPFNI

SEQ ID NO: 646 - protein, 14 aa, Oryctolagus cuniculus
GLYSASGWSYCFDI

SEQ ID NO: 647 - protein, 13 aa, Oryctolagus cuniculus
FDFLVGLTYAGVL

SEQ ID NO: 648 - protein, 13 aa, Oryctolagus cuniculus
NGASGTYYSSLYI

SEQ ID NO: 649 - protein, 14 aa, Oryctolagus cuniculus
FPPGSNSGTDYFNI

SEQ ID NO: 650 - protein, 6 aa, Oryctolagus cuniculus
GSGWDL

SEQ ID NO: 651 - protein, 11 aa, Oryctolagus cuniculus
GLGAASATWDI

SEQ ID NO: 652 - protein, 11 aa, Oryctolagus cuniculus
DKAGDSYYFNL

SEQ ID NO: 653 - protein, 7 aa, Oryctolagus cuniculus
GVAVGDI

SEQ ID NO: 654 - protein, 7 aa, Oryctolagus cuniculus
GILVSDL

SEQ ID NO: 655 - protein, 13 aa, Oryctolagus cuniculus
GPIMVVSPSYFNF

SEQ ID NO: 656 - protein, 15 aa, Oryctolagus cuniculus
SYYSGGYKYVYVFDL

SEQ ID NO: 657 - protein, 7 aa, Oryctolagus cuniculus
GIAVASL

SEQ ID NO: 658 - protein, 9 aa, Oryctolagus cuniculus
LDTYDDYDL

SEQ ID NO: 659 - protein, 13 aa, Oryctolagus cuniculus
MFYAGDSGHYFDL

SEQ ID NO: 660 - protein, 16 aa, Oryctolagus cuniculus
DSDYDDYGNSYYGMDP

SEQ ID NO: 661 - protein, 11 aa, Oryctolagus cuniculus
EYVGSQGYFNL

SEQ ID NO: 662 - protein, 13 aa, Oryctolagus cuniculus
FDYLVGGTWAGVL

SEQ ID NO: 663 - protein, 12 aa, Oryctolagus cuniculus
GVGDTTDTQLDL

SEQ ID NO: 664 - protein, 10 aa, Oryctolagus cuniculus
DPSAWGGLDL

SEQ ID NO: 665 - protein, 10 aa, Oryctolagus cuniculus
YNNGWDYFNL

SEQ ID NO: 666 - skipped

SEQ ID NO: 667 - protein, 14 aa, Oryctolagus cuniculus
RYGAGSGYFISPNL

SEQ ID NO: 668 - protein, 11 aa, Oryctolagus cuniculus
EYVDSQGYFNL

SEQ ID NO: 669 - protein, 11 aa, Oryctolagus cuniculus
GRSGGWDAFDP

SEQ ID NO: 670 - skipped

SEQ ID NO: 671 - protein, 11 aa, Oryctolagus cuniculus
DTGNSNYQFNL

SEQ ID NO: 672 - protein, 17 aa, Oryctolagus cuniculus
DDVSVGDANYPYTAFDL

SEQ ID NO: 673 - protein, 12 aa, Oryctolagus cuniculus
EAYSSANSYYDL

SEQ ID NO: 674 - protein, 12 aa, Oryctolagus cuniculus
DPTAAGGVYFDL

SEQ ID NO: 675 - protein, 9 aa, Oryctolagus cuniculus
GSGYSKFRL

SEQ ID NO: 676 - protein, 9 aa, Oryctolagus cuniculus
DRGDTDISL

SEQ ID NO: 677 - protein, 13 aa, Oryctolagus cuniculus
GPYYVNNENVFDP

SEQ ID NO: 678 - protein, 11 aa, Oryctolagus cuniculus
SYAGNRYDFAI

SEQ ID NO: 679 - protein, 7 aa, Oryctolagus cuniculus
GPYSFDF

SEQ ID NO: 680 - protein, 12 aa, Oryctolagus cuniculus
GDAYRDDYASDL

SEQ ID NO: 681 - protein, 12 aa, Oryctolagus cuniculus
YIGSVGYRRMDI

SEQ ID NO: 682 - protein, 13 aa, Oryctolagus cuniculus
MFYAGDSGHYFDL

SEQ ID NO: 683 - protein, 13 aa, Oryctolagus cuniculus
NGAGGYYYSSLYI

SEQ ID NO: 684 - protein, 9 aa, Oryctolagus cuniculus
DRGGTDISL

SEQ ID NO: 685 - protein, 11 aa, Oryctolagus cuniculus
SSSTYAYGFDP

SEQ ID NO: 686 - protein, 9 aa, Oryctolagus cuniculus
KGYFHYFNL

SEQ ID NO: 687 - protein, 11 aa, Oryctolagus cuniculus
DRAGNSYYFNL

SEQ ID NO: 688 - protein, 4 aa, Oryctolagus cuniculus
VWSL

SEQ ID NO: 689 - protein, 11 aa, Oryctolagus cuniculus
GYDGYGYVLVL

SEQ ID NO: 690 - protein, 12 aa, Oryctolagus cuniculus
DPTAAGGVYFDL

SEQ ID NO: 691 - protein, 14 aa, Oryctolagus cuniculus
GSGSIYYTPSYFDL

SEQ ID NO: 692 - skipped

SEQ ID NO: 693 - protein, 10 aa, Oryctolagus cuniculus
DDKVEHGYGL

SEQ ID NO: 694 - protein, 19 aa, Oryctolagus cuniculus
SMEAYGYAGYAMPGYYFNL

SEQ ID NO: 695 - protein, 16 aa, Oryctolagus cuniculus
DSDYDDYGDSYYGMDP

SEQ ID NO: 696 - protein, 18 aa, Oryctolagus cuniculus
DYDTYDYDGYTYAAGFDL

SEQ ID NO: 697 - protein, 11 aa, Oryctolagus cuniculus
GLGGASTTWDI

SEQ ID NO: 698 - protein, 14 aa, Oryctolagus cuniculus
DIITDSVWITRLDL

SEQ ID NO: 699 - protein, 13 aa, Oryctolagus cuniculus
FDYLVGDTYAGVL

SEQ ID NO: 700 - protein, 14 aa, Oryctolagus cuniculus
MFYAGDSSGNYLHL

SEQ ID NO: 701 - protein, 12 aa, Oryctolagus cuniculus
EGSSAYPSYFNF

SEQ ID NO: 702 - protein, 11 aa, Oryctolagus cuniculus
SYGGNRYDFNI

SEQ ID NO: 703 - protein, 14 aa, Oryctolagus cuniculus
MFYAGHTSGHYFDL

SEQ ID NO: 704 - protein, 21 aa, Oryctolagus cuniculus
GFDYTYGDAGYTYSTSHYFNL

SEQ ID NO: 705 - protein, 11 aa, Oryctolagus cuniculus
EGADYQGHFNL

SEQ ID NO: 706 - protein, 16 aa, Oryctolagus cuniculus
DSDYDDYGNSYYGMDP

SEQ ID NO: 707 - protein, 14 aa, Oryctolagus cuniculus
EIGSGYDAPYYFNL

SEQ ID NO: 708 - protein, 10 aa, Oryctolagus cuniculus
DDRVEHGYGL

SEQ ID NO: 709 - protein, 11 aa, Oryctolagus cuniculus
DLSSSIYDMDL

SEQ ID NO: 710 - protein, 12 aa, Oryctolagus cuniculus
VLNGWGEYYFNL

SEQ ID NO: 711 - protein, 7 aa, Oryctolagus cuniculus
GVAAGDI

SEQ ID NO: 712 - protein, 7 aa, Oryctolagus cuniculus
NISGSAV

SEQ ID NO: 713 - protein, 11 aa, Oryctolagus cuniculus
GGDGYGYVLVL

SEQ ID NO: 714 - protein, 7 aa, Oryctolagus cuniculus
GISYALL

SEQ ID NO: 715 - protein, 10 aa, Oryctolagus cuniculus
GGVGHEVNNL

SEQ ID NO: 716 - protein, 12 aa, Oryctolagus cuniculus
KLSDWDYGYFNL

SEQ ID NO: 717 - protein, 18 aa, Oryctolagus cuniculus
GYAGYYGYGYPTPSWLDL

SEQ ID NO: 718 - protein, 13 aa, Oryctolagus cuniculus
GGTTGSNYYGMDP

SEQ ID NO: 719 - protein, 4 aa, Oryctolagus cuniculus
GIRF

SEQ ID NO: 720 - protein, 17 aa, Oryctolagus cuniculus
VLGAGSSYYTSYDRLDL

SEQ ID NO: 721 - protein, 10 aa, Oryctolagus cuniculus
IADVNTQLDL

SEQ ID NO: 722 - protein, 11 aa, Oryctolagus cuniculus
GAGYAGYGFNL

SEQ ID NO: 723 - protein, 15 aa, Oryctolagus cuniculus
GNAGSYWDIYYGMDL

SEQ ID NO: 724 - protein, 10 aa, Oryctolagus cuniculus
GSGGYFVDNL

SEQ ID NO: 725 - protein, 13 aa, Oryctolagus cuniculus
MFYAGDSGHYFDL

SEQ ID NO: 726 - protein, 12 aa, Oryctolagus cuniculus
DHPAFSTVDLDI

SEQ ID NO: 727 - protein, 11 aa, Oryctolagus cuniculus
DAGSSGYYINL

SEQ ID NO: 728 - protein, 10 aa, Oryctolagus cuniculus
YNNGWDYFNL

SEQ ID NO: 729 - protein, 11 aa, Oryctolagus cuniculus
HKPAGGSSYIL

SEQ ID NO: 730 - protein, 7 aa, Oryctolagus cuniculus
GILVSNL

SEQ ID NO: 731 - protein, 7 aa, Oryctolagus cuniculus
GTYPFTL

SEQ ID NO: 732 - protein, 13 aa, Oryctolagus cuniculus
GSGYGTGWDAFDP

SEQ ID NO: 733 - protein, 9 aa, Oryctolagus cuniculus
GSTNMEFWF

SEQ ID NO: 734 - protein, 14 aa, Oryctolagus cuniculus
ADYYPDTTGWYLNI

SEQ ID NO: 735 - protein, 8 aa, Oryctolagus cuniculus
DGDSYFKL

SEQ ID NO: 736 - protein, 11 aa, Oryctolagus cuniculus
DSYGGDYAFNL

SEQ ID NO: 737 - protein, 12 aa, Oryctolagus cuniculus
DGYDDYGDPFNL

SEQ ID NO: 738 - protein, 18 aa, Oryctolagus cuniculus
LHYSPYGDAGYPYVSFNL

SEQ ID NO: 739 - protein, 9 aa, Oryctolagus cuniculus
NGASGTFDI

SEQ ID NO: 740 - protein, 11 aa, Oryctolagus cuniculus
GGGSGGVDNNL

SEQ ID NO: 741 - protein, 13 aa, Oryctolagus cuniculus
QASQSLYNNKNLA

SEQ ID NO: 742 - protein, 13 aa, Oryctolagus cuniculus
QSSQSVYDKKWLG

SEQ ID NO: 743 - protein, 13 aa, Oryctolagus cuniculus
QASQSLYNNKNLA

SEQ ID NO: 744 - protein, 13 aa, Oryctolagus cuniculus
QSSESVYNNNLLS

SEQ ID NO: 745 - protein, 11 aa, Oryctolagus cuniculus
QASQSVSNLLA

SEQ ID NO: 746 - protein, 13 aa, Oryctolagus cuniculus
QASQSLYNNKNLA

SEQ ID NO: 747 - protein, 11 aa, Oryctolagus cuniculus
QASEDIESYLA

SEQ ID NO: 748 - protein, 13 aa, Oryctolagus cuniculus
QASQSLYNNKNLG

SEQ ID NO: 749 - protein, 11 aa, Oryctolagus cuniculus
QASQTISSYLA

SEQ ID NO: 750 - protein, 13 aa, Oryctolagus cuniculus
QSSQSVYDNNALA

SEQ ID NO: 751 - protein, 13 aa, Oryctolagus cuniculus
QSSQNVDRNNRLA

SEQ ID NO: 752 - protein, 11 aa, Oryctolagus cuniculus
QASQSIGSNLA

SEQ ID NO: 753 - protein, 11 aa, Oryctolagus cuniculus
QASEDIESYLA

SEQ ID NO: 754 - protein, 11 aa, Oryctolagus cuniculus
QASEDIESYLA

SEQ ID NO: 755 - protein, 11 aa, Oryctolagus cuniculus
QASQNIYDNLA

SEQ ID NO: 756 - protein, 13 aa, Oryctolagus cuniculus
QSSPSVYNNNRLS

SEQ ID NO: 757 - protein, 11 aa, Oryctolagus cuniculus
QASQNIGNNLA

SEQ ID NO: 758 - protein, 11 aa, Oryctolagus cuniculus
QASEDIESYLA

SEQ ID NO: 759 - protein, 11 aa, Oryctolagus cuniculus
QASQNINSWLS

SEQ ID NO: 760 - protein, 13 aa, Oryctolagus cuniculus
QSSQSVYSNNHLA

SEQ ID NO: 761 - protein, 13 aa, Oryctolagus cuniculus
QSSQIVHNNNNLA

SEQ ID NO: 762 - protein, 13 aa, Oryctolagus cuniculus
QASQSLYNKKNLA

SEQ ID NO: 763 - protein, 13 aa, Oryctolagus cuniculus
QSSQSVYDNKWLG

SEQ ID NO: 764 - protein, 13 aa, Oryctolagus cuniculus
QSSQSVYDNKWLG

SEQ ID NO: 765 - protein, 13 aa, Oryctolagus cuniculus
QSSKSVFDNNWLS

SEQ ID NO: 766 - protein, 13 aa, Oryctolagus cuniculus
QASQSLYNKKNLA

SEQ ID NO: 767 - protein, 11 aa, Oryctolagus cuniculus
QASETIYSYLN

SEQ ID NO: 768 - protein, 13 aa, Oryctolagus cuniculus
QSSQNIYNKNQLS

SEQ ID NO: 769 - protein, 11 aa, Oryctolagus cuniculus
QASQSIGGSLA

SEQ ID NO: 770 - protein, 13 aa, Oryctolagus cuniculus
QSSQSVNNNKNLA

SEQ ID NO: 771 - protein, 11 aa, Oryctolagus cuniculus
QASQNIGSTLA

SEQ ID NO: 772 - protein, 11 aa, Oryctolagus cuniculus
QASEDIETYLA

SEQ ID NO: 773 - protein, 11 aa, Oryctolagus cuniculus
QASEDIENYLA

SEQ ID NO: 774 - protein, 12 aa, Oryctolagus cuniculus
QSSQSVDNNWLS

SEQ ID NO: 775 - protein, 13 aa, Oryctolagus cuniculus
QSSQSVYSNNHLA

SEQ ID NO: 776 - protein, 13 aa, Oryctolagus cuniculus
QSSQSVHNNNNLA

SEQ ID NO: 777 - protein, 11 aa, Oryctolagus cuniculus
QASEDISSSLA

SEQ ID NO: 778 - protein, 13 aa, Oryctolagus cuniculus
QASQSVHNNNNLA

SEQ ID NO: 779 - protein, 11 aa, Oryctolagus cuniculus
QASEDIESYLA

SEQ ID NO: 780 - protein, 11 aa, Oryctolagus cuniculus
QATEDIESFLA

SEQ ID NO: 781 - protein, 11 aa, Oryctolagus cuniculus
RASEDIKSYLA

SEQ ID NO: 782 - protein, 13 aa, Oryctolagus cuniculus
QASQSVYNHKNLA

SEQ ID NO: 783 - protein, 11 aa, Oryctolagus cuniculus
QASQSIGSSLA

SEQ ID NO: 784 - protein, 13 aa, Oryctolagus cuniculus
QSSQSVYGVNELS

SEQ ID NO: 785 - protein, 11 aa, Oryctolagus cuniculus
QASQSISNLLA

SEQ ID NO: 786 - protein, 13 aa, Oryctolagus cuniculus
QSSKSVYNNNWLS

SEQ ID NO: 787 - protein, 13 aa, Oryctolagus cuniculus
QSSPSVYNNNRLS

SEQ ID NO: 788 - protein, 11 aa, Oryctolagus cuniculus
QASQSIGSYLS

SEQ ID NO: 789 - protein, 11 aa, Oryctolagus cuniculus
QASQNIGNNLA

SEQ ID NO: 790 - protein, 11 aa, Oryctolagus cuniculus
QASEDIYSNLA

SEQ ID NO: 791 - protein, 13 aa, Oryctolagus cuniculus
QASQSLYNNKNLA

SEQ ID NO: 792 - protein, 13 aa, Oryctolagus cuniculus
QSSKTVYNNNWLA

SEQ ID NO: 793 - protein, 13 aa, Oryctolagus cuniculus
QSSPSVYNNVRLS

SEQ ID NO: 794 - protein, 12 aa, Oryctolagus cuniculus
QSSQSVYSTNLA

SEQ ID NO: 795 - protein, 11 aa, Oryctolagus cuniculus
QASENIANHLA

SEQ ID NO: 796 - protein, 13 aa, Oryctolagus cuniculus
QSSQSVYGNNELS

SEQ ID NO: 797 - protein, 13 aa, Oryctolagus cuniculus
QASQSLYNKKNLA

SEQ ID NO: 798 - protein, 13 aa, Oryctolagus cuniculus
QSSQSVYGSDALA

SEQ ID NO: 799 - protein, 11 aa, Oryctolagus cuniculus
QASQSISSNLA

SEQ ID NO: 800 - protein, 11 aa, Oryctolagus cuniculus
QASENIYSFLA

SEQ ID NO: 801 - protein, 11 aa, Oryctolagus cuniculus
QASQSISDYLS

SEQ ID NO: 802 - protein, 11 aa, Oryctolagus cuniculus
QASQSISSYLS

SEQ ID NO: 803 - protein, 11 aa, Oryctolagus cuniculus
QASQNINNLLA

SEQ ID NO: 804 - protein, 13 aa, Oryctolagus cuniculus
QASQSVYANNYLA

SEQ ID NO: 805 - protein, 11 aa, Oryctolagus cuniculus
QASESISNYLS

SEQ ID NO: 806 - protein, 13 aa, Oryctolagus cuniculus
QSSQSVYNNNWLS

SEQ ID NO: 807 - protein, 13 aa, Oryctolagus cuniculus
QASQSVHKHKNLA

SEQ ID NO: 808 - protein, 11 aa, Oryctolagus cuniculus
QASQSISSYLS

SEQ ID NO: 809 - protein, 11 aa, Oryctolagus cuniculus
QASQNINNELS

SEQ ID NO: 810 - protein, 11 aa, Oryctolagus cuniculus
RASEDIESYLA

SEQ ID NO: 811 - protein, 13 aa, Oryctolagus cuniculus
QSSQSVYNDNDLA

SEQ ID NO: 812 - protein, 11 aa, Oryctolagus cuniculus
QASESIYSGLA

SEQ ID NO: 813 - protein, 11 aa, Oryctolagus cuniculus
QASQSISYYLN

SEQ ID NO: 814 - protein, 13 aa, Oryctolagus cuniculus
QASQSVYKNNYLA

SEQ ID NO: 815 - protein, 13 aa, Oryctolagus cuniculus
QSSQSVYNNNWLG

SEQ ID NO: 816 - protein, 11 aa, Oryctolagus cuniculus
QASEDIYNLLA

SEQ ID NO: 817 - protein, 11 aa, Oryctolagus cuniculus
QASEDIESYLA

SEQ ID NO: 818 - protein, 13 aa, Oryctolagus cuniculus
QASQSVYSNNYLS

SEQ ID NO: 819 - protein, 11 aa, Oryctolagus cuniculus
QASESIDSYLN

SEQ ID NO: 820 - protein, 11 aa, Oryctolagus cuniculus
QASQNIYSSLA

SEQ ID NO: 821 - protein, 11 aa, Oryctolagus cuniculus
QASQSISYYLA

SEQ ID NO: 822 - protein, 11 aa, Oryctolagus cuniculus
QASQNIYSRLA

SEQ ID NO: 823 - protein, 12 aa, Oryctolagus cuniculus
QSSQSVTDNFLS

SEQ ID NO: 824 - protein, 11 aa, Oryctolagus cuniculus
QASEDIESYLA

SEQ ID NO: 825 - protein, 11 aa, Oryctolagus cuniculus
QASQSIGSSLA

SEQ ID NO: 826 - protein, 11 aa, Oryctolagus cuniculus
QASQSISSYLA

SEQ ID NO: 827 - protein, 11 aa, Oryctolagus cuniculus
QASQNIGSDLA

SEQ ID NO: 828 - protein, 11 aa, Oryctolagus cuniculus
QASQSISSYLA

SEQ ID NO: 829 - protein, 13 aa, Oryctolagus cuniculus
QASESVVGKNELS

SEQ ID NO: 830 - protein, 13 aa, Oryctolagus cuniculus
QASQSVHNNKNLA

SEQ ID NO: 831 - protein, 13 aa, Oryctolagus cuniculus
QSSQSVYRNNELS

SEQ ID NO: 832 - protein, 11 aa, Oryctolagus cuniculus
QASEDIESFLA

SEQ ID NO: 833 - protein, 11 aa, Oryctolagus cuniculus
QASEDISSRLA

SEQ ID NO: 834 - protein, 11 aa, Oryctolagus cuniculus
QASQNIYSNLA

SEQ ID NO: 835 - protein, 11 aa, Oryctolagus cuniculus
QASENIYSFLA

SEQ ID NO: 836 - protein, 13 aa, Oryctolagus cuniculus
QSSQSVADNNLLA

SEQ ID NO: 837 - protein, 13 aa, Oryctolagus cuniculus
QASQSVYGTNRLA

SEQ ID NO: 838 - protein, 11 aa, Oryctolagus cuniculus
QASQNIYSKFA

SEQ ID NO: 839 - protein, 11 aa, Oryctolagus cuniculus
QASQSIGVSLA

SEQ ID NO: 840 - protein, 13 aa, Oryctolagus cuniculus
QASQSVYNNNYLG

SEQ ID NO: 841 - protein, 11 aa, Oryctolagus cuniculus
QASESIDNWLA

SEQ ID NO: 842 - protein, 13 aa, Oryctolagus cuniculus
QSSQSVYSNNNLA

SEQ ID NO: 843 - protein, 11 aa, Oryctolagus cuniculus
QASQSISSYLS

SEQ ID NO: 844 - protein, 11 aa, Oryctolagus cuniculus
QASQSIRSYLA

SEQ ID NO: 845 - protein, 11 aa, Oryctolagus cuniculus
QASESISVNLA

SEQ ID NO: 846 - protein, 13 aa, Oryctolagus cuniculus
QSSESIYKNNYLA

SEQ ID NO: 847 - protein, 11 aa, Oryctolagus cuniculus
QASQNIYSDFA

SEQ ID NO: 848 - protein, 13 aa, Oryctolagus cuniculus
QASQSVYNHKNLA

SEQ ID NO: 849 - protein, 11 aa, Oryctolagus cuniculus
QASQSISAYLS

SEQ ID NO: 850 - protein, 11 aa, Oryctolagus cuniculus
QASQTITSYLA

SEQ ID NO: 851 - protein, 13 aa, Oryctolagus cuniculus
QASQSVYNNKNLA

SEQ ID NO: 852 - protein, 11 aa, Oryctolagus cuniculus
QASENIYSLLA

SEQ ID NO: 853 - protein, 11 aa, Oryctolagus cuniculus
QASEDIYSLLA

SEQ ID NO: 854 - protein, 11 aa, Oryctolagus cuniculus
QASQSISTYLS

SEQ ID NO: 855 - protein, 11 aa, Oryctolagus cuniculus
QASENIYSSLA

SEQ ID NO: 856 - protein, 11 aa, Oryctolagus cuniculus
QASESIGSWLA

SEQ ID NO: 857 - protein, 13 aa, Oryctolagus cuniculus
QSSQSVYNNNRLS

SEQ ID NO: 858 - protein, 13 aa, Oryctolagus cuniculus
QASQSVYNNNNLA

SEQ ID NO: 859 - protein, 11 aa, Oryctolagus cuniculus
QASQSIGSYLS

SEQ ID NO: 860 - protein, 13 aa, Oryctolagus cuniculus
QSSESVYNNNLLS

SEQ ID NO: 861 - protein, 12 aa, Oryctolagus cuniculus
QASQSVYNNRLA

SEQ ID NO: 862 - protein, 11 aa, Oryctolagus cuniculus
QASQSISTYSS

SEQ ID NO: 863 - protein, 13 aa, Oryctolagus cuniculus
QSSQSVYASVWLG

SEQ ID NO: 864 - protein, 11 aa, Oryctolagus cuniculus
QASQSIYNYLS

SEQ ID NO: 865 - protein, 11 aa, Oryctolagus cuniculus
QASQNIYSYLA

SEQ ID NO: 866 - protein, 11 aa, Oryctolagus cuniculus
QASQSIYSYLA

SEQ ID NO: 867 - protein, 11 aa, Oryctolagus cuniculus
QASESIGSVLA

SEQ ID NO: 868 - protein, 11 aa, Oryctolagus cuniculus
QASQNIYSNLA

SEQ ID NO: 869 - protein, 13 aa, Oryctolagus cuniculus
QSNKNVYDNNALS

SEQ ID NO: 870 - protein, 11 aa, Oryctolagus cuniculus
QASQSIINYLS

SEQ ID NO: 871 - protein, 11 aa, Oryctolagus cuniculus
QASQSIYSYLS

SEQ ID NO: 872 - protein, 11 aa, Oryctolagus cuniculus
QASQSISSWLA

SEQ ID NO: 873 - protein, 13 aa, Oryctolagus cuniculus
QSSQSVNNAKNLA

SEQ ID NO: 874 - protein, 13 aa, Oryctolagus cuniculus
QSSKSVYDNNWLS

SEQ ID NO: 875 - protein, 11 aa, Oryctolagus cuniculus
QASQSIGSSLA

SEQ ID NO: 876 - protein, 11 aa, Oryctolagus cuniculus
QASENIYRNLA

SEQ ID NO: 877 - protein, 11 aa, Oryctolagus cuniculus
QASEDIESYLA

SEQ ID NO: 878 - protein, 11 aa, Oryctolagus cuniculus
QASQSISSWLS

SEQ ID NO: 879 - protein, 11 aa, Oryctolagus cuniculus
QASQSIGSDLA

SEQ ID NO: 880 - protein, 11 aa, Oryctolagus cuniculus
QGSQSISSYLS

SEQ ID NO: 881 - protein, 12 aa, Oryctolagus cuniculus
QSSPSVYSVYLS

SEQ ID NO: 882 - protein, 13 aa, Oryctolagus cuniculus
QSSKSVYNNKWLS

SEQ ID NO: 883 - protein, 11 aa, Oryctolagus cuniculus
QASESVGDALA

SEQ ID NO: 884 - protein, 13 aa, Oryctolagus cuniculus
QSSKTIYNDNWLS

SEQ ID NO: 885 - protein, 11 aa, Oryctolagus cuniculus
RASEDIKSYLA

SEQ ID NO: 886 - protein, 11 aa, Oryctolagus cuniculus
QASQSIYSNLA

SEQ ID NO: 887 - protein, 13 aa, Oryctolagus cuniculus
QASQSVYNNNYLA

SEQ ID NO: 888 - protein, 11 aa, Oryctolagus cuniculus
RASEDIERFLA

SEQ ID NO: 889 - protein, 7 aa, Oryctolagus cuniculus
DVSTLAS

SEQ ID NO: 890 - protein, 7 aa, Oryctolagus cuniculus
KASTLAS

SEQ ID NO: 891 - protein, 7 aa, Oryctolagus cuniculus
DVSTLAS

SEQ ID NO: 892 - protein, 7 aa, Oryctolagus cuniculus
TTSSLAS

SEQ ID NO: 893 - protein, 7 aa, Oryctolagus cuniculus
GASNLES

SEQ ID NO: 894 - protein, 7 aa, Oryctolagus cuniculus
DASTLAS

SEQ ID NO: 895 - protein, 7 aa, Oryctolagus cuniculus
DASDLAS

SEQ ID NO: 896 - protein, 7 aa, Oryctolagus cuniculus
DVSTLAS

SEQ ID NO: 897 - protein, 7 aa, Oryctolagus cuniculus
GASTLAS

SEQ ID NO: 898 - protein, 7 aa, Oryctolagus cuniculus
ETSTLAS

SEQ ID NO: 899 - protein, 7 aa, Oryctolagus cuniculus
YASILAS

SEQ ID NO: 900 - protein, 7 aa, Oryctolagus cuniculus
KASTLAS

SEQ ID NO: 901 - protein, 7 aa, Oryctolagus cuniculus
QASKLAS

SEQ ID NO: 902 - protein, 7 aa, Oryctolagus cuniculus
SASTLAS

SEQ ID NO: 903 - protein, 7 aa, Oryctolagus cuniculus
GASNLES

SEQ ID NO: 904 - protein, 7 aa, Oryctolagus cuniculus
YASTLAS

SEQ ID NO: 905 - protein, 7 aa, Oryctolagus cuniculus
YASTLAS

SEQ ID NO: 906 - protein, 7 aa, Oryctolagus cuniculus
GASNLAS

SEQ ID NO: 907 - protein, 7 aa, Oryctolagus cuniculus
KASTLAS

SEQ ID NO: 908 - protein, 7 aa, Oryctolagus cuniculus
RASKLAS

SEQ ID NO: 909 - protein, 7 aa, Oryctolagus cuniculus
QASTLAS

SEQ ID NO: 910 - protein, 7 aa, Oryctolagus cuniculus
DASTLTS

SEQ ID NO: 911 - protein, 7 aa, Oryctolagus cuniculus
SASTLAS

SEQ ID NO: 912 - protein, 7 aa, Oryctolagus cuniculus
KASTLAS

SEQ ID NO: 913 - protein, 7 aa, Oryctolagus cuniculus
KASTLAS

SEQ ID NO: 914 - protein, 7 aa, Oryctolagus cuniculus
DASTLAS

SEQ ID NO: 915 - protein, 7 aa, Oryctolagus cuniculus
SASTLAS

SEQ ID NO: 916 - protein, 7 aa, Oryctolagus cuniculus
EASKLAS

SEQ ID NO: 917 - protein, 7 aa, Oryctolagus cuniculus
SASNLAS

SEQ ID NO: 918 - protein, 7 aa, Oryctolagus cuniculus
DTSTLAS

SEQ ID NO: 919 - protein, 7 aa, Oryctolagus cuniculus
GASTLSS

SEQ ID NO: 920 - protein, 7 aa, Oryctolagus cuniculus
RASTLAS

SEQ ID NO: 921 - protein, 7 aa, Oryctolagus cuniculus
SASTLAS

SEQ ID NO: 922 - protein, 7 aa, Oryctolagus cuniculus
TTSKLAS

SEQ ID NO: 923 - protein, 7 aa, Oryctolagus cuniculus
RASKLAS

SEQ ID NO: 924 - protein, 7 aa, Oryctolagus cuniculus
QASTLAS

SEQ ID NO: 925 - protein, 7 aa, Oryctolagus cuniculus
RASNLAS

SEQ ID NO: 926 - protein, 7 aa, Oryctolagus cuniculus
QASTLAS

SEQ ID NO: 927 - protein, 7 aa, Oryctolagus cuniculus
RASTLAS

SEQ ID NO: 928 - protein, 7 aa, Oryctolagus cuniculus
RASTLES

SEQ ID NO: 929 - protein, 7 aa, Oryctolagus cuniculus
DASDLAS

SEQ ID NO: 930 - protein, 7 aa, Oryctolagus cuniculus
DTSTLAS

SEQ ID NO: 931 - protein, 7 aa, Oryctolagus cuniculus
YVSNLES

SEQ ID NO: 932 - protein, 7 aa, Oryctolagus cuniculus
KAATLAS

SEQ ID NO: 933 - protein, 7 aa, Oryctolagus cuniculus
DASDLAS

SEQ ID NO: 934 - protein, 7 aa, Oryctolagus cuniculus
GASTLAS

SEQ ID NO: 935 - protein, 7 aa, Oryctolagus cuniculus
YASTLAS

SEQ ID NO: 936 - protein, 7 aa, Oryctolagus cuniculus
DASTLAS

SEQ ID NO: 937 - protein, 7 aa, Oryctolagus cuniculus
DASDLAS

SEQ ID NO: 938 - protein, 7 aa, Oryctolagus cuniculus
SASTLAS

SEQ ID NO: 939 - protein, 7 aa, Oryctolagus cuniculus
DVSTLAS

SEQ ID NO: 940 - protein, 7 aa, Oryctolagus cuniculus
GASTLAS

SEQ ID NO: 941 - protein, 7 aa, Oryctolagus cuniculus
SASTLAS

SEQ ID NO: 942 - protein, 7 aa, Oryctolagus cuniculus
YASTLAS

SEQ ID NO: 943 - protein, 7 aa, Oryctolagus cuniculus
SASALAS

SEQ ID NO: 944 - protein, 7 aa, Oryctolagus cuniculus
DASKLAS

SEQ ID NO: 945 - protein, 7 aa, Oryctolagus cuniculus
DVSTLAS

SEQ ID NO: 946 - protein, 7 aa, Oryctolagus cuniculus
GASTLAS

SEQ ID NO: 947 - protein, 7 aa, Oryctolagus cuniculus
LASTLAS

SEQ ID NO: 948 - protein, 7 aa, Oryctolagus cuniculus
SASTLES

SEQ ID NO: 949 - protein, 7 aa, Oryctolagus cuniculus
RASNLAS

SEQ ID NO: 950 - protein, 7 aa, Oryctolagus cuniculus
DASDLAS

SEQ ID NO: 951 - protein, 7 aa, Oryctolagus cuniculus
KASTLAS

SEQ ID NO: 952 - protein, 7 aa, Oryctolagus cuniculus
KASTLAS

SEQ ID NO: 953 - protein, 7 aa, Oryctolagus cuniculus
YDSTLES

SEQ ID NO: 954 - protein, 7 aa, Oryctolagus cuniculus
GASTLAS

SEQ ID NO: 955 - protein, 7 aa, Oryctolagus cuniculus
EASKLAS

SEQ ID NO: 956 - protein, 7 aa, Oryctolagus cuniculus
RASSLKS

SEQ ID NO: 957 - protein, 7 aa, Oryctolagus cuniculus
KASTLAS

SEQ ID NO: 958 - protein, 7 aa, Oryctolagus cuniculus
SASSLAS

SEQ ID NO: 959 - protein, 7 aa, Oryctolagus cuniculus
GASTLAS

SEQ ID NO: 960 - protein, 7 aa, Oryctolagus cuniculus
RASTLES

SEQ ID NO: 961 - protein, 7 aa, Oryctolagus cuniculus
RASTLAS

SEQ ID NO: 962 - protein, 7 aa, Oryctolagus cuniculus
SASTLDS

SEQ ID NO: 963 - protein, 7 aa, Oryctolagus cuniculus
SASTLAS

SEQ ID NO: 964 - protein, 7 aa, Oryctolagus cuniculus
GASTLAS

SEQ ID NO: 965 - protein, 7 aa, Oryctolagus cuniculus
GASTLAS

SEQ ID NO: 966 - protein, 7 aa, Oryctolagus cuniculus
DASDLAS

SEQ ID NO: 967 - protein, 7 aa, Oryctolagus cuniculus
GASTLAS

SEQ ID NO: 968 - protein, 7 aa, Oryctolagus cuniculus
GASNLES

SEQ ID NO: 969 - protein, 7 aa, Oryctolagus cuniculus
RASTLAS

SEQ ID NO: 970 - protein, 7 aa, Oryctolagus cuniculus
AASTLAS

SEQ ID NO: 971 - protein, 7 aa, Oryctolagus cuniculus
GASTLAS

SEQ ID NO: 972 - protein, 7 aa, Oryctolagus cuniculus
SASTLAS

SEQ ID NO: 973 - protein, 7 aa, Oryctolagus cuniculus
SASNLAS

SEQ ID NO: 974 - protein, 7 aa, Oryctolagus cuniculus
RTSILES

SEQ ID NO: 975 - protein, 7 aa, Oryctolagus cuniculus
DASALAS

SEQ ID NO: 976 - protein, 7 aa, Oryctolagus cuniculus
RASTLAS

SEQ ID NO: 977 - protein, 7 aa, Oryctolagus cuniculus
GTSTLAS

SEQ ID NO: 978 - protein, 7 aa, Oryctolagus cuniculus
DVSTVAS

SEQ ID NO: 979 - protein, 7 aa, Oryctolagus cuniculus
DASNLAS

SEQ ID NO: 980 - protein, 7 aa, Oryctolagus cuniculus
SASTLAS

SEQ ID NO: 981 - protein, 7 aa, Oryctolagus cuniculus
RASTLAS

SEQ ID NO: 982 - protein, 7 aa, Oryctolagus cuniculus
GASNLES

SEQ ID NO: 983 - protein, 7 aa, Oryctolagus cuniculus
DSSTLAS

SEQ ID NO: 984 - protein, 7 aa, Oryctolagus cuniculus
KASTLAS

SEQ ID NO: 985 - protein, 7 aa, Oryctolagus cuniculus
DASTLAS

SEQ ID NO: 986 - protein, 7 aa, Oryctolagus cuniculus
SASTLAS

SEQ ID NO: 987 - protein, 7 aa, Oryctolagus cuniculus
SASTLAS

SEQ ID NO: 988 - protein, 7 aa, Oryctolagus cuniculus
SASKLES

SEQ ID NO: 989 - protein, 7 aa, Oryctolagus cuniculus
SASNLAS

SEQ ID NO: 990 - protein, 7 aa, Oryctolagus cuniculus
DASNLAS

SEQ ID NO: 991 - protein, 7 aa, Oryctolagus cuniculus
RASSLES

SEQ ID NO: 992 - protein, 7 aa, Oryctolagus cuniculus
RASTLES

SEQ ID NO: 993 - protein, 7 aa, Oryctolagus cuniculus
LASTLAS

SEQ ID NO: 994 - protein, 7 aa, Oryctolagus cuniculus
RASTLTS

SEQ ID NO: 995 - protein, 7 aa, Oryctolagus cuniculus
SASALAS

SEQ ID NO: 996 - protein, 7 aa, Oryctolagus cuniculus
SASSLAS

SEQ ID NO: 997 - protein, 7 aa, Oryctolagus cuniculus
DASDLAS

SEQ ID NO: 998 - protein, 7 aa, Oryctolagus cuniculus
RASILES

SEQ ID NO: 999 - protein, 7 aa, Oryctolagus cuniculus
DASKLAS

SEQ ID NO: 1000 - protein, 7 aa, Oryctolagus cuniculus
RASTLAS

SEQ ID NO: 1001 - protein, 7 aa, Oryctolagus cuniculus
AASTLAS

SEQ ID NO: 1002 - protein, 7 aa, Oryctolagus cuniculus
RATTLES

SEQ ID NO: 1003 - protein, 7 aa, Oryctolagus cuniculus
DASDLAS

SEQ ID NO: 1004 - protein, 7 aa, Oryctolagus cuniculus
SASSLAS

SEQ ID NO: 1005 - protein, 7 aa, Oryctolagus cuniculus
RSSTLAS

SEQ ID NO: 1006 - protein, 7 aa, Oryctolagus cuniculus
TASSLAS

SEQ ID NO: 1007 - protein, 7 aa, Oryctolagus cuniculus
YASDLES

SEQ ID NO: 1008 - protein, 7 aa, Oryctolagus cuniculus
KASTLDS

SEQ ID NO: 1009 - protein, 7 aa, Oryctolagus cuniculus
EASTLTS

SEQ ID NO: 1010 - protein, 7 aa, Oryctolagus cuniculus
YASDLES

SEQ ID NO: 1011 - protein, 7 aa, Oryctolagus cuniculus
AASTLAS

SEQ ID NO: 1012 - protein, 7 aa, Oryctolagus cuniculus
GASDLAS

SEQ ID NO: 1013 - protein, 7 aa, Oryctolagus cuniculus
DASDLES

SEQ ID NO: 1014 - protein, 7 aa, Oryctolagus cuniculus
GASTLAS

SEQ ID NO: 1015 - protein, 7 aa, Oryctolagus cuniculus
SASTLAS

SEQ ID NO: 1016 - protein, 7 aa, Oryctolagus cuniculus
GASDLES

SEQ ID NO: 1017 - protein, 7 aa, Oryctolagus cuniculus
RASTLAS

SEQ ID NO: 1018 - protein, 7 aa, Oryctolagus cuniculus
RASTLES

SEQ ID NO: 1019 - protein, 7 aa, Oryctolagus cuniculus
QASILAS

SEQ ID NO: 1020 - protein, 7 aa, Oryctolagus cuniculus
RASTLES

SEQ ID NO: 1021 - protein, 7 aa, Oryctolagus cuniculus
DASTLAS

SEQ ID NO: 1022 - protein, 7 aa, Oryctolagus cuniculus
QASTLAS

SEQ ID NO: 1023 - protein, 7 aa, Oryctolagus cuniculus
YTSTLAS

SEQ ID NO: 1024 - protein, 7 aa, Oryctolagus cuniculus
KASTLAS

SEQ ID NO: 1025 - protein, 7 aa, Oryctolagus cuniculus
SASTLAS

SEQ ID NO: 1026 - protein, 7 aa, Oryctolagus cuniculus
DASDLAS

SEQ ID NO: 1027 - protein, 7 aa, Oryctolagus cuniculus
DASSLES

SEQ ID NO: 1028 - protein, 7 aa, Oryctolagus cuniculus
GASTLAS

SEQ ID NO: 1029 - protein, 7 aa, Oryctolagus cuniculus
RASTLAS

SEQ ID NO: 1030 - protein, 7 aa, Oryctolagus cuniculus
GAFTLAS

SEQ ID NO: 1031 - protein, 7 aa, Oryctolagus cuniculus
RASTLES

SEQ ID NO: 1032 - protein, 7 aa, Oryctolagus cuniculus
GASTLAS

SEQ ID NO: 1033 - protein, 7 aa, Oryctolagus cuniculus
DASDLAS

SEQ ID NO: 1034 - protein, 7 aa, Oryctolagus cuniculus
GASNLES

SEQ ID NO: 1035 - protein, 7 aa, Oryctolagus cuniculus
LASTLAS

SEQ ID NO: 1036 - protein, 7 aa, Oryctolagus cuniculus
KASTLAS

SEQ ID NO: 1037 - protein, 13 aa, Oryctolagus cuniculus
QGEFSCSSGDCYA

SEQ ID NO: 1038 - protein, 10 aa, Oryctolagus cuniculus
AGGYSGNIWS

SEQ ID NO: 1039 - protein, 13 aa, Oryctolagus cuniculus
QGEFSCSSGDCYA

SEQ ID NO: 1040 - protein, 10 aa, Oryctolagus cuniculus
QGGYTDATYA

SEQ ID NO: 1041 - protein, 6 aa, Oryctolagus cuniculus
QSGYYT

SEQ ID NO: 1042 - protein, 13 aa, Oryctolagus cuniculus
QGEFSCGSGDCYA

SEQ ID NO: 1043 - protein, 12 aa, Oryctolagus cuniculus
QSYYYGSSYVVA

SEQ ID NO: 1044 - protein, 13 aa, Oryctolagus cuniculus
QGEFSCSSGDCYA

SEQ ID NO: 1045 - protein, 13 aa, Oryctolagus cuniculus
LYSYYTSNSADNT

SEQ ID NO: 1046 - protein, 11 aa, Oryctolagus cuniculus
AGGYNSGSDAA

SEQ ID NO: 1047 - protein, 10 aa, Oryctolagus cuniculus
QGYYSGDINV

SEQ ID NO: 1048 - protein, 13 aa, Oryctolagus cuniculus
QSYYGTSNSYGDA

SEQ ID NO: 1049 - protein, 13 aa, Oryctolagus cuniculus
QCTLYGVNFVPNV

SEQ ID NO: 1050 - protein, 13 aa, Oryctolagus cuniculus
QCILYGVNFVPNT

SEQ ID NO: 1051 - protein, 13 aa, Oryctolagus cuniculus
QCSYDGGSYVPNA

SEQ ID NO: 1052 - protein, 11 aa, Oryctolagus cuniculus
AGGYSTISDNA

SEQ ID NO: 1053 - protein, 12 aa, Oryctolagus cuniculus
QCTFYGSGYVAA

SEQ ID NO: 1054 - protein, 13 aa, Oryctolagus cuniculus
QCGIYGVNFVPNV

SEQ ID NO: 1055 - protein, 12 aa, Oryctolagus cuniculus
QQGAGWNNLDNA

SEQ ID NO: 1056 - protein, 11 aa, Oryctolagus cuniculus
LGVYDDDADNA

SEQ ID NO: 1057 - protein, 12 aa, Oryctolagus cuniculus
AGGYSTNTDTYI

SEQ ID NO: 1058 - protein, 13 aa, Oryctolagus cuniculus
QGEFSCSAGDCYA

SEQ ID NO: 1059 - protein, 10 aa, Oryctolagus cuniculus
AGGYSGNIWS

SEQ ID NO: 1060 - protein, 10 aa, Oryctolagus cuniculus
AGGYSGNIWS

SEQ ID NO: 1061 - protein, 11 aa, Oryctolagus cuniculus
AGIYSSDSDNA

SEQ ID NO: 1062 - protein, 13 aa, Oryctolagus cuniculus
QGEFSCSSGDCYA

SEQ ID NO: 1063 - protein, 12 aa, Oryctolagus cuniculus
QQGYSGRNVENT

SEQ ID NO: 1064 - protein, 11 aa, Oryctolagus cuniculus
LGGYISSSDTT

SEQ ID NO: 1065 - protein, 12 aa, Oryctolagus cuniculus
QCTYYDDSYDVP

SEQ ID NO: 1066 - protein, 12 aa, Oryctolagus cuniculus
AGGYSSSADTFA

SEQ ID NO: 1067 - protein, 14 aa, Oryctolagus cuniculus
QSNYGSNSGGYVFP

SEQ ID NO: 1068 - protein, 13 aa, Oryctolagus cuniculus
QCTLYGVNFVANA

SEQ ID NO: 1069 - protein, 11 aa, Oryctolagus cuniculus
QSYYDGAVTFT

SEQ ID NO: 1070 - protein, 13 aa, Oryctolagus cuniculus
LGGYDSMSADCFA

SEQ ID NO: 1071 - protein, 11 aa, Oryctolagus cuniculus
LGVYDDDADNA

SEQ ID NO: 1072 - protein, 12 aa, Oryctolagus cuniculus
AGGYSTNTDTFT

SEQ ID NO: 1073 - protein, 14 aa, Oryctolagus cuniculus
QAYYYSISDDLYNA

SEQ ID NO: 1074 - protein, 12 aa, Oryctolagus cuniculus
AGGYSTNTDTFT

SEQ ID NO: 1075 - protein, 13 aa, Oryctolagus cuniculus
QCTIYGVNFVPNA

SEQ ID NO: 1076 - protein, 13 aa, Oryctolagus cuniculus
QCTVYGVNFVANA

SEQ ID NO: 1077 - protein, 10 aa, Oryctolagus cuniculus
QSVWYAGGAA

SEQ ID NO: 1078 - protein, 13 aa, Oryctolagus cuniculus
AGEFSCASADCFA

SEQ ID NO: 1079 - protein, 12 aa, Oryctolagus cuniculus
QSYGYGSGYVFA

SEQ ID NO: 1080 - protein, 13 aa, Oryctolagus cuniculus
LGNYDCESDDCYA

SEQ ID NO: 1081 - protein, 15 aa, Oryctolagus cuniculus
QCTYGSSSSSAYGWA

SEQ ID NO: 1082 - protein, 11 aa, Oryctolagus cuniculus
LGSYISSSDNA

SEQ ID NO: 1083 - protein, 11 aa, Oryctolagus cuniculus
AGGYSSISDNG

SEQ ID NO: 1084 - protein, 14 aa, Oryctolagus cuniculus
QGYYYYISNTYGYP

SEQ ID NO: 1085 - protein, 12 aa, Oryctolagus cuniculus
QCTYGYSGYVSA

SEQ ID NO: 1086 - protein, 12 aa, Oryctolagus cuniculus
LGVYTYISADNA

SEQ ID NO: 1087 - protein, 13 aa, Oryctolagus cuniculus
QGEFSCSSGDCYA

SEQ ID NO: 1088 - protein, 11 aa, Oryctolagus cuniculus
LGSYISSSDNG

SEQ ID NO: 1089 - protein, 11 aa, Oryctolagus cuniculus
AGGYSDISDNA

SEQ ID NO: 1090 - protein, 13 aa, Oryctolagus cuniculus
QGEFNCGSGDCST

SEQ ID NO: 1091 - protein, 12 aa, Oryctolagus cuniculus
QCTFWDINNFGG

SEQ ID NO: 1092 - protein, 11 aa, Oryctolagus cuniculus
LGGYDADADNA

SEQ ID NO: 1093 - protein, 13 aa, Oryctolagus cuniculus
QGEFSCSSGDCYA

SEQ ID NO: 1094 - protein, 10 aa, Oryctolagus cuniculus
AGAYSGNVGT

SEQ ID NO: 1095 - protein, 12 aa, Oryctolagus cuniculus
QQTYSGSNVENS

SEQ ID NO: 1096 - protein, 13 aa, Oryctolagus cuniculus
QQTYIYNNAEDNT

SEQ ID NO: 1097 - protein, 14 aa, Oryctolagus cuniculus
QCTFGATNDDYGNA

SEQ ID NO: 1098 - protein, 15 aa, Oryctolagus cuniculus
QCTVGSSGVTGYGNA

SEQ ID NO: 1099 - protein, 14 aa, Oryctolagus cuniculus
QNYYGYGLSTNYVV

SEQ ID NO: 1100 - protein, 13 aa, Oryctolagus cuniculus
QGEFSCSSGDCTA

SEQ ID NO: 1101 - protein, 14 aa, Oryctolagus cuniculus
QCTAGSINVSYGNA

SEQ ID NO: 1102 - protein, 13 aa, Oryctolagus cuniculus
LGSYDCSSVDCNA

SEQ ID NO: 1103 - protein, 12 aa, Oryctolagus cuniculus
AGGYDSTIDTFT

SEQ ID NO: 1104 - protein, 15 aa, Oryctolagus cuniculus
QCTYGSSTSSRSGNA

SEQ ID NO: 1105 - protein, 15 aa, Oryctolagus cuniculus
QSYYYGISSTYAFYT

SEQ ID NO: 1106 - protein, 12 aa, Oryctolagus cuniculus
QCTYWDSSTVGA

SEQ ID NO: 1107 - protein, 11 aa, Oryctolagus cuniculus
SGGYISSSDNA

SEQ ID NO: 1108 - protein, 11 aa, Oryctolagus cuniculus
QSTYYGSSGNA

SEQ ID NO: 1109 - protein, 13 aa, Oryctolagus cuniculus
LYGYVTSSNADFA

SEQ ID NO: 1110 - protein, 13 aa, Oryctolagus cuniculus
LGTYDCVSADCGA

SEQ ID NO: 1111 - protein, 12 aa, Oryctolagus cuniculus
QGTYSNNGWYFA

SEQ ID NO: 1112 - protein, 15 aa, Oryctolagus cuniculus
QSYYYGISSTYAFYT

SEQ ID NO: 1113 - protein, 11 aa, Oryctolagus cuniculus
QTYYGGINIFT

SEQ ID NO: 1114 - protein, 13 aa, Oryctolagus cuniculus
LGTYDCSSTDCYA

SEQ ID NO: 1115 - protein, 13 aa, Oryctolagus cuniculus
QCTVYGVNFVPNA

SEQ ID NO: 1116 - protein, 12 aa, Oryctolagus cuniculus
QGGYYISSTDNA

SEQ ID NO: 1117 - protein, 12 aa, Oryctolagus cuniculus
QQGYSSSNVDNA

SEQ ID NO: 1118 - protein, 12 aa, Oryctolagus cuniculus
QGGYYGSSDTVT

SEQ ID NO: 1119 - protein, 12 aa, Oryctolagus cuniculus
AGGYSGSSDVFA

SEQ ID NO: 1120 - protein, 13 aa, Oryctolagus cuniculus
QCTVYGVNYVPNA

SEQ ID NO: 1121 - protein, 12 aa, Oryctolagus cuniculus
QCTYYGGSGDVP

SEQ ID NO: 1122 - protein, 14 aa, Oryctolagus cuniculus
QCTYGTTNTGHYVG

SEQ ID NO: 1123 - protein, 11 aa, Oryctolagus cuniculus
QCTYYSGSPHT

SEQ ID NO: 1124 - protein, 16 aa, Oryctolagus cuniculus
QSNYGSSSISNYGGGA

SEQ ID NO: 1125 - protein, 10 aa, Oryctolagus cuniculus
AGGYSGNMYV

SEQ ID NO: 1126 - protein, 12 aa, Oryctolagus cuniculus
AGGYGSYTDTFA

SEQ ID NO: 1127 - protein, 11 aa, Oryctolagus cuniculus
LGGYDDDADNT

SEQ ID NO: 1128 - protein, 13 aa, Oryctolagus cuniculus
QCTIYGVNFVPNA

SEQ ID NO: 1129 - protein, 12 aa, Oryctolagus cuniculus
QSNYAIISCGAA

SEQ ID NO: 1130 - protein, 12 aa, Oryctolagus cuniculus
QSAYYSSSAVYA

SEQ ID NO: 1131 - protein, 13 aa, Oryctolagus cuniculus
QQTYIYNNAESNA

SEQ ID NO: 1132 - protein, 10 aa, Oryctolagus cuniculus
VGGYSTSGYA

SEQ ID NO: 1133 - protein, 13 aa, Oryctolagus cuniculus
QGEFSCSNGDCIA

SEQ ID NO: 1134 - protein, 12 aa, Oryctolagus cuniculus
QGGYYGSSDTVT

SEQ ID NO: 1135 - protein, 12 aa, Oryctolagus cuniculus
QQGYTSSNVDNV

SEQ ID NO: 1136 - protein, 13 aa, Oryctolagus cuniculus
LGSYDCSSADCNV

SEQ ID NO: 1137 - protein, 13 aa, Oryctolagus cuniculus
QSTFYGVNPVPNA

SEQ ID NO: 1138 - protein, 11 aa, Oryctolagus cuniculus
LGVYDDDADNA

SEQ ID NO: 1139 - protein, 15 aa, Oryctolagus cuniculus
QCTYGSSTSSRSGNA

SEQ ID NO: 1140 - protein, 13 aa, Oryctolagus cuniculus
QCTYGSSGSSFLA

SEQ ID NO: 1141 - protein, 12 aa, Oryctolagus cuniculus
QQTYSGSNVENS

SEQ ID NO: 1142 - protein, 11 aa, Oryctolagus cuniculus
AGDYSSSSDNT

SEQ ID NO: 1143 - protein, 12 aa, Oryctolagus cuniculus
QSTYWESNNIGT

SEQ ID NO: 1144 - protein, 12 aa, Oryctolagus cuniculus
AGGYSGSADTFA

SEQ ID NO: 1145 - protein, 11 aa, Oryctolagus cuniculus
QSYAGISSGVA

SEQ ID NO: 1146 - protein, 14 aa, Oryctolagus cuniculus
QCTYGTTNTGHYVG

SEQ ID NO: 1147 - protein, 12 aa, Oryctolagus cuniculus
AGGYDSSVDTFA

SEQ ID NO: 1148 - protein, 15 aa, Oryctolagus cuniculus
QSHYCCSSNYDYIYA

SEQ ID NO: 1149 - protein, 14 aa, Oryctolagus cuniculus
QSYYYSISDSVDYP

SEQ ID NO: 1150 - protein, 15 aa, Oryctolagus cuniculus
QCTYGSSASSSYGNA

SEQ ID NO: 1151 - protein, 11 aa, Oryctolagus cuniculus
QTYYPSSVTYA

SEQ ID NO: 1152 - protein, 13 aa, Oryctolagus cuniculus
QSTFYGVNPVPTA

SEQ ID NO: 1153 - protein, 11 aa, Oryctolagus cuniculus
AGGYSSSSDNA

SEQ ID NO: 1154 - protein, 10 aa, Oryctolagus cuniculus
QGYYSGYINA

SEQ ID NO: 1155 - protein, 14 aa, Oryctolagus cuniculus
QCTYGSISSSAGNA

SEQ ID NO: 1156 - protein, 10 aa, Oryctolagus cuniculus
QGGYTDATYA

SEQ ID NO: 1157 - protein, 13 aa, Oryctolagus cuniculus
QGEFSCSNGDCIA

SEQ ID NO: 1158 - protein, 14 aa, Oryctolagus cuniculus
QCTYGSISSSSGNA

SEQ ID NO: 1159 - protein, 10 aa, Oryctolagus cuniculus
AGGYIGDIYA

SEQ ID NO: 1160 - protein, 15 aa, Oryctolagus cuniculus
QCTYGSSRVSSYGDA

SEQ ID NO: 1161 - protein, 10 aa, Oryctolagus cuniculus
QSYYGISAYA

SEQ ID NO: 1162 - protein, 13 aa, Oryctolagus cuniculus
QDNYGSSTTYGNS

SEQ ID NO: 1163 - protein, 15 aa, Oryctolagus cuniculus
QSYYHSTSGSSYGNT

SEQ ID NO: 1164 - protein, 13 aa, Oryctolagus cuniculus
QSTYYNISADFYA

SEQ ID NO: 1165 - protein, 11 aa, Oryctolagus cuniculus
AGDYISDSDNT

SEQ ID NO: 1166 - protein, 15 aa, Oryctolagus cuniculus
QCTYGSSSGSYGGWA

SEQ ID NO: 1167 - protein, 12 aa, Oryctolagus cuniculus
QSNYGFSSGSYA

SEQ ID NO: 1168 - protein, 14 aa, Oryctolagus cuniculus
QCTYGSLSSTYGWA

SEQ ID NO: 1169 - protein, 12 aa, Oryctolagus cuniculus
AGGYDRFIDTFA

SEQ ID NO: 1170 - protein, 11 aa, Oryctolagus cuniculus
AGGYITNSDNG

SEQ ID NO: 1171 - protein, 12 aa, Oryctolagus cuniculus
QSYGYGSGYVFA

SEQ ID NO: 1172 - protein, 13 aa, Oryctolagus cuniculus
LYSYYIDSNVDFA

SEQ ID NO: 1173 - protein, 13 aa, Oryctolagus cuniculus
QCTLYGVNFVPNV

SEQ ID NO: 1174 - protein, 15 aa, Oryctolagus cuniculus
QCTVGSSGVTGYGNA

SEQ ID NO: 1175 - protein, 11 aa, Oryctolagus cuniculus
QCTYYGGSPNV

SEQ ID NO: 1176 - protein, 12 aa, Oryctolagus cuniculus
QQGYTTSNVDNT

SEQ ID NO: 1177 - protein, 11 aa, Oryctolagus cuniculus
AGAYVGSSDNT

SEQ ID NO: 1178 - protein, 11 aa, Oryctolagus cuniculus
AGDYSSNSDDA

SEQ ID NO: 1179 - protein, 14 aa, Oryctolagus cuniculus
QSYWYTMGNSYGNT

SEQ ID NO: 1180 - protein, 11 aa, Oryctolagus cuniculus
LGSYINSSDNA

SEQ ID NO: 1181 - protein, 13 aa, Oryctolagus cuniculus
QSAYYSSSTDGGA

SEQ ID NO: 1182 - protein, 13 aa, Oryctolagus cuniculus
QGYYYADSDDNIA

SEQ ID NO: 1183 - protein, 10 aa, Oryctolagus cuniculus
QGYYSTGMFA

SEQ ID NO: 1184 - protein, 13 aa, Oryctolagus cuniculus
QCTLYGVNFVPNA

SEQ ID NO: 1185 - protein, 117 aa, synthetic construct
  source 1..117: note = MAB-17-0119 HC VR
EVQLEESGGRLVQPGTSLRLSCAVSGFSLNSYDMSWVRQAPGKGLEYVGIIYNSGTTYYANWAKGRFTISKDTSKTTLYLQMNSLRAEDTATYFCARTHNTLPFYIWGQGTLVTVSS

SEQ ID NO: 1186 - protein, 122 aa, synthetic construct
  source 1..122: note = MAB-17-0127 HC VR
EVQLVESGGGLVQPGGSLRLSCAASGFSFSSSYYMCWVRQAPGKGLEWVACIYAGSSGSTYYASWAKGRFTISKDISKTTLYLQMNSLRAEDTAVYFCARGGGSGGVDNNLWGQGTLVTVSS

SEQ ID NO: 1187 - protein, 121 aa, synthetic construct
  source 1..121: note = MAB-17-0193 HC VR
EVQLEESGGGLVQPGGSLRLSCAASGFSFNNNYYMCWVRQAPGKGLEWVACIYTGSTGSTYYANWAKGRFTISKDLSKTTLYLQMNSLRAEDTATYFCARDDKVEHGYGLWGQGTLVTVSS

SEQ ID NO: 1188 - protein, 123 aa, synthetic construct
  source 1..123: note = MAB-17-0200 HC VR
EVQLEESGGRLVQPGTSLRLSCAASGFSLSSNSISWVRQAPGKGLEWVGIISSSGSTYYASWAKGRFTISKDASKTTLYLQMNSLRAEDTATYFCAKGLGRGEYTSNDAFDPWGQGTLVTVSS

SEQ ID NO: 1189 - protein, 122 aa, synthetic construct
  source 1..122: note = MAB-17-0201 HC VR
EVQLEESGGDLVQPGGSLRLSCAASGFSFNGNYYICWVRQAPGKGLEWVACIYAGSSGSTYYASWAKGRFTISRDTSKNTLYLQMNSLRAEDTAVYFCVRDKPAGGSSYTLWGQGTLVTVSS

SEQ ID NO: 1190 - protein, 122 aa, synthetic construct
  source 1..122: note = MAB-17-0212 HC VR
EVQLEESGGDLVQPGGSLRLSCAASGFDFSSNYYMCWVRQAPGKGLEWVACIYTGSSGSTYYASWAKGRFTISKDTSKNTLYLQMNSLRAEDTAVYFCARGAGSYGGAVRLWGQGTLVTVSS

SEQ ID NO: 1191 - protein, 121 aa, synthetic construct
  source 1..121: note = MAB-17-0218 HC VR
EVQLEESGGDLVQPGGSLRLSCAASGFSFSRSYYMCWVRQAPGKGLEWVACIYAGSSDSTYYASWAKGRFTISRDTSKNTLYLQMNSLRAEDTAVYFCARGGGIIYTQNLWGQGTLVTVSS

SEQ ID NO: 1192 - protein, 121 aa, synthetic construct
  source 1..121: note = MAB-17-0223 HC VR
EVQLEESGGDLVQPGGSLRLSCAASGFSFSSSYYMCWVRQAPGKGLEWVACIYAGSSGSTYYASWAKGRFTISRDNSKNTLYLQMNSLRAEDTAVYFCARGAGSNGDFNLWGQGTLVTVSS

SEQ ID NO: 1193 - protein, 120 aa, synthetic construct
  source 1..120: note = MAB-17-0225 HC VR
EVQLEESGGDLVQPGGSLRLSCAASGFSFSSSYYMCWVRQAPGKGLEWVACVYAGSSGSTYYASWAKGRFTISRDNSKNTLYLQMNSLRAEDTAVYFCARDRGGTDISLWGQGTLVTVSS

SEQ ID NO: 1194 - protein, 111 aa, synthetic construct
  source 1..111: note = MAB-17-0119 LC VR
DIVMTQSPSSLSASVGDRVTITCQSSPSVYNNNRLSWFQQKPGQAPKLLIYYASTLASGVPSRFSGSGSGTDFTLTISSLQPEDFATYYCAGGYSSISDNGFGQGTKVVIK

SEQ ID NO: 1195 - protein, 111 aa, synthetic construct
  source 1..111: note = MAB-17-0127 LC VR
DIQMTQSPSSLSASVGDRVTITCRASEDIERFLAWYQQKPGQAPKLLIYKASTLASGVPSRFSGSGSGTDFTLTISSLQPEDFATYYCQCTLYGVNFVPNAFGGGTKVVIK

SEQ ID NO: 1196 - protein, 111 aa, synthetic construct
  source 1..111: note = MAB-17-0193 LC VR
DIQMTQSPSSLSASVGDRVTITCQASESIDNWLAWYQQKPGQAPKLLIYSASNLASGVPSRFSGSGSGTDFTLTISSLQPEDFATYYCQSTFYGVNPVPNAFGQGTKVVIK

SEQ ID NO: 1197 - protein, 110 aa, synthetic construct
  source 1..110: note = MAB-17-0200 LC VR
DIQMTQSPSSLSASVGDRVTITCQASETIYSYLNWYQQKPGQAPKLLIYSASTLASGVPSRFSGSGSGTDFTLTISSLQPEDFATYYCQQGYSGRNVENTFGQGTKVVIK

SEQ ID NO: 1198 - protein, 111 aa, synthetic construct
  source 1..111: note = MAB-17-0201 LC VR
DIQMTQSPSSLSASVGDRVTITCQASEDIESYLAWYQQKPGQAPKLLIYQASKLASGVPSRFSGSGSGTDFTLTISSLQPEDFATYYCQCTLYGVNFVPNVFGGGTKVVIK

SEQ ID NO: 1199 - protein, 111 aa, synthetic construct
  source 1..111: note = MAB-17-0212 LC VR
DIQMTQSPSSLSASVGDRVTITCQATEDIESFLAWYQQKPGQAPKLLIYRASTLESGVPSRFSGSGSGTDFTLTISSLQPEDFATYYCQCTVYGVNFVANAFGGGTKVVIK

SEQ ID NO: 1200 - protein, 111 aa, synthetic construct
  source 1..111: note = MAB-17-0218 LC VR
DIQMTQSPSSLSASVGDRVTITCQASEDIESYLAWYQQKPGQAPKLLIYSASTLASGVPSRFSGSGSGTDFTLTISSLQPEDFATYYCQCILYGVNFVPNTFGGGTKVVIK

SEQ ID NO: 1201 - protein, 111 aa, synthetic construct
  source 1..111: note = MAB-17-0223 LC VR
DIQMTQSPSSLSASVGDRVTITCQASEDIESYLAWYQQKPGQAPKLLIYRASTLASGVPSRFSGSGSGTDFTLTISSLQPEDFATYYCQCTIYGVNFVPNAFGGGTKVVIK

SEQ ID NO: 1202 - protein, 111 aa, synthetic construct
  source 1..111: note = MAB-17-0225 LC VR
DIQMTQSPSSLSASVGDRVTITCQASEDIESFLAWYQQKPGQAPKLLIYSASTLASGVPSRFSGSGSGTDFTLTISSLQPEDFATYFCQCTIYGVNFVPNAFGGGTKVVIK

SEQ ID NO: 1203 - protein, 111 aa, synthetic construct
  source 1..111: note = MAB-17-0545 LC VR
DIQMTQSPSSLSASVGDRVTITCQASEDIESYLAWYQQKPGQAPKLLIYQASKLASGVPSRFSGSGSGTDFTLTISSLQPEDFATYYCQSTLYGVNFVPNVFGGGTKVVIK

SEQ ID NO: 1204 - protein, 111 aa, synthetic construct
  source 1..111: note = MAB-17-0547 LC VR
DIQMTQSPSSLSASVGDRVTITCQASEDIESYLAWYQQKPGQAPKLLIYRASTLASGVPSRFSGSGSGTDFTLTISSLQPEDFATYYCQSTIYGVNFVPNAFGGGTKVVIK

SEQ ID NO: 1205 - protein, 13 aa, synthetic construct
  source 1..13: note = MAB-17-0545 CDR H3
QSTLYGVNFVPNV

SEQ ID NO: 1206 - protein, 13 aa, synthetic construct
  source 1..13: note = MAB-17-0547 CDR H3
QSTIYGVNFVPNA